European Patent Specification EP 3 833 746 B1, published March 29, 2023. Title: MINI-GDE FOR THE TREATMENT OF GLYCOGEN STORAGE DISEASE III. Applicant: GENETHON ET AL. The sequence listing filed with the application follows.

SEQUENCE LISTING (63 sequences)

SEQ ID NO: 1 - protein, 1532 aa, Homo sapiens
MGHSKQIRILLLNEMEKLEKTLFRLEQGYELQFRLGPTLQGKAVTVYTNYPFPGETFNREKFRSLDWENPTEREDDSDKYCKLNLQQSGSFQYYFLQGNEKSGGGYIVVDPILRVGADNHVLPLDCVTLQTFLAKCLGPFDEWESRLRVAKESGYNMIHFTPLQTLGLSRSCYSLANQLELNPDFSRPNRKYTWNDVGQLVEKLKKEWNVICITDVVYNHTAANSKWIQEHPECAYNLVNSPHLKPAWVLDRALWRFSCDVAEGKYKEKGIPALIENDHHMNSIRKIIWEDIFPKLKLWEFFQVDVNKAVEQFRRLLTQENRRVTKSDPNQHLTIIQDPEYRRFGCTVDMNIALTTFIPHDKGPAAIEECCNWFHKRMEELNSEKHRLINYHQEQAVNCLLGNVFYERLAGHGPKLGPVTRKHPLVTRYFTFPFEEIDFSMEESMIHLPNKACFLMAHNGWVMGDDPLRNFAEPGSEVYLRRELICWGDSVKLRYGNKPEDCPYLWAHMKKYTEITATYFQGVRLDNCHSTPLHVAEYMLDAARNLQPNLYVVAELFTGSEDLDNVFVTRLGISSLIREAMSAYNSHEEGRLVYRYGGEPVGSFVQPCLRPLMPAIAHALFMDITHDNECPIVHRSAYDALPSTTIVSMACCASGSTRGYDELVPHQISVVSEERFYTKWNPEALPSNTGEVNFQSGIIAARCAISKLHQELGAKGFIQVYVDQVDEDIVAVTRHSPSIHQSVVAVTRTAFRNPKTSFYSKEVPQMCIPGKIEEVVLEARTIERNTKPYRKDENSINGTPDITVEIREHIQLNESKIVKQAGVATKGPNEYIQEIEFENLSPGSVIIFRVSLDPHAQVAVGILRNHLTQFSPHFKSGSLAVDNADPILKIPFASLAYRLTLAELNQILYRCESEEKEDGGGCYDIPNWSALKYAGLQGLMSVLAEIRPKNDLGHPFCNNLRSGDWMIDYVSNRLISRSGTIAEVGKWLQAMFFYLKQIPRYLIPCYFDAILIGAYTTLLDTAWKQMSSFVQNGSTFVKHLSLGSVQLCGVGKFPSLPILSPALMDVPYRLNEITKEKEQCCVSLAAGLPHFSSGIFRCWGRDTFIALRGILLITGRYVEARNIILAFAGTLRHGLIPNLLGEGIYARYNCRDAVWWWLQCIQDYCKMVPNGLDILKCPVSRMYPTDDSAPLPAGTLDQPLFEVIQEAMQKHMQGIQFRERNAGPQIDRNMKDEGFNITAGVDEETGFVYGGNRFNCGTWMDKMGESDRARNRGIPATPRDGSAVEIVGLSKSAVRWLLELSKKNIFPYHEVTVKRHGKAIKVSYDEWNRKIQDNFEKLFHVSEDPSDLNEKHPNLVHKRGIYKDSYGASSPWCDYQLRPNFTIAMVVAPELFTTEKAWKALEIAEKKLLGPLGMKTLDPDDMVYCGIYDNALDNDNYNLAKGFNYHQGPEWLWPIGYFLRAKLYFSRLMGPETTAKTIVLVKNVLSRHYVHLERSPWKGLPELTNENAQYCPFSCETQAWSIATILETLYDL

SEQ ID NO: 2 - protein, 1376 aa, artificial
  D1 hGDE
MIHFTPLQTLGLSRSCYSLANQLELNPDFSRPNRKYTWNDVGQLVEKLKKEWNVICITDVVYNHTAANSKWIQEHPECAYNLVNSPHLKPAWVLDRALWRFSCDVAEGKYKEKGIPALIENDHHMNSIRKIIWEDIFPKLKLWEFFQVDVNKAVEQFRRLLTQENRRVTKSDPNQHLTIIQDPEYRRFGCTVDMNIALTTFIPHDKGPAAIEECCNWFHKRMEELNSEKHRLINYHQEQAVNCLLGNVFYERLAGHGPKLGPVTRKHPLVTRYFTFPFEEIDFSMEESMIHLPNKACFLMAHNGWVMGDDPLRNFAEPGSEVYLRRELICWGDSVKLRYGNKPEDCPYLWAHMKKYTEITATYFQGVRLDNCHSTPLHVAEYMLDAARNLQPNLYVVAELFTGSEDLDNVFVTRLGISSLIREAMSAYNSHEEGRLVYRYGGEPVGSFVQPCLRPLMPAIAHALFMDITHDNECPIVHRSAYDALPSTTIVSMACCASGSTRGYDELVPHQISVVSEERFYTKWNPEALPSNTGEVNFQSGIIAARCAISKLHQELGAKGFIQVYVDQVDEDIVAVTRHSPSIHQSVVAVTRTAFRNPKTSFYSKEVPQMCIPGKIEEVVLEARTIERNTKPYRKDENSINGTPDITVEIREHIQLNESKIVKQAGVATKGPNEYIQEIEFENLSPGSVIIFRVSLDPHAQVAVGILRNHLTQFSPHFKSGSLAVDNADPILKIPFASLAYRLTLAELNQILYRCESEEKEDGGGCYDIPNWSALKYAGLQGLMSVLAEIRPKNDLGHPFCNNLRSGDWMIDYVSNRLISRSGTIAEVGKWLQAMFFYLKQIPRYLIPCYFDAILIGAYTTLLDTAWKQMSSFVQNGSTFVKHLSLGSVQLCGVGKFPSLPILSPALMDVPYRLNEITKEKEQCCVSLAAGLPHFSSGIFRCWGRDTFIALRGILLITGRYVEARNIILAFAGTLRHGLIPNLLGEGIYARYNCRDAVWWWLQCIQDYCKMVPNGLDILKCPVSRMYPTDDSAPLPAGTLDQPLFEVIQEAMQKHMQGIQFRERNAGPQIDRNMKDEGFNITAGVDEETGFVYGGNRFNCGTWMDKMGESDRARNRGIPATPRDGSAVEIVGLSKSAVRWLLELSKKNIFPYHEVTVKRHGKAIKVSYDEWNRKIQDNFEKLFHVSEDPSDLNEKHPNLVHKRGIYKDSYGASSPWCDYQLRPNFTIAMVVAPELFTTEKAWKALEIAEKKLLGPLGMKTLDPDDMVYCGIYDNALDNDNYNLAKGFNYHQGPEWLWPIGYFLRAKLYFSRLMGPETTAKTIVLVKNVLSRHYVHLERSPWKGLPELTNENAQYCPFSCETQAWSIATILETLYDL

SEQ ID NO: 3 - protein, 1464 aa, artificial
  D2 hGDE
MGHSKQIRILLLNEMEKLEKTLFRLEQGYELQFRLGPTLQGKAVTVYTNYPFPGETFNREKFRSLDWENPTEREDDSDKYCKLNLQQSGSFQYYFLQGNEKSGGGYIVVDPILRVGADNHVLPLDCVTLQTFLAKCLGPFDEWESRLRVAKESGYNMIHFTPLQTLGLSRSCYSLANQLELNPDFSRPNRKYTWNDVGQLVEKLKKEWNVICITDVVYNHTAANSKWIQEHPECAYNLVNSPHLKPAWVLDRALWRFSCDVAEGKYKEKGIPALIENDHHMNSIRKIIWEDIFPKLKLWEFFQVDVNKAVEQFRRLLTQENRRVTKSDPNQHLTIIQDPEYRRFGCTVDMNIALTTFIPHYFTFPFEEIDFSMEESMIHLPNKACFLMAHNGWVMGDDPLRNFAEPGSEVYLRRELICWGDSVKLRYGNKPEDCPYLWAHMKKYTEITATYFQGVRLDNCHSTPLHVAEYMLDAARNLQPNLYVVAELFTGSEDLDNVFVTRLGISSLIREAMSAYNSHEEGRLVYRYGGEPVGSFVQPCLRPLMPAIAHALFMDITHDNECPIVHRSAYDALPSTTIVSMACCASGSTRGYDELVPHQISVVSEERFYTKWNPEALPSNTGEVNFQSGIIAARCAISKLHQELGAKGFIQVYVDQVDEDIVAVTRHSPSIHQSVVAVTRTAFRNPKTSFYSKEVPQMCIPGKIEEVVLEARTIERNTKPYRKDENSINGTPDITVEIREHIQLNESKIVKQAGVATKGPNEYIQEIEFENLSPGSVIIFRVSLDPHAQVAVGILRNHLTQFSPHFKSGSLAVDNADPILKIPFASLAYRLTLAELNQILYRCESEEKEDGGGCYDIPNWSALKYAGLQGLMSVLAEIRPKNDLGHPFCNNLRSGDWMIDYVSNRLISRSGTIAEVGKWLQAMFFYLKQIPRYLIPCYFDAILIGAYTTLLDTAWKQMSSFVQNGSTFVKHLSLGSVQLCGVGKFPSLPILSPALMDVPYRLNEITKEKEQCCVSLAAGLPHFSSGIFRCWGRDTFIALRGILLITGRYVEARNIILAFAGTLRHGLIPNLLGEGIYARYNCRDAVWWWLQCIQDYCKMVPNGLDILKCPVSRMYPTDDSAPLPAGTLDQPLFEVIQEAMQKHMQGIQFRERNAGPQIDRNMKDEGFNITAGVDEETGFVYGGNRFNCGTWMDKMGESDRARNRGIPATPRDGSAVEIVGLSKSAVRWLLELSKKNIFPYHEVTVKRHGKAIKVSYDEWNRKIQDNFEKLFHVSEDPSDLNEKHPNLVHKRGIYKDSYGASSPWCDYQLRPNFTIAMVVAPELFTTEKAWKALEIAEKKLLGPLGMKTLDPDDMVYCGIYDNALDNDNYNLAKGFNYHQGPEWLWPIGYFLRAKLYFSRLMGPETTAKTIVLVKNVLSRHYVHLERSPWKGLPELTNENAQYCPFSCETQAWSIATILETLYDL

SEQ ID NO: 4 - protein, 1430 aa, artificial
  D3 hGDE
MGHSKQIRILLLNEMEKLEKTLFRLEQGYELQFRLGPTLQGKAVTVYTNYPFPGETFNREKFRSLDWENPTEREDDSDKYCKLNLQQSGSFQYYFLQGNEKSGGGYIVVDPILRVGADNHVLPLDCVTLQTFLAKCLGPFDEWESRLRVAKESGYNMIHFTPLQTLGLSRSCYSLANQLELNPDFSRPNRKYTWNDVGQLVEKLKKEWNVICITDVVYNHTAANSKWIQEHPECAYNLVNSPHLKPAWVLDRALWRFSCDVAEGKYKEKGIPALIENDHHMNSIRKIIWEDIFPKLKLWEFFQVDVNKAVEQFRRLLTQENRRVTKSDPNQHLTIIQDPEYRRFGCTVDMNIALTTFIPHDKGPAAIEECCNWFHKRMEELNSEKHRLINYHQEQAVNCLLGNVFYERLAGHGPKLGPVTRKHPLVTRYFTFPFEEIDFSMEESMIHLPNKACFLMAHNGWVMGDDPLRNFAEPGSEVYLRRELICWGDSVKLRYGNKPEDCPYLWAHMKKYTEITATYFQGVRLDNCHSTPLHVAEYMLDAARNLQPNLYVVAELFTGSEDLDNVFVTRLGISSLIREAMSAYNSHEEGRLVYRYGGEPVGSFVQPCLRPLMPAIAHALFMDITHDNECPIVHRSAYDALPSTTIVSMACCASGSTRGYDELVPHQGKIEEVVLEARTIERNTKPYRKDENSINGTPDITVEIREHIQLNESKIVKQAGVATKGPNEYIQEIEFENLSPGSVIIFRVSLDPHAQVAVGILRNHLTQFSPHFKSGSLAVDNADPILKIPFASLAYRLTLAELNQILYRCESEEKEDGGGCYDIPNWSALKYAGLQGLMSVLAEIRPKNDLGHPFCNNLRSGDWMIDYVSNRLISRSGTIAEVGKWLQAMFFYLKQIPRYLIPCYFDAILIGAYTTLLDTAWKQMSSFVQNGSTFVKHLSLGSVQLCGVGKFPSLPILSPALMDVPYRLNEITKEKEQCCVSLAAGLPHFSSGIFRCWGRDTFIALRGILLITGRYVEARNIILAFAGTLRHGLIPNLLGEGIYARYNCRDAVWWWLQCIQDYCKMVPNGLDILKCPVSRMYPTDDSAPLPAGTLDQPLFEVIQEAMQKHMQGIQFRERNAGPQIDRNMKDEGFNITAGVDEETGFVYGGNRFNCGTWMDKMGESDRARNRGIPATPRDGSAVEIVGLSKSAVRWLLELSKKNIFPYHEVTVKRHGKAIKVSYDEWNRKIQDNFEKLFHVSEDPSDLNEKHPNLVHKRGIYKDSYGASSPWCDYQLRPNFTIAMVVAPELFTTEKAWKALEIAEKKLLGPLGMKTLDPDDMVYCGIYDNALDNDNYNLAKGFNYHQGPEWLWPIGYFLRAKLYFSRLMGPETTAKTIVLVKNVLSRHYVHLERSPWKGLPELTNENAQYCPFSCETQAWSIATILETLYDL

SEQ ID NO: 5 - protein, 1362 aa, artificial
  D2,3 hGDE
MGHSKQIRILLLNEMEKLEKTLFRLEQGYELQFRLGPTLQGKAVTVYTNYPFPGETFNREKFRSLDWENPTEREDDSDKYCKLNLQQSGSFQYYFLQGNEKSGGGYIVVDPILRVGADNHVLPLDCVTLQTFLAKCLGPFDEWESRLRVAKESGYNMIHFTPLQTLGLSRSCYSLANQLELNPDFSRPNRKYTWNDVGQLVEKLKKEWNVICITDVVYNHTAANSKWIQEHPECAYNLVNSPHLKPAWVLDRALWRFSCDVAEGKYKEKGIPALIENDHHMNSIRKIIWEDIFPKLKLWEFFQVDVNKAVEQFRRLLTQENRRVTKSDPNQHLTIIQDPEYRRFGCTVDMNIALTTFIPHYFTFPFEEIDFSMEESMIHLPNKACFLMAHNGWVMGDDPLRNFAEPGSEVYLRRELICWGDSVKLRYGNKPEDCPYLWAHMKKYTEITATYFQGVRLDNCHSTPLHVAEYMLDAARNLQPNLYVVAELFTGSEDLDNVFVTRLGISSLIREAMSAYNSHEEGRLVYRYGGEPVGSFVQPCLRPLMPAIAHALFMDITHDNECPIVHRSAYDALPSTTIVSMACCASGSTRGYDELVPHQGKIEEVVLEARTIERNTKPYRKDENSINGTPDITVEIREHIQLNESKIVKQAGVATKGPNEYIQEIEFENLSPGSVIIFRVSLDPHAQVAVGILRNHLTQFSPHFKSGSLAVDNADPILKIPFASLAYRLTLAELNQILYRCESEEKEDGGGCYDIPNWSALKYAGLQGLMSVLAEIRPKNDLGHPFCNNLRSGDWMIDYVSNRLISRSGTIAEVGKWLQAMFFYLKQIPRYLIPCYFDAILIGAYTTLLDTAWKQMSSFVQNGSTFVKHLSLGSVQLCGVGKFPSLPILSPALMDVPYRLNEITKEKEQCCVSLAAGLPHFSSGIFRCWGRDTFIALRGILLITGRYVEARNIILAFAGTLRHGLIPNLLGEGIYARYNCRDAVWWWLQCIQDYCKMVPNGLDILKCPVSRMYPTDDSAPLPAGTLDQPLFEVIQEAMQKHMQGIQFRERNAGPQIDRNMKDEGFNITAGVDEETGFVYGGNRFNCGTWMDKMGESDRARNRGIPATPRDGSAVEIVGLSKSAVRWLLELSKKNIFPYHEVTVKRHGKAIKVSYDEWNRKIQDNFEKLFHVSEDPSDLNEKHPNLVHKRGIYKDSYGASSPWCDYQLRPNFTIAMVVAPELFTTEKAWKALEIAEKKLLGPLGMKTLDPDDMVYCGIYDNALDNDNYNLAKGFNYHQGPEWLWPIGYFLRAKLYFSRLMGPETTAKTIVLVKNVLSRHYVHLERSPWKGLPELTNENAQYCPFSCETQAWSIATILETLYDL

SEQ ID NO: 6 - protein, 1339 aa, artificial
  D4 hGDE
MGHSKQIRILLLNEMEKLEKTLFRLEQGYELQFRLGPTLQGKAVTVYTNYPFPGETFNREKFRSLDWENPTEREDDSDKYCKLNLQQSGSFQYYFLQGNEKSGGGYIVVDPILRVGADNHVLPLDCVTLQTFLAKCLGPFDEWESRLRVAKESGYNMIHFTPLQTLGLSRSCYSLANQLELNPDFSRPNRKYTWNDVGQLVEKLKKEWNVICITDVVYNHTAANSKWIQEHPECAYNLVNSPHLKPAWVLDRALWRFSCDVAEGKYKEKGIPALIENDHHMNSIRKIIWEDIFPKLKLWEFFQVDVNKAVEQFRRLLTQENRRVTKSDPNQHLTIIQDPEYRRFGCTVDMNIALTTFIPHDKGPAAIEECCNWFHKRMEELNSEKHRLINYHQEQAVNCLLGNVFYERLAGHGPKLGPVTRKHPLVTRYFTFPFEEIDFSMEESMIHLPNKACFLMAHNGWVMGDDPLRNFAEPGSEVYLRRELICWGDSVKLRYGNKPEDCPYLWAHMKKYTEITATYFQGVRLDNCHSTPLHVAEYMLDAARNLQPNLYVVAELFTGSEDLDNVFVTRLGISSLIREAMSAYNSHEEGRLVYRYGGEPVGSFVQPCLRPLMPAIAHALFMDITHDNECPIVHRSAYDALPSTTIVSMACCASGSTRGYDELVPHQISVVSEERFYTKWNPEALPSNTGEVNFQSGIIAARCAISKLHQELGAKGFIQVYVDQVDEDIVAVTRHSPSIHQSVVAVTRTAFRNPKTSFYSKEVPQMCIPGKIEEVVLEARTIERNTKPYRKDENSINGTPDITVEIREHIQLNESKIVKQAGVATKGPNEYIQEIEFENLSPGSVIIFRVSLDPHAQVAVGILRNHLTQFSPHFKSGSLAVDNADPILKIPFASLPHFSSGIFRCWGRDTFIALRGILLITGRYVEARNIILAFAGTLRHGLIPNLLGEGIYARYNCRDAVWWWLQCIQDYCKMVPNGLDILKCPVSRMYPTDDSAPLPAGTLDQPLFEVIQEAMQKHMQGIQFRERNAGPQIDRNMKDEGFNITAGVDEETGFVYGGNRFNCGTWMDKMGESDRARNRGIPATPRDGSAVEIVGLSKSAVRWLLELSKKNIFPYHEVTVKRHGKAIKVSYDEWNRKIQDNFEKLFHVSEDPSDLNEKHPNLVHKRGIYKDSYGASSPWCDYQLRPNFTIAMVVAPELFTTEKAWKALEIAEKKLLGPLGMKTLDPDDMVYCGIYDNALDNDNYNLAKGFNYHQGPEWLWPIGYFLRAKLYFSRLMGPETTAKTIVLVKNVLSRHYVHLERSPWKGLPELTNENAQYCPFSCETQAWSIATILETLYDL

SEQ ID NO: 7 - protein, 1313 aa, artificial
  D5 hGDE
MGHSKQIRILLLNEMEKLEKTLFRLEQGYELQFRLGPTLQGKAVTVYTNYPFPGETFNREKFRSLDWENPTEREDDSDKYCKLNLQQSGSFQYYFLQGNEKSGGGYIVVDPILRVGADNHVLPLDCVTLQTFLAKCLGPFDEWESRLRVAKESGYNMIHFTPLQTLGLSRSCYSLANQLELNPDFSRPNRKYTWNDVGQLVEKLKKEWNVICITDVVYNHTANRRVTKSDPNQHLTIIQDPEYRRFGCTVDMNIALTTFIPYFTFPFEEIDFSMEESMIHLPNKACFLMAHNGWVMGDDPLRNFAEPGSEVYLRRELICWGDSVKLRYGNKPEDCPYLWAHMKKYTEITATYFQGVRLDNCHSTPLHVAEYMLDAARNLQPNLYVVAELFTGSEDLDNVFVTRLGISSLIREAMSAYNSHEEGRLVYRYGGEPVGSFVQPCLRPLMPAIAHALFMDITHDNECPIVHRSAYDALPSTTIVSMACCASGSTRGYDELVPHQIYVDQVDEDIVAVTRHSPSIHQSVVAVTRTAFRNPKTSFYSKEVPQMCIPGKIEEVVLEARTIERNTKPYRKDENSINGTPDITVEIREHIQLNESKIVKQAGVATKGPNEYIQEIEFENLSPGSVIIFRVSLDPHAQVAVGILRNHLTQFSPHFKSGSLAVDNADPILKIPFASLAYRLTLAELNQILYRCESEEKEDGGGCYDIPNWSALKYAGLQGLMSVLAEIRPKNDLGHPFCNNLRSGDWMIDYVSNRLISRSGTIAEVGKWLQAMFFYLKQIPRYLIPCYFDAILIGAYTTLLDTAWKQMSSFVQNGSTFVKHLSLGSVQLCGVGKFPSLPILSPALMDVPYRLNEITKEKEQCCVSLAAGLPHFSSGIFRCWGRDTFIALRGILLITGRYVEARNIILAFAGTLRHGLIPNLLGEGIYARYNCRDAVWWWLQCIQDYCKMVPNGLDILKCPVSRMYPTDDSAPLPAGTLDQPLFEVIQEAMQKHMQGIQFRERNAGPQIDRNMKDEGFNITAGVDEETGFVYGGNRFNCGTWMDKMGESDRARNRGIPATPRDGSAVEIVGLSKSAVRWLLELSKKNIFPYHEVTVKRHGKAIKVSYDEWNRKIQDNFEKLFHVSEDPSDLNEKHPNLVHKRGIYKDSYGASSPWCDYQLRPNFTIAMVVAPELFTTEKAWKALEIAEKKLLGPLGMKTLDPDDMVYCGIYDNALDNDNYNLAKGFNYHQGPEWLWPIGYFLRAKLYFSRLMGPETTAKTIVLVKNVLSRHYVHLERSPWKGLPELTNENAQYCPFSCETQAWSIATILETLYDL

SEQ ID NO: 8 - protein, 1252 aa, artificial
  D6 hGDE
MNSIRKIIWEDIFPKLKLWEFFQVDVNKAVEQFRRLLTQENRRVTKSDPNQHLTIIQDPEYRRFGCTVDMNIALTTFIPHDKGPAAIEECCNWFHKRMEELNSEKHRLINYHQEQAVNCLLGNVFYERLAGHGPKLGPVTRKHPLVTRYFTFPFEEIDFSMEESMIHLPNKACFLMAHNGWVMGDDPLRNFAEPGSEVYLRRELICWGDSVKLRYGNKPEDCPYLWAHMKKYTEITATYFQGVRLDNCHSTPLHVAEYMLDAARNLQPNLYVVAELFTGSEDLDNVFVTRLGISSLIREAMSAYNSHEEGRLVYRYGGEPVGSFVQPCLRPLMPAIAHALFMDITHDNECPIVHRSAYDALPSTTIVSMACCASGSTRGYDELVPHQISVVSEERFYTKWNPEALPSNTGEVNFQSGIIAARCAISKLHQELGAKGFIQVYVDQVDEDIVAVTRHSPSIHQSVVAVTRTAFRNPKTSFYSKEVPQMCIPGKIEEVVLEARTIERNTKPYRKDENSINGTPDITVEIREHIQLNESKIVKQAGVATKGPNEYIQEIEFENLSPGSVIIFRVSLDPHAQVAVGILRNHLTQFSPHFKSGSLAVDNADPILKIPFASLAYRLTLAELNQILYRCESEEKEDGGGCYDIPNWSALKYAGLQGLMSVLAEIRPKNDLGHPFCNNLRSGDWMIDYVSNRLISRSGTIAEVGKWLQAMFFYLKQIPRYLIPCYFDAILIGAYTTLLDTAWKQMSSFVQNGSTFVKHLSLGSVQLCGVGKFPSLPILSPALMDVPYRLNEITKEKEQCCVSLAAGLPHFSSGIFRCWGRDTFIALRGILLITGRYVEARNIILAFAGTLRHGLIPNLLGEGIYARYNCRDAVWWWLQCIQDYCKMVPNGLDILKCPVSRMYPTDDSAPLPAGTLDQPLFEVIQEAMQKHMQGIQFRERNAGPQIDRNMKDEGFNITAGVDEETGFVYGGNRFNCGTWMDKMGESDRARNRGIPATPRDGSAVEIVGLSKSAVRWLLELSKKNIFPYHEVTVKRHGKAIKVSYDEWNRKIQDNFEKLFHVSEDPSDLNEKHPNLVHKRGIYKDSYGASSPWCDYQLRPNFTIAMVVAPELFTTEKAWKALEIAEKKLLGPLGMKTLDPDDMVYCGIYDNALDNDNYNLAKGFNYHQGPEWLWPIGYFLRAKLYFSRLMGPETTAKTIVLVKNVLSRHYVHLERSPWKGLPELTNENAQYCPFSCETQAWSIATILETLYDL

SEQ ID NO: 9 - protein, 1108 aa, artificial
  D7 hGDE
MVTRYFTFPFEEIDFSMEESMIHLPNKACFLMAHNGWVMGDDPLRNFAEPGSEVYLRRELICWGDSVKLRYGNKPEDCPYLWAHMKKYTEITATYFQGVRLDNCHSTPLHVAEYMLDAARNLQPNLYVVAELFTGSEDLDNVFVTRLGISSLIREAMSAYNSHEEGRLVYRYGGEPVGSFVQPCLRPLMPAIAHALFMDITHDNECPIVHRSAYDALPSTTIVSMACCASGSTRGYDELVPHQISVVSEERFYTKWNPEALPSNTGEVNFQSGIIAARCAISKLHQELGAKGFIQVYVDQVDEDIVAVTRHSPSIHQSVVAVTRTAFRNPKTSFYSKEVPQMCIPGKIEEVVLEARTIERNTKPYRKDENSINGTPDITVEIREHIQLNESKIVKQAGVATKGPNEYIQEIEFENLSPGSVIIFRVSLDPHAQVAVGILRNHLTQFSPHFKSGSLAVDNADPILKIPFASLAYRLTLAELNQILYRCESEEKEDGGGCYDIPNWSALKYAGLQGLMSVLAEIRPKNDLGHPFCNNLRSGDWMIDYVSNRLISRSGTIAEVGKWLQAMFFYLKQIPRYLIPCYFDAILIGAYTTLLDTAWKQMSSFVQNGSTFVKHLSLGSVQLCGVGKFPSLPILSPALMDVPYRLNEITKEKEQCCVSLAAGLPHFSSGIFRCWGRDTFIALRGILLITGRYVEARNIILAFAGTLRHGLIPNLLGEGIYARYNCRDAVWWWLQCIQDYCKMVPNGLDILKCPVSRMYPTDDSAPLPAGTLDQPLFEVIQEAMQKHMQGIQFRERNAGPQIDRNMKDEGFNITAGVDEETGFVYGGNRFNCGTWMDKMGESDRARNRGIPATPRDGSAVEIVGLSKSAVRWLLELSKKNIFPYHEVTVKRHGKAIKVSYDEWNRKIQDNFEKLFHVSEDPSDLNEKHPNLVHKRGIYKDSYGASSPWCDYQLRPNFTIAMVVAPELFTTEKAWKALEIAEKKLLGPLGMKTLDPDDMVYCGIYDNALDNDNYNLAKGFNYHQGPEWLWPIGYFLRAKLYFSRLMGPETTAKTIVLVKNVLSRHYVHLERSPWKGLPELTNENAQYCPFSCETQAWSIATILETLYDL

SEQ ID NO: 10 - protein, 1303 aa, artificial
  D8 hGDE
MHPECAYNLVNSPHLKPAWVLDRALWRFSCDVAEGKYKEKGIPALIENDHHMNSIRKIIWEDIFPKLKLWEFFQVDVNKAVEQFRRLLTQENRRVTKSDPNQHLTIIQDPEYRRFGCTVDMNIALTTFIPHDKGPAAIEECCNWFHKRMEELNSEKHRLINYHQEQAVNCLLGNVFYERLAGHGPKLGPVTRKHPLVTRYFTFPFEEIDFSMEESMIHLPNKACFLMAHNGWVMGDDPLRNFAEPGSEVYLRRELICWGDSVKLRYGNKPEDCPYLWAHMKKYTEITATYFQGVRLDNCHSTPLHVAEYMLDAARNLQPNLYVVAELFTGSEDLDNVFVTRLGISSLIREAMSAYNSHEEGRLVYRYGGEPVGSFVQPCLRPLMPAIAHALFMDITHDNECPIVHRSAYDALPSTTIVSMACCASGSTRGYDELVPHQISVVSEERFYTKWNPEALPSNTGEVNFQSGIIAARCAISKLHQELGAKGFIQVYVDQVDEDIVAVTRHSPSIHQSVVAVTRTAFRNPKTSFYSKEVPQMCIPGKIEEVVLEARTIERNTKPYRKDENSINGTPDITVEIREHIQLNESKIVKQAGVATKGPNEYIQEIEFENLSPGSVIIFRVSLDPHAQVAVGILRNHLTQFSPHFKSGSLAVDNADPILKIPFASLAYRLTLAELNQILYRCESEEKEDGGGCYDIPNWSALKYAGLQGLMSVLAEIRPKNDLGHPFCNNLRSGDWMIDYVSNRLISRSGTIAEVGKWLQAMFFYLKQIPRYLIPCYFDAILIGAYTTLLDTAWKQMSSFVQNGSTFVKHLSLGSVQLCGVGKFPSLPILSPALMDVPYRLNEITKEKEQCCVSLAAGLPHFSSGIFRCWGRDTFIALRGILLITGRYVEARNIILAFAGTLRHGLIPNLLGEGIYARYNCRDAVWWWLQCIQDYCKMVPNGLDILKCPVSRMYPTDDSAPLPAGTLDQPLFEVIQEAMQKHMQGIQFRERNAGPQIDRNMKDEGFNITAGVDEETGFVYGGNRFNCGTWMDKMGESDRARNRGIPATPRDGSAVEIVGLSKSAVRWLLELSKKNIFPYHEVTVKRHGKAIKVSYDEWNRKIQDNFEKLFHVSEDPSDLNEKHPNLVHKRGIYKDSYGASSPWCDYQLRPNFTIAMVVAPELFTTEKAWKALEIAEKKLLGPLGMKTLDPDDMVYCGIYDNALDNDNYNLAKGFNYHQGPEWLWPIGYFLRAKLYFSRLMGPETTAKTIVLVKNVLSRHYVHLERSPWKGLPELTNENAQYCPFSCETQAWSIATILETLYDL

SEQ ID NO: 11 - protein, 1377 aa, Equus caballus
MIHFTPLQTLGLSRSSYSLADQLELNPDFSRPNKKYTWHDVGQLVEKLKKEWDILCITDVVYNHTAANSKWIHEHPESAYNLVNSPHLKPAWVLDRALWHLSCDVAEGKYREKGVPALIENDHQMNCIRKIIWEDIYPKIHLWEFFQVDVHKAVEQFRGLLTQENRKIISQPDPKQHLKIIQDPEYRRLGCTVDMNIALATFIPHDNGPAAIDECCNWFRKRIEELNAEKHQLVNYHQEQAVNCLLGNVFYERLAGHGPKLGPVTRKHPLVTRYFTFPFEEMTPSTEESMIHLPNKACFLMAHNGWVMGDDPLRNFAEPGSDVYLRRELICWGDSVKLRYGNKPEDCPYLWAHMKKYTEITATHFQGVRLDNCHSTPIHVAEYMLDAARKLQPNLYVVAELFTGSEDLDNIFVTRLGISSLIREAMSAADSHEEGRLVYRYGGEPVGSFVQPCLRPLMPAIAHALFMDITHDNECPIVHRSAYDALPSSTIVSMASCASGSTKGYDELVPHQISVVSEERFYTKWNPEALPSNTGEVNFQSGIIAARRAINKLHQELGAKGFIQVYVDQVDQDIVAVTRHSPSIHQSVVSVSRTAFRNPKTSFYSKEVPHMYIPGKIEEVVLEARTIERHTIPYKKDENSINGMPDITVEIREHIQLNESKIVKHAGIVTKGPNEFVQEIEFENLTPGSVIIFRVSLDPHAQVAVGILRNHLTQFSPHFKSGSLAVDNADPILKIPFASIASKLTLAELNQVLYRCESEEQEDGGGCYNIPNWSSLKYAGLQGLMSILAEIRPRNDLGHPFCDNLRSGDWMIDYVSSRLISRSGTIAEVGKWLQAMFLYLKQIPRYLIPCYFDAILIGAYTTLLDIAWKQMSSFVQNGSTFVKHLSLGSVQMCGVGKFPSLPLLSPSLTDLPYRVNEITKEKEQCCGSLAAGLPHFSAGIFRCWGRDTFIALRGLLLVTGRYLEARNIILAFAGTLRHGLIPNLLGEGTHARYNCRDAVWWWLQCIQDYCKIVPNGLDILRCPVSRMYPTDDSVPLSAGTVDQPLFEVIQEAMQRHVQGIQFRERNAGPQIDRNMKDEGFNITAGVDEETGFVYGGNRFNCGTWMDKMGESDRARNRGIPATPRDGSAVEIVGLSKSAVRWLLELSRKNIFPYHEVRVKRHGKFVTVSYDEWNRKIQDNFEKLFHVSEDPSDFNEKHPELVHKRGIYKDSYGASSPWCDYQLRPNFTIAMVVAPELFTPEKAWKALEIAEKKLLGPLGMKTLDPDDMVYCGIYDNALDNDNYNLAKGFNYHQGPEWLWPTGYFLRAKLYFSKLMGPETNAKTMFLVKNVLSRHYVHLERSPWKGLPELTNENGQYCPFSCETQAWSIATVLETLYDL

SEQ ID NO: 12 - protein, 1365 aa, Gorilla gorilla
MGHSKQIRILLLNEMEKLEKTLFRLEQGYELQFRLGPTLQGKAVTVYTNYPFPGETFNREKFRSLDWENPTEREDDSDKYCKLNLQQSGSFQYYFLQGNEKSGGGYIVVDPILRVGADNHVLPLDCVTLQTFLAKCLGPFDEWESRLRVAKESGYNMIHFTPLQTLGLSRSCYSLANQLELNPDFSRPNRKYTWNDVGQLVEKLKKEWNVICITDVVYNHTAANSKWIQEHPECAYNLVNSPHLKPAWVLDRALWRFSCDVAEGKYKEKGIPALIENDHHMNSIRKIIWEDIFPKLKLWEFFQVDVNKAVEQFRRLLTQENRRVTKSDPNQHLTIIQDPEYRRFGCTVDMNIALTTFIPHEYFTFPFEEIDFSMEESMIHLPNKACFLMAHNGWVMGDDPLRNFAEPGSEVYLRRELICWGDSVKLRYGNKPEDCPYLWAHMKKYTEITATYFQGVRLDNCHSTPLHVAEYMLDAARNLQPNLYVVAELFTGSEDLDNVFVTRLGISSLIREAMSAYNSHEEGRLVYRYGGEPVGSFVQPCLRPLMPAIAHALFMDITHDNECPIVHRSAYDALPSTTIVSMACCASGSTRGYDELVPHQFLGKIEEVVLEARTIERNMKPYRKDENSINGTPDITVEIREHIQLNESKIVKQAGVATKGPNEYIQEIEFENLSPGSVIIFRVSLDPHAQVAVGILRNHLTQFSPHFKSGSLAVDNADPILKIPFASIASRLTLAELNQILYRCESEEKEDGGGCYDIPNWSALKYAGLQGLMSVLAEIRPKNDLGHPFCNNLRSGDWMIDYVSNRLISRSGTIAEVGKWLQAMFFYLKQIPRYLIPCYFDAILIGAYTTLLDTAWKQMSSFVQNGSTFVKHLSLGSVQLCGVGKFPSLPILSPALMDVPYRLNEITKEKEQCCVSLAAGLPHFSSGIFRCWGRDTFIALRGILLITGRYVEARNIILAFAGTLRHGLIPNLLGEGIYARYNCRDAVWWWLQCIQDYCKMVPNGVDILKCPVSRMYPTDDSAPLPAGTLDQPLFEVIQEAMQKHMQGIQFRERNAGPQIDRNMKDEGFNITAGVDEETGFVYGGNRFNCGTWMDKMGESDRARNRGIPATPRDGSAVEIVGLSKSAVRWLLELSKKNIFPYHEVTVKRHGKAIKVSYDEWNRKIQDNFEKLFHVSEDPSDLNEKHPNLVHKRGIYKDSYGASSPWCDYQLRPNFTIAMVVAPELFTTEKAWKALEIAEKKLLGPLGMKTLDPDDMVYCGIYDNALDNDNYNLAKGFNYHQGPEWLWPIGYFLRAKLYFSRLMGPETTAKTIVLVKNVLSRHYVHLERSPWKGLPELTNENAQYCPFSCETQAWSIATILETLYDL

SEQ ID NO: 13 - protein, 1299 aa, Pongo abelii
MGHSKQIRILLLNEMEKLEKTLFRLEQGYELQFRLGPTLQGKAVTVYTNYPFPGETFNREKFRSLDWENPTEREDDSDKYCKLNLQQSGSFQYYFLQGNEKSGGGYIVVDPILRVGADNHVLPLDCVTLQTFLAKCLGPFDEWESRLRVAKESGYNMIHFTPLQTLGLSRSCYSLANQLELNPDFSRPNRKYTWNDVGQLVEKLKKEWNVICITDVVYNHTAANSKWIQEHPECAYNLVNSPHLKPAWVLDRALWRFSCDVAEGKYKEKGIPALIENDHHMNSIRKIIWEDIFPKLKLWEFFEVDVNKAVEQFRRLLTQENRRVTKSDPNQHLTIIQDPEYRRFGCTVDMNIALTTFIPHDNGPAAIEECCNWFRKRIEELNSEKHQLINYHQEQAVNCLLGNVFYERLAGHGPKLGPVTRKHPLVTRYFTFPFEEMDFSMEESMIHLPNKACLLMAHNGWVMGDDPLRNFAEPGSEVYLRRELICWGDSVKLRYGNKPEDCPYLWAHMKKYTEITATYFQGVRLDNCHSTPLHVAEYMLDAARNLQPNLYVVAELFTGSEDLDNVFVTRLGISSLIREAMSAYDSHEEGRLVYRYGGEPVGSFVQPCLRPLMPAIAHALFMDITHDNECPIVHRSAYDALPSTTIVSMACCASGSTRGYDELVPHQISVVSEERFYTKWNPEALPSNTGEVNFQSGIIAARCAINKLHQELGAKGFIQVYVDQVDEDIVAVTRHSPSIHQSVVAVSRTAFRNPKTSFYSKEVPQMCIPGKIEEVVLEARTIERNTKPYRKDENSINGTPDITVEIREHIQLNESKIVKQAGVATKGPNEFIQEIEFENLSPGSVIIFRVSLDPHAQVAVGILRNHLTQFSPHFKSGSLAVDNADPILKIPFALPHFSSGIFRCWGRDTFIALRGMLLITGRYVEARNIILAFAGTLRHGLIPNLLGEGTYARYNCRDAVWWWLQCIQDYCKVVPNGLDILKCPVSRMYPTDDSAPLPAGALFNITAGVDEETGFVYGGNRFNCGTWMDKMGESDRARNRGIPATPRDGSAVEIVGLSKSAVRWLLELSKKNIFPYHEVTVKHGKAIKVSYDEWNRKIQDNFEKLFHVSEDPSDLNEKHPNLVHKRGIYKDSYGASSPWCDYQLRPNFTIAMVVAPELFTTEKAWKALEIAEKKLLGPLGMKTLDPDDMVYCGIYDNALDNDNYNLAKGFNYHQGPEWLWPIGYFLRAKLYFSRLMGPETTAKTIVLVKNVLSRHYVHLERSPWKGLPELTNENAQYCPFSCETQAWSVATILETLYDL

SEQ ID NO: 14 - protein, 1390 aa, Pteropus alecto
MGHGKQIRILLLNEMEKLEKTLFRLEQGFELQFRLGPTLQGKTVTVHTNYPYPGETFNREKFRSLEWENPSEREDDSDKYCKLNLQQAGSFQYYFLRGNEKSGGGYIVVDPVLRVGTDNHVLPLDCVTLQTFLAKCLGPLDEWESRLRVAKESGYNMIHFTPLQTLGQSRSCYSLADQLELNPDFSRPNKKCTWDDVGQLVEKLKKEWNILCITDVVYNHTGNRKITKPDPKEHLKIIQDPEYRRLGCTVDMNIALATFIPNEYFTFPFEEMTLSTEESMIHLPNKACFLMAHNGWVMGDDPLRNFAEPGSDVYLRRELICWGDSVKLRYGNKPEDCPYLWAHMKKYTEITATYFQGVRLDNCHSTPLHVAEYMLDAARKLQPNLYIVAELFTGSEDLDNVFVTRLGISSLIREAMSAHDSHEEGRLVYRYGGEPVGSFVQPCLRPLMPAIAHALFMDITHDNECPIVHRSAYDALPSSMIVSMACCASGSTKGYDELVPHQVYVDQVDEDIVAVTRHSPSIHQSVVAVSRTAFKNPKTSFYSKEVPQMCIPGKIEEVVLEARTIERNTKPYKRDENSINGMPDITAEIREHIQLNESKIVKQAGIATKGPNEYIQEIEFENLSPGSVIVFRVSLDPHAQVAVGILRNHLTQFSPHFKSGSLSADSSDPILKIPFAYIASKLTLAELNQILYRCESEEQEDGGGCYNIPNWSSLKYAGLQENSSLELAPYVGFGGGCGAAPAGLNRGGGVRSDQASLERFLTTLLATVDYTALVSTSVCSPHITGHEQQPRLWERIASANNIACYFYDFSGLMSVLAEMRPKNDLGHPFCDNLRSGDWMIDYVSNRLISRSGTIAEVGRWLQAMFFYLKQIPRYLIPCYFDAVLIGAYTTLLDTAWKQMSSFVQNGSTFVKHLSLGSVQLCGVGKYASLPLLSPSLMDVPYRLNEITKEKEQCCVTLAAGLPHFSSGIFRCWGRDTFIALRGILLITGRYLEARNIILAFAGTLRHGLIPNLLGEGTYARYNCRDAVWWWLQCIQDYCKVVPNGLDILKCPVSRMYPTDDSVPLSAGTVDQPLFEVIQEAMQRHMQGIQFRERNAGPQIDRNMKDEGFNITVGVDEETGFVYGGNRFNCGTWMDKMGESDRARNRGIPATPRDGSAVEIVGLSKSAIRWLLELSKKNIFPYHEVTVKRDGKVVTVSYDEWNRKIQDNFEKLFYVSEDPSDFNEKNPNLVHKRGIYKDSYGASSPWCDYQLRPNFTIAMVVAPELFTTEKAWKALQVAEKKLLGPLGMKTLDPDDMVYCGVYDNALDNDNYNLAKGFNYHQGPEWLWLIGYFLRAKLYFSKLMGPETNAKTIFLVKNVLSRHYVHLESLACFALTTLLQLLNKILSASQIP

SEQ ID NO: 15 - protein, 1252 aa, Cercocebus atys
MNSIRKMIWEDIFPKLKLWEFFQVDVNKKKKKKKRLLTQENRRVTKSDPHQHLKIIQDPEYRRFGCTVDMNIALTTFIPHDNGPAAIEECCNWFRKRIEELNSEKHRLINYHQEQAVNCLLGNVFYERLAGHGPKLGPVTRKHPLVTRYFTFPFEEMDFSVEESMIHLPNKACFLMAHNGWVMGDDPLRNFAEPGSEVYLRRELICWGDSVKLRYGNKPEDCPFLWAHMKKYTEITATYFQGVRLDNCHSTPLHVAEYMLDAARNLQPNLYVVAELFTGSEDLDNIFVTRLGISSLIREAMSAYNSHEEGRLVYRYGGEPVGSFVQPCLRPLMPAIAHALFMDITHDNECPIVHRSAYDALPSTTIVSMACCASGSTRGYDELVPHQISVVSEERFYTKWNPGALPSNTGEVNFQSGIIAARCAINKLHQELGAKGFIQVYVDQVDEDIVAVTRHSPSIHQSVVAVSRTAFRNPKTSFYSKEVPQMCIPGKIEEVVLEARTIERNTKPYRKDENSINGMPDITVEIREHIQLNESKIVKQAGVATKGPNEYIQEIEFENLSPGSVIIFRVSLDPHAQVAVGILRNHLTQFSPHFKSGSLAVDNSDPILKIPFASIASKLTLAELNQILYRCESEEKEDGGGCYDIPNWSALKYAGLQGLMSVLAEIRPKNDLGHPFCNNLRSGDWMIDYVSNRLISRSGTIAEVGKWLQAMFFYLKQIPRYLIPCYFDAILIGAYTTLLDIAWKQMSSFVQNGSTFVKHLSLGSVQLCGVGKFPSLPILSPALTGVPYRLNEITKEKEQCCVSLAAGLPHFSSGIFRCWGRDTFIALRGILLITGRYVEARNIILAFAGTLRHGLIPNLLGEGTYARYNCRDAVWWWLQCIQDYCKMVPNGLDILKCPVSRMYPTDDSAPLPAGTLDQPLFEVIQEAMQRHMQGIQFRERNAGPKIDRNMKDEGFNVTAGVDEETGFVYGGNRFNCGTWMDKMGESDRARNTGIPATPRDGSAVEIVGLSKSAVRWLLELSKKNIFPYHEVTVKRHGKVVKVSYDEWNRKIQDNFEKLFHVSEDPSDLNEKHPNLVHKRGIYKDSYGASSPWCDYQLRPNFTIAMVVAPELFTTAKAWKALEIAEKKLLGPLGMKTLDPDDMVYCGIYDNALDNDNYNLAKGFNYHQGPEWLWPIGYFLRAKLYFSRLMGPETTAKTIVLVKNVLSRHYVHLERSPWKGLPELTNENAQYCPFSCETQAWSISTILETLYDL

SEQ ID NO: 16 - protein, 1116 aa, Ornithorhynchus anatinus
MFEGRAEGVVGEYFTFPYGEMTSVEEESLMHQPEKACFFMAHNGWVMGDDPLRNFAEPGSDVYLRRELVCWGDSVKLRYGNKPEDCPYLWAHMKKYTEITAKYFQGVRLDNCHSTPLHVAEYMLDAARKLQPNLYVVAELFTGSEELDNIFVTRLGISSLIREAMSAYNSHEEGRLVYRFGGEPVGSFVQPCLRPLMPAIAHALFMDITHDNECPIVHRSAYDALPSSTIVSMACCASGSTRGYDELVPHQISVVSEERFYTKWNPAATLSNPSEVNLQTGIIAGRRAINKLHQELGAKGFIQVYVDQVDEDIVAVTRHCPSSHQSVVAVSRTAFRNPKTSAYSKEVPQMCIPGKIEEVVLEARTVERNVGSYVKDAKSINGMPDITVEIREHIQLNESKIVKQAGVATKGLHEYVQEIEFENLTPGSVIIFRVSLDPHAQVAVGILRNHLTQFSPNFKIGSLPVDNSDPILKIPFASISSKLTLADLNQLLYRCESEEQEDGGGCYDVPNWSPLKYGGLQGLMSVMAEIRPKNDLGHPFCNNLRSGDWMIDYVSNRLISRSGSIAEVGKWFQAMFFYLKQIPRYLIPCYFDAILIGAYTTLLDIAWKQMSSFVQNGSTFVKHLSLGSVQMCGIGKFPSLPFLSPSLGDVPYRLNEITQEKEQCCVSLAAGLPHFSSGIFRCWGRDTFIALRGLLLITGRFLEARNIILAFAGTLRHGLIPNLLGQGTYARFNCRDAVWWWLQCIQDYCKIVPKGTDILKCPVSRMYPSDDSSALPAGTLDQPLYEVIQEAMQRHMQGIQFREKNAGPQIDRNMKDEGFNVTAGVDDESGFVYGGNHFNCGTWMDKMGESDRGRNRGIPATPRDGSAVEIVGLSKSTVRWLVELSKKNVFPYHGVTVKRNEKEVLITYDEWNRKIQDHFEKLFYVSEDPSDTNEKHPNLVHKRGIYKDSYGASSPWCDYQLRPNFTIAMVVAPELFTPQKAWKALEIAEKKLLGPLGMKTLDPDDMVYCGVYDNALDNDNYNLAKGFNYHQGPEWLWPVGYFLRAKLYFSKLMGQETYTKTVFLIKNVLSRHYVHLERSPWKGLPELTNENGQYCSFSCETQAWSIAVILETLYDL

SEQ ID NO: 17 - protein, 1304 aa, Anas platyrhynchos
MHPECGYNLVNSPHLKPAWVLDRALWHLTCMVADGKCIDKGVPPLIENDHHLNCVRKIIWEEIYPKIKLWEFFQVDVNKAVEQFRTLLTQGKESKMSTKSDPNQHLQIVQDPEYRRFGCTVDMNIALATFIPHSNGPGAIEECCNWFRKRIEELNAEQHRQIHHHQEQAVNCLAGTVVYERLAGHGPKLGPISRKYPLVTRYFTYPFKDMTVEEEEAMIHRPDKACYFMAHNGWVMGDDPLRNFAEPGSNVYLRRELICWGDSVKLRYGNKPEDCPYLWAHMKKYTEITAKYFHGVRLDNCHSTPIHVAEYMLDTARKLRADLFVVAELFTGNEELDNIFVNRLGITSLIREAMTAYNSHEEGRLVYRFGGEPVGSFVQPRLRPLMPAIAHALFMDITHDNECPIQHRSAYDALPSAMIVSMACCATGSTKGYDELVPHQISVVSEERFYSTWNPAAHLTSGEVNFQTGILAGRLAINRLHQELGAKGFNQVYVDQVDEDIVAVTRHCPNTHQSVVAVSRTAFRDPKTSFYSKEVPEMCIPGKIEEVVLEARTIERNTNPYKKDERFINGLPNFTVELREHIQIKDSKIIKQAGTAIKGPNEFVQEIEFENLTPGSVIVFRVSLDPKAQEAVGVLRSHLIQFSPHFKSGSLPDDHSAPILKTLFSSIASKLSLADLNQVLYRCEAEEQEDGGGCYNIPNWSPLKYAGLQGLMSVMADIRPKNDLGHPFCDNLRSGDWMIDYVSNRLISRTGACAEVGKWLKAMFIYLKKIPRYLIPCYFDAILVGAYTTLLDVGWHQMSSFVQNGSTFVKHLSLGSIQMCGIGKYSCLPDLSPSLHDVPYRLNEITNEKEQCCVSLAAGLPHFSSGIFRSWGRDTFIALRGLMLVTGRYLEARNIILAFGGTLRHGLIPNLLGQGTHARYNCRDAVWWWLQCIQDYCKIVPNGLDILRCPVSRMYPRDDSSPQPAGSVDQPLYEVIQEAMQRHMEGINFRERNAGPQIDQNMRDEGFNVTAGVDRETGFVFGGNRFNCGTWMDKMGESDRARNRGIPATPRDGSAVEIVGLCKSTVRWLLDLSRKNEFPFHGVTIKRHGKEETITYDEWDRKIQAHFEKLFFVSENPADPNEKHPNLVHKRGIYKDSYGASSPWCDYQLRPNFTIAMVVAPELFTPERAWKALQIAEEKLLGPLGMKTLDPDDMVYCGVYDNALDNDNYNVARGFNYHQGPEWLWPIGYFLRAKLYFSKLIGPQIYAKTVVMIKNVLSRHYVHLERSSWKGLPELTNENGQYCPFSCETQAWSISVILEILYDL

SEQ ID NO: 18 - DNA, 4131 bp, artificial
  Nucleic acid sequence encoding D1 hGDEWT
atgattcattttaccccattgcagactcttggactatctaggtcatgctactcccttgccaatcagttagaattaaatcctgacttttcaagacctaatagaaagtatacctggaatgatgttggacagctagtggaaaaattaaaaaaggaatggaatgttatttgtattactgatgttgtctacaatcatactgctgctaatagtaaatggatccaggaacatccagaatgtgcctataatcttgtaaattctccacacttaaaacctgcctgggtcttagacagagcactttggcgtttctcctgtgatgttgcagaagggaaatacaaagaaaagggaatacctgctttgattgaaaatgatcaccatatgaactccatccgaaaaataatttgggaggatatttttccaaagcttaaactctgggaatttttccaagtagatgtcaacaaagcggttgagcaatttagaagacttcttacacaagaaaataggcgagtaaccaagtctgatccaaaccaacaccttacgattattcaagatcctgaatacagacggtttggctgtactgtagatatgaacattgcactaacgactttcataccacatgacaaggggccagcagcaattgaagaatgctgtaattggtttcataaaagaatggaggaattaaattcagagaagcatcgactcattaactatcatcaggaacaggcagttaattgccttttgggaaatgtgttttatgaacgactggctggccatggtccaaaactaggacctgtcactagaaagcatcctttagttaccaggtattttactttcccatttgaagagatagacttctccatggaagaatctatgattcatctgccaaataaagcttgttttctgatggcacacaatggatgggtaatgggagatgatcctcttcgaaactttgctgaaccgggttcagaagtttacctaaggagagaacttatttgctggggagacagtgttaaattacgctatgggaataaaccagaggactgtccttatctctgggcacacatgaaaaaatacactgaaataactgcaacttatttccagggagtacgtcttgataactgccactcaacacctcttcacgtagctgagtacatgttggatgctgctaggaatttgcaacccaatttatatgtagtagctgaactgttcacaggaagtgaggacctagacaatgtctttgttactagactgggcattagttccttaataagagaggcaatgagtgcatataatagtcatgaagagggcagattagtttaccgatatggaggagaacctgttggatcctttgttcagccctgtttgaggcctttaatgccagctattgcacatgccctgtttatggatattacgcatgataatgagtgtcctattgtgcatagatcagcgtatgatgctcttccaagtactacaattgtttctatggcatgttgtgctagtggaagtacaagaggctatgatgaattagtgcctcatcagatttcagtggtttctgaagaacggttttacactaagtggaatcctgaagcattgccttcaaacacaggtgaagttaatttccaaagcggcattattgcagccaggtgtgctatcagtaaacttcatcaggagcttggagccaagggttttattcaggtgtatgtggatcaagttgatgaagacatagtggcagtaacaagacactcacctagcatccatcagtctgttgtggctgtaactagaactgctttcaggaatcccaagacttcattttacagcaaggaagtgcctcaaatgtgcatccctggcaaaattgaagaagtagttcttgaagctagaactattgagagaaacacgaaaccttataggaaggatgaaaattcaatcaatggaacaccagatatcacagtagaaattagagaacatattcagcttaatgaaagtaaaattgttaaacaagctggagttgccacaaaagggcccaatgaatatattcaagaaatagaatttgaaaacttgtctccaggaagtgttattatattcagagttagtcttgatccacatgcacaagtcgctgttggcattcttcgaaatcatctgacacaattcagtcctcactttaaatctggcagcctagctgttgacaatgcagatcctatattaaaaattccttttgcttctcttgcctatagattaactttggctgagctaaatcagatcctttaccgatgtgaatcagaagaaaaggaagatggtggagggtgctatgacataccaaactggtcagcccttaaatatgcaggtcttcaaggtttaatgtctgtattggcagaaataagaccaaagaatgacttggggcatcctttttgtaataatttgaggtctggagattggatgattgactatgtcagtaaccggcttatttcacgatcaggaactattgctgaagttggtaaatggttgcaggctatgttcttctacctgaagcagatcccacgttaccttatcccatgttactttgatgctatattaattggtgcatataccactcttctggatacagcatggaagcagatgtcaagctttgttcagaatggttcaacctttgtgaaacacctttcattgggttcagttcaactgtgtggagtaggaaaattcccttccctgccaattctttcacctgccctaatggatgtaccttataggttaaatgagatcacaaaagaaaaggagcaatgttgtgtttctctagctgcaggcttacctcatttttcttctggtattttccgctgctggggaagggatacttttattgcacttagaggtatactgctgattactggacgctatgtagaagccaggaatattattttagcatttgcgggtaccctgaggcatggtctcattcctaatctactgggtgaaggaatttatgccagatacaattgtcgggatgctgtgtggtggtggctgcagtgtatccaggattactgtaaaatggttccaaatggactagacattctcaagtgcccagtttccagaatgtatcctacagatgattctgctcctttgcctgctggcacactggatcagccattgtttgaagtcatacaggaagcaatgcaaaaacacatgcagggcatacagttccgagaaaggaatgctggtccccagatagatcgaaacatgaaggacgaaggttttaatataactgcaggagttgatgaagaaacaggatttgtttatggaggaaatcgtttcaattgtggcacatggatggataaaatgggagaaagtgacagagctagaaacagaggaatcccagccacaccaagagatgggtctgctgtggaaattgtgggcctgagtaaatctgctgttcgctggttgctggaattatccaaaaaaaatattttcccttatcatgaagtcacagtaaaaagacatggaaaggctataaaggtctcatatgatgagtggaacagaaaaatacaagacaactttgaaaagctatttcatgtttccgaagacccttcagatttaaatgaaaagcatccaaatctggttcacaaacgtggcatatacaaagatagttatggagcttcaagtccttggtgtgactatcagctcaggcctaattttaccatagcaatggttgtggcccctgagctctttactacagaaaaagcatggaaagctttggagattgcagaaaaaaaattgcttggtccccttggcatgaaaactttagatccagatgatatggtttactgtggaatttatgacaacgcattagacaatgacaactacaatcttgctaaaggtttcaattatcaccaaggacctgagtggctgtggcctattgggtattttcttcgtgcaaaattatatttttccagattgatgggcccggagactactgcaaagactatagttttggttaaaaatgttctttcccgacattatgttcatcttgagagatccccttggaaaggacttccagaactgaccaatgagaatgcccagtactgtcctttcagctgtgaaacacaagcctggtcaattgctactattcttgagacactttatgatttatag

SEQ ID NO: 19 - DNA, 4131 bp, artificial
  Nucleic acid sequence encoding D1 hGDE co2
atgatccacttcacccctctgcagaccctgggcctgagcagaagctgttacagcctggccaaccagctggaactgaaccccgacttcagcagacccaaccggaagtacacctggaacgatgtgggccagctggtggaaaaactgaagaaagaatggaacgtgatctgcatcaccgacgtggtgtacaaccacaccgccgccaacagcaagtggatccaagagcaccctgagtgcgcctacaacctggtcaacagccctcacctgaaacctgcctgggtgctcgatagagccctgtggcggtttagctgtgatgtggccgagggcaagtacaaagagaagggcatccccgctctgatcgagaacgaccaccacatgaacagcatccggaagatcatctgggaagatattttccccaagctgaagctgtgggagttcttccaggtggacgtgaacaaggccgtggaacagttcagacggctgctgacccaagagaacagaagagtgaccaagagcgaccccaaccagcacctgaccatcattcaggaccccgagtatcggagattcggctgcaccgtggacatgaatatcgccctgaccaccttcattccccacgacaaaggacctgccgccatcgaggaatgctgcaactggttccacaagcggatggaagaattgaacagcgagaagcaccggctgatcaactaccaccaagagcaggccgtgaactgcctgctgggcaacgtgttctatgagagactggccggacacggccctaagctgggacctgtgacaagaaagcaccctctggttacccggtacttcacctttccattcgaagagatcgacttctccatggaagagagcatgatccatctgcctaacaaggcctgcttcctgatggctcacaacggctgggttatgggcgacgaccctctgagaaatttcgccgagcctggcagcgaggtgtacctgagaagagaactgatctgttggggcgacagcgtgaagctgagatacggcaacaagcccgaggactgcccttacctgtgggcccatatgaagaagtacacagagatcaccgccacctactttcagggcgtcagactggacaactgccacagcacacctctgcacgtggccgagtacatgctggacgccgctagaaatctgcagcccaacctgtatgtggtggccgagctgtttaccggctccgaggacctggacaatgtgttcgtgaccagactgggcatcagcagcctgatcagagaagccatgtccgcctacaatagccacgaagagggcagactggtgtacagatatggcggcgagcctgtgggcagcttcgttcagccttgtctgaggcctctgatgcccgccattgctcacgccctgttcatggacatcacccacgataacgagtgccccatcgtgcacagaagcgcctacgacgctctgcctagcaccaccattgtgtccatggcctgttgtgccagcggcagcacaagaggctatgacgaactggtgccccaccagatttccgtggtgtccgaggaacggttctacaccaagtggaaccccgaggctctgcccagcaataccggcgaagtgaatttccagagcggcatcattgccgccagatgcgccatcagcaagctgcaccaagaactgggcgccaagggcttcattcaggtgtacgtggaccaggtcgacgaggacattgtggccgtgacaagacacagccccagcatccatcagagcgtggtggctgtgaccagaaccgccttcagaaaccccaagaccagcttctacagcaaagaggtgccccagatgtgcatccccggcaagattgaggaagtggtgctcgaggcccggaccatcgagagaaacaccaagccttaccggaaggacgagaactccatcaacggcacccctgacatcaccgtggaaatcagagagcacatccagctcaacgagagcaagatcgtgaaacaggccggcgtggccacaaagggccccaacgagtatatccaagagattgagttcgagaatctgagccccggcagcgtgatcatcttcagagtgtccctggatcctcacgctcaggtggccgtgggcatcctgagaaatcacctgacacagttcagcccacacttcaagagcggaagcctggccgtggacaacgccgatcctatcctgaagatccccttcgcctctctggcctacagactgacactggctgagctgaaccagatcctgtacagatgcgagtccgaagagaaagaggatggcggaggctgctacgacatccccaattggagcgccctgaagtatgccggactgcagggactgatgtctgtgctggccgagatcagacccaagaacgacctgggacaccccttctgcaacaacctgagatccggcgactggatgatcgactacgtgtccaacagactgatcagcagatccggcacaatcgccgaagtcggcaaatggctgcaggccatgttcttctacctgaagcagatccctcggtatctgatcccctgctacttcgacgccatcctgatcggcgcctacaccacactgctggataccgcctggaagcagatgtccagcttcgtgcagaacggcagcaccttcgtgaagcacctgtctctgggaagcgtgcagctgtgtggcgtgggcaaatttcccagcctgcctatcctgtctcctgcactgatggacgtgccctaccggctgaatgagatcaccaaagaaaaagagcagtgctgcgtcagcctggctgctggcctgcctcatttttccagcggcatcttccggtgttggggcagagacacctttattgccctgagaggcatcctgctgattaccggcagatacgtggaagcccggaacatcatcctggcctttgccggcacactgcggcacggactgattcctaatctgctcggcgagggcatctacgccagatacaactgcagagatgccgtgtggtggtggctccagtgcatccaggactactgcaagatggtgcccaacggcctggacatcctgaagtgccctgtgtccagaatgtaccctaccgacgatagcgcccctctgcctgccggaacacttgaccagcctctgttcgaagtgattcaagaggccatgcagaaacacatgcagggaatccagtttcgcgagcggaatgccggacctcagatcgacagaaacatgaaggatgagggcttcaacatcaccgctggcgtggacgaagagacaggctttgtgtacggcggcaaccggttcaattgcggcacctggatggacaagatgggcgagtctgaccgggccagaaacagaggaattcccgccacacctagagatggcagcgctgtggaaatcgtgggcctgtctaagtctgctgtgcggtggctgctcgaactgagcaagaagaatatctttccgtaccacgaagtgaccgtgaagcggcacggcaaggccatcaaggtgtcctacgacgagtggaacagaaagatccaggacaacttcgaaaagctgttccatgtgtctgaggaccccagcgacctgaacgaaaagcaccccaacctggtgcacaagcgcggcatctacaaggacagctacggcgcctcttctccttggtgcgattaccagctgcggcccaacttcaccattgccatggtggttgcccctgagctgttcaccacagagaaggcctggaaggccctggaaatcgccgagaagaaactgctgggccctctgggcatgaagacactggaccccgacgacatggtgtactgcggaatctacgacaacgccctggataacgacaactacaatctggccaaggggttcaattaccatcagggacccgagtggctgtggcctatcggctatttcctgcgggccaagctgtacttctccagactgatgggccctgagacaaccgccaagacaatcgtgctcgtgaagaacgtgctgagccggcactatgtgcacctggaaagaagcccctggaagggactgcccgagctgaccaatgagaacgcccagtactgccccttcagctgcgaaacacaggcctggtctatcgccaccatcctggaaaccctgtacgacctgtga

SEQ ID NO: 20 - DNA, 4395 bp, artificial
  Nucleic acid sequence encoding D2 hGDE
atgggacacagtaaacagattcgaattttacttctgaacgaaatggagaaactggaaaagaccctcttcagacttgaacaagggtatgagctacagttccgattaggcccaactttacagggaaaagcagttaccgtgtatacaaattacccatttcctggagaaacatttaatagagaaaaattccgttctctggattgggaaaatccaacagaaagagaagatgattctgataaatactgtaaacttaatctgcaacaatctggttcatttcagtattatttccttcaaggaaatgagaaaagtggtggaggttacatagttgtggaccccattttacgtgttggtgctgataatcatgtgctacccttggactgtgttactcttcagacatttttagctaagtgtttgggaccttttgatgaatgggaaagcagacttagggttgcaaaagaatcaggctacaacatgattcattttaccccattgcagactcttggactatctaggtcatgctactcccttgccaatcagttagaattaaatcctgacttttcaagacctaatagaaagtatacctggaatgatgttggacagctagtggaaaaattaaaaaaggaatggaatgttatttgtattactgatgttgtctacaatcatactgctgctaatagtaaatggatccaggaacatccagaatgtgcctataatcttgtaaattctccacacttaaaacctgcctgggtcttagacagagcactttggcgtttctcctgtgatgttgcagaagggaaatacaaagaaaagggaatacctgctttgattgaaaatgatcaccatatgaactccatccgaaaaataatttgggaggatatttttccaaagcttaaactctgggaatttttccaagtagatgtcaacaaagcggttgagcaatttagaagacttcttacacaagaaaataggcgagtaaccaagtctgatccaaaccaacaccttacgattattcaagatcctgaatacagacggtttggctgtactgtagatatgaacattgcactaacgactttcataccacattattttactttcccatttgaagagatagacttctccatggaagaatctatgattcatctgccaaataaagcttgttttctgatggcacacaatggatgggtaatgggagatgatcctcttcgaaactttgctgaaccgggttcagaagtttacctaaggagagaacttatttgctggggagacagtgttaaattacgctatgggaataaaccagaggactgtccttatctctgggcacacatgaaaaaatacactgaaataactgcaacttatttccagggagtacgtcttgataactgccactcaacacctcttcacgtagctgagtacatgttggatgctgctaggaatttgcaacccaatttatatgtagtagctgaactgttcacaggaagtgaggacctagacaatgtctttgttactagactgggcattagttccttaataagagaggcaatgagtgcatataatagtcatgaagagggcagattagtttaccgatatggaggagaacctgttggatcctttgttcagccctgtttgaggcctttaatgccagctattgcacatgccctgtttatggatattacgcatgataatgagtgtcctattgtgcatagatcagcgtatgatgctcttccaagtactacaattgtttctatggcatgttgtgctagtggaagtacaagaggctatgatgaattagtgcctcatcagatttcagtggtttctgaagaacggttttacactaagtggaatcctgaagcattgccttcaaacacaggtgaagttaatttccaaagcggcattattgcagccaggtgtgctatcagtaaacttcatcaggagcttggagccaagggttttattcaggtgtatgtggatcaagttgatgaagacatagtggcagtaacaagacactcacctagcatccatcagtctgttgtggctgtaactagaactgctttcaggaatcccaagacttcattttacagcaaggaagtgcctcaaatgtgcatccctggcaaaattgaagaagtagttcttgaagctagaactattgagagaaacacgaaaccttataggaaggatgaaaattcaatcaatggaacaccagatatcacagtagaaattagagaacatattcagcttaatgaaagtaaaattgttaaacaagctggagttgccacaaaagggcccaatgaatatattcaagaaatagaatttgaaaacttgtctccaggaagtgttattatattcagagttagtcttgatccacatgcacaagtcgctgttggcattcttcgaaatcatctgacacaattcagtcctcactttaaatctggcagcctagctgttgacaatgcagatcctatattaaaaattccttttgcttctcttgcctatagattaactttggctgagctaaatcagatcctttaccgatgtgaatcagaagaaaaggaagatggtggagggtgctatgacataccaaactggtcagcccttaaatatgcaggtcttcaaggtttaatgtctgtattggcagaaataagaccaaagaatgacttggggcatcctttttgtaataatttgaggtctggagattggatgattgactatgtcagtaaccggcttatttcacgatcaggaactattgctgaagttggtaaatggttgcaggctatgttcttctacctgaagcagatcccacgttaccttatcccatgttactttgatgctatattaattggtgcatataccactcttctggatacagcatggaagcagatgtcaagctttgttcagaatggttcaacctttgtgaaacacctttcattgggttcagttcaactgtgtggagtaggaaaattcccttccctgccaattctttcacctgccctaatggatgtaccttataggttaaatgagatcacaaaagaaaaggagcaatgttgtgtttctctagctgcaggcttacctcatttttcttctggtattttccgctgctggggaagggatacttttattgcacttagaggtatactgctgattactggacgctatgtagaagccaggaatattattttagcatttgcgggtaccctgaggcatggtctcattcctaatctactgggtgaaggaatttatgccagatacaattgtcgggatgctgtgtggtggtggctgcagtgtatccaggattactgtaaaatggttccaaatggactagacattctcaagtgcccagtttccagaatgtatcctacagatgattctgctcctttgcctgctggcacactggatcagccattgtttgaagtcatacaggaagcaatgcaaaaacacatgcagggcatacagttccgagaaaggaatgctggtccccagatagatcgaaacatgaaggacgaaggttttaatataactgcaggagttgatgaagaaacaggatttgtttatggaggaaatcgtttcaattgtggcacatggatggataaaatgggagaaagtgacagagctagaaacagaggaatcccagccacaccaagagatgggtctgctgtggaaattgtgggcctgagtaaatctgctgttcgctggttgctggaattatccaaaaaaaatattttcccttatcatgaagtcacagtaaaaagacatggaaaggctataaaggtctcatatgatgagtggaacagaaaaatacaagacaactttgaaaagctatttcatgtttccgaagacccttcagatttaaatgaaaagcatccaaatctggttcacaaacgtggcatatacaaagatagttatggagcttcaagtccttggtgtgactatcagctcaggcctaattttaccatagcaatggttgtggcccctgagctctttactacagaaaaagcatggaaagctttggagattgcagaaaaaaaattgcttggtccccttggcatgaaaactttagatccagatgatatggtttactgtggaatttatgacaacgcattagacaatgacaactacaatcttgctaaaggtttcaattatcaccaaggacctgagtggctgtggcctattgggtattttcttcgtgcaaaattatatttttccagattgatgggcccggagactactgcaaagactatagttttggttaaaaatgttctttcccgacattatgttcatcttgagagatccccttggaaaggacttccagaactgaccaatgagaatgcccagtactgtcctttcagctgtgaaacacaagcctggtcaattgctactattcttgagacactttatgatttatag

SEQ ID NO: 21 - DNA, 4293 bp, artificial
  Nucleic acid sequence encoding D3 hGDE
atgggacacagtaaacagattcgaattttacttctgaacgaaatggagaaactggaaaagaccctcttcagacttgaacaagggtatgagctacagttccgattaggcccaactttacagggaaaagcagttaccgtgtatacaaattacccatttcctggagaaacatttaatagagaaaaattccgttctctggattgggaaaatccaacagaaagagaagatgattctgataaatactgtaaacttaatctgcaacaatctggttcatttcagtattatttccttcaaggaaatgagaaaagtggtggaggttacatagttgtggaccccattttacgtgttggtgctgataatcatgtgctacccttggactgtgttactcttcagacatttttagctaagtgtttgggaccttttgatgaatgggaaagcagacttagggttgcaaaagaatcaggctacaacatgattcattttaccccattgcagactcttggactatctaggtcatgctactcccttgccaatcagttagaattaaatcctgacttttcaagacctaatagaaagtatacctggaatgatgttggacagctagtggaaaaattaaaaaaggaatggaatgttatttgtattactgatgttgtctacaatcatactgctgctaatagtaaatggatccaggaacatccagaatgtgcctataatcttgtaaattctccacacttaaaacctgcctgggtcttagacagagcactttggcgtttctcctgtgatgttgcagaagggaaatacaaagaaaagggaatacctgctttgattgaaaatgatcaccatatgaactccatccgaaaaataatttgggaggatatttttccaaagcttaaactctgggaatttttccaagtagatgtcaacaaagcggttgagcaatttagaagacttcttacacaagaaaataggcgagtaaccaagtctgatccaaaccaacaccttacgattattcaagatcctgaatacagacggtttggctgtactgtagatatgaacattgcactaacgactttcataccacatgacaaggggccagcagcaattgaagaatgctgtaattggtttcataaaagaatggaggaattaaattcagagaagcatcgactcattaactatcatcaggaacaggcagttaattgccttttgggaaatgtgttttatgaacgactggctggccatggtccaaaactaggacctgtcactagaaagcatcctttagttaccaggtattttactttcccatttgaagagatagacttctccatggaagaatctatgattcatctgccaaataaagcttgttttctgatggcacacaatggatgggtaatgggagatgatcctcttcgaaactttgctgaaccgggttcagaagtttacctaaggagagaacttatttgctggggagacagtgttaaattacgctatgggaataaaccagaggactgtccttatctctgggcacacatgaaaaaatacactgaaataactgcaacttatttccagggagtacgtcttgataactgccactcaacacctcttcacgtagctgagtacatgttggatgctgctaggaatttgcaacccaatttatatgtagtagctgaactgttcacaggaagtgaggacctagacaatgtctttgttactagactgggcattagttccttaataagagaggcaatgagtgcatataatagtcatgaagagggcagattagtttaccgatatggaggagaacctgttggatcctttgttcagccctgtttgaggcctttaatgccagctattgcacatgccctgtttatggatattacgcatgataatgagtgtcctattgtgcatagatcagcgtatgatgctcttccaagtactacaattgtttctatggcatgttgtgctagtggaagtacaagaggctatgatgaattagtgcctcatcagggcaaaattgaagaagtagttcttgaagctagaactattgagagaaacacgaaaccttataggaaggatgaaaattcaatcaatggaacaccagatatcacagtagaaattagagaacatattcagcttaatgaaagtaaaattgttaaacaagctggagttgccacaaaagggcccaatgaatatattcaagaaatagaatttgaaaacttgtctccaggaagtgttattatattcagagttagtcttgatccacatgcacaagtcgctgttggcattcttcgaaatcatctgacacaattcagtcctcactttaaatctggcagcctagctgttgacaatgcagatcctatattaaaaattccttttgcttctcttgcctatagattaactttggctgagctaaatcagatcctttaccgatgtgaatcagaagaaaaggaagatggtggagggtgctatgacataccaaactggtcagcccttaaatatgcaggtcttcaaggtttaatgtctgtattggcagaaataagaccaaagaatgacttggggcatcctttttgtaataatttgaggtctggagattggatgattgactatgtcagtaaccggcttatttcacgatcaggaactattgctgaagttggtaaatggttgcaggctatgttcttctacctgaagcagatcccacgttaccttatcccatgttactttgatgctatattaattggtgcatataccactcttctggatacagcatggaagcagatgtcaagctttgttcagaatggttcaacctttgtgaaacacctttcattgggttcagttcaactgtgtggagtaggaaaattcccttccctgccaattctttcacctgccctaatggatgtaccttataggttaaatgagatcacaaaagaaaaggagcaatgttgtgtttctctagctgcaggcttacctcatttttcttctggtattttccgctgctggggaagggatacttttattgcacttagaggtatactgctgattactggacgctatgtagaagccaggaatattattttagcatttgcgggtaccctgaggcatggtctcattcctaatctactgggtgaaggaatttatgccagatacaattgtcgggatgctgtgtggtggtggctgcagtgtatccaggattactgtaaaatggttccaaatggactagacattctcaagtgcccagtttccagaatgtatcctacagatgattctgctcctttgcctgctggcacactggatcagccattgtttgaagtcatacaggaagcaatgcaaaaacacatgcagggcatacagttccgagaaaggaatgctggtccccagatagatcgaaacatgaaggacgaaggttttaatataactgcaggagttgatgaagaaacaggatttgtttatggaggaaatcgtttcaattgtggcacatggatggataaaatgggagaaagtgacagagctagaaacagaggaatcccagccacaccaagagatgggtctgctgtggaaattgtgggcctgagtaaatctgctgttcgctggttgctggaattatccaaaaaaaatattttcccttatcatgaagtcacagtaaaaagacatggaaaggctataaaggtctcatatgatgagtggaacagaaaaatacaagacaactttgaaaagctatttcatgtttccgaagacccttcagatttaaatgaaaagcatccaaatctggttcacaaacgtggcatatacaaagatagttatggagcttcaagtccttggtgtgactatcagctcaggcctaattttaccatagcaatggttgtggcccctgagctctttactacagaaaaagcatggaaagctttggagattgcagaaaaaaaattgcttggtccccttggcatgaaaactttagatccagatgatatggtttactgtggaatttatgacaacgcattagacaatgacaactacaatcttgctaaaggtttcaattatcaccaaggacctgagtggctgtggcctattgggtattttcttcgtgcaaaattatatttttccagattgatgggcccggagactactgcaaagactatagttttggttaaaaatgttctttcccgacattatgttcatcttgagagatccccttggaaaggacttccagaactgaccaatgagaatgcccagtactgtcctttcagctgtgaaacacaagcctggtcaattgctactattcttgagacactttatgatttatag

SEQ ID NO: 22 - DNA, 4089 bp, artificial
  Nucleic acid sequence encoding D2,3 hGDE WT
atgggacacagtaaacagattcgaattttacttctgaacgaaatggagaaactggaaaagaccctcttcagacttgaacaagggtatgagctacagttccgattaggcccaactttacagggaaaagcagttaccgtgtatacaaattacccatttcctggagaaacatttaatagagaaaaattccgttctctggattgggaaaatccaacagaaagagaagatgattctgataaatactgtaaacttaatctgcaacaatctggttcatttcagtattatttccttcaaggaaatgagaaaagtggtggaggttacatagttgtggaccccattttacgtgttggtgctgataatcatgtgctacccttggactgtgttactcttcagacatttttagctaagtgtttgggaccttttgatgaatgggaaagcagacttagggttgcaaaagaatcaggctacaacatgattcattttaccccattgcagactcttggactatctaggtcatgctactcccttgccaatcagttagaattaaatcctgacttttcaagacctaatagaaagtatacctggaatgatgttggacagctagtggaaaaattaaaaaaggaatggaatgttatttgtattactgatgttgtctacaatcatactgctgctaatagtaaatggatccaggaacatccagaatgtgcctataatcttgtaaattctccacacttaaaacctgcctgggtcttagacagagcactttggcgtttctcctgtgatgttgcagaagggaaatacaaagaaaagggaatacctgctttgattgaaaatgatcaccatatgaactccatccgaaaaataatttgggaggatatttttccaaagcttaaactctgggaatttttccaagtagatgtcaacaaagcggttgagcaatttagaagacttcttacacaagaaaataggcgagtaaccaagtctgatccaaaccaacaccttacgattattcaagatcctgaatacagacggtttggctgtactgtagatatgaacattgcactaacgactttcataccacattattttactttcccatttgaagagatagacttctccatggaagaatctatgattcatctgccaaataaagcttgttttctgatggcacacaatggatgggtaatgggagatgatcctcttcgaaactttgctgaaccgggttcagaagtttacctaaggagagaacttatttgctggggagacagtgttaaattacgctatgggaataaaccagaggactgtccttatctctgggcacacatgaaaaaatacactgaaataactgcaacttatttccagggagtacgtcttgataactgccactcaacacctcttcacgtagctgagtacatgttggatgctgctaggaatttgcaacccaatttatatgtagtagctgaactgttcacaggaagtgaggacctagacaatgtctttgttactagactgggcattagttccttaataagagaggcaatgagtgcatataatagtcatgaagagggcagattagtttaccgatatggaggagaacctgttggatcctttgttcagccctgtttgaggcctttaatgccagctattgcacatgccctgtttatggatattacgcatgataatgagtgtcctattgtgcatagatcagcgtatgatgctcttccaagtactacaattgtttctatggcatgttgtgctagtggaagtacaagaggctatgatgaattagtgcctcatcagggcaaaattgaagaagtagttcttgaagctagaactattgagagaaacacgaaaccttataggaaggatgaaaattcaatcaatggaacaccagatatcacagtagaaattagagaacatattcagcttaatgaaagtaaaattgttaaacaagctggagttgccacaaaagggcccaatgaatatattcaagaaatagaatttgaaaacttgtctccaggaagtgttattatattcagagttagtcttgatccacatgcacaagtcgctgttggcattcttcgaaatcatctgacacaattcagtcctcactttaaatctggcagcctagctgttgacaatgcagatcctatattaaaaattccttttgcttctcttgcctatagattaactttggctgagctaaatcagatcctttaccgatgtgaatcagaagaaaaggaagatggtggagggtgctatgacataccaaactggtcagcccttaaatatgcaggtcttcaaggtttaatgtctgtattggcagaaataagaccaaagaatgacttggggcatcctttttgtaataatttgaggtctggagattggatgattgactatgtcagtaaccggcttatttcacgatcaggaactattgctgaagttggtaaatggttgcaggctatgttcttctacctgaagcagatcccacgttaccttatcccatgttactttgatgctatattaattggtgcatataccactcttctggatacagcatggaagcagatgtcaagctttgttcagaatggttcaacctttgtgaaacacctttcattgggttcagttcaactgtgtggagtaggaaaattcccttccctgccaattctttcacctgccctaatggatgtaccttataggttaaatgagatcacaaaagaaaaggagcaatgttgtgtttctctagctgcaggcttacctcatttttcttctggtattttccgctgctggggaagggatacttttattgcacttagaggtatactgctgattactggacgctatgtagaagccaggaatattattttagcatttgcgggtaccctgaggcatggtctcattcctaatctactgggtgaaggaatttatgccagatacaattgtcgggatgctgtgtggtggtggctgcagtgtatccaggattactgtaaaatggttccaaatggactagacattctcaagtgcccagtttccagaatgtatcctacagatgattctgctcctttgcctgctggcacactggatcagccattgtttgaagtcatacaggaagcaatgcaaaaacacatgcagggcatacagttccgagaaaggaatgctggtccccagatagatcgaaacatgaaggacgaaggttttaatataactgcaggagttgatgaagaaacaggatttgtttatggaggaaatcgtttcaattgtggcacatggatggataaaatgggagaaagtgacagagctagaaacagaggaatcccagccacaccaagagatgggtctgctgtggaaattgtgggcctgagtaaatctgctgttcgctggttgctggaattatccaaaaaaaatattttcccttatcatgaagtcacagtaaaaagacatggaaaggctataaaggtctcatatgatgagtggaacagaaaaatacaagacaactttgaaaagctatttcatgtttccgaagacccttcagatttaaatgaaaagcatccaaatctggttcacaaacgtggcatatacaaagatagttatggagcttcaagtccttggtgtgactatcagctcaggcctaattttaccatagcaatggttgtggcccctgagctctttactacagaaaaagcatggaaagctttggagattgcagaaaaaaaattgcttggtccccttggcatgaaaactttagatccagatgatatggtttactgtggaatttatgacaacgcattagacaatgacaactacaatcttgctaaaggtttcaattatcaccaaggacctgagtggctgtggcctattgggtattttcttcgtgcaaaattatatttttccagattgatgggcccggagactactgcaaagactatagttttggttaaaaatgttctttcccgacattatgttcatcttgagagatccccttggaaaggacttccagaactgaccaatgagaatgcccagtactgtcctttcagctgtgaaacacaagcctggtcaattgctactattcttgagacactttatgatttatag

SEQ ID NO: 23 - DNA, 4089 bp, artificial
  Nucleic acid sequence encoding D2,3 hGDE co2
atgggccacagcaagcagatcagaatcctgctgctgaacgagatggaaaagctggaaaagaccctgttccggctcgagcagggctacgagctgcagtttagactgggccctacactgcagggcaaagccgtgaccgtgtacacaaactaccccttccctggcgaaaccttcaaccgcgagaagttcagaagcctggactgggagaaccccaccgagagagaggacgacagcgacaagtactgcaagctgaacctgcagcagagcggctccttccagtactacttcctgcaaggcaacgagaagtccggcggaggctacatcgtggtggaccctattctgagagtgggcgccgacaatcacgtgctgcctctggattgtgtgaccctgcagaccttcctggccaagtgtctgggccctttcgatgagtgggagagcagactgcgcgtggccaaagaaagcggctacaacatgatccacttcacccctctgcagaccctgggcctgagcagaagctgttacagcctggccaaccagctggaactgaaccccgacttcagcagacccaaccggaagtacacctggaacgatgtgggccagctggtggaaaaactgaagaaagaatggaacgtgatctgcatcaccgacgtggtgtacaaccacaccgccgccaacagcaagtggatccaagagcaccctgagtgcgcctacaacctggtcaacagccctcacctgaaacctgcctgggtgctcgatagagccctgtggcggtttagctgtgatgtggccgagggcaagtacaaagagaagggcatccccgctctgatcgagaacgaccaccacatgaacagcatccggaagatcatctgggaagatattttccccaagctgaagctgtgggagttcttccaggtggacgtgaacaaggccgtggaacagttcagacggctgctgacccaagagaacagaagagtgaccaagagcgaccccaaccagcacctgaccatcattcaggaccccgagtatcggagattcggctgcaccgtggacatgaatatcgccctgaccaccttcattccccactacttcacctttccattcgaagagatcgacttctccatggaagagagcatgatccatctgcctaacaaggcctgcttcctgatggctcacaacggctgggttatgggcgacgaccctctgagaaatttcgccgagcctggcagcgaggtgtacctgagaagagaactgatctgttggggcgacagcgtgaagctgagatacggcaacaagcccgaggactgcccttacctgtgggcccatatgaagaagtacacagagatcaccgccacctactttcagggcgtcagactggacaactgccacagcacacctctgcacgtggccgagtacatgctggacgccgctagaaatctgcagcccaacctgtatgtggtggccgagctgtttaccggctccgaggacctggacaatgtgttcgtgaccagactgggcatcagcagcctgatcagagaagccatgtccgcctacaatagccacgaagagggcagactggtgtacagatatggcggcgagcctgtgggcagcttcgttcagccttgtctgaggcctctgatgcccgccattgctcacgccctgttcatggacatcacccacgataacgagtgccccatcgtgcacagaagcgcctacgacgctctgcctagcaccaccattgtgtccatggcctgttgtgccagcggcagcacaagaggctatgacgaactggtgccccaccagggcaagattgaggaagtggtgctcgaggcccggaccatcgagagaaacaccaagccttaccggaaggacgagaactccatcaacggcacccctgacatcaccgtggaaatcagagagcacatccagctcaacgagagcaagatcgtgaaacaggccggcgtggccacaaagggccccaacgagtatatccaagagattgagttcgagaatctgagccccggcagcgtgatcatcttcagagtgtccctggatcctcacgctcaggtggccgtgggcatcctgagaaatcacctgacacagttcagcccacacttcaagagcggaagcctggccgtggacaacgccgatcctatcctgaagatccccttcgcctctctggcctacagactgacactggctgagctgaaccagatcctgtacagatgcgagtccgaagagaaagaggatggcggaggctgctacgacatccccaattggagcgccctgaagtatgccggactgcagggactgatgtctgtgctggccgagatcagacccaagaacgacctgggacaccccttctgcaacaacctgagatccggcgactggatgatcgactacgtgtccaacagactgatcagcagatccggcacaatcgccgaagtcggcaaatggctgcaggccatgttcttctacctgaagcagatccctcggtatctgatcccctgctacttcgacgccatcctgatcggcgcctacaccacactgctggataccgcctggaagcagatgtccagcttcgtgcagaacggcagcaccttcgtgaagcacctgtctctgggaagcgtgcagctgtgtggcgtgggcaaatttcccagcctgcctatcctgtctcctgcactgatggacgtgccctaccggctgaatgagatcaccaaagaaaaagagcagtgctgcgtcagcctggctgctggcctgcctcatttttccagcggcatcttccggtgttggggcagagacacctttattgccctgagaggcatcctgctgattaccggcagatacgtggaagcccggaacatcatcctggcctttgccggcacactgcggcacggactgattcctaatctgctcggcgagggcatctacgccagatacaactgcagagatgccgtgtggtggtggctccagtgcatccaggactactgcaagatggtgcccaacggcctggacatcctgaagtgccctgtgtccagaatgtaccctaccgacgatagcgcccctctgcctgccggaacacttgaccagcctctgttcgaagtgattcaagaggccatgcagaaacacatgcagggaatccagtttcgcgagcggaatgccggacctcagatcgacagaaacatgaaggatgagggcttcaacatcaccgctggcgtggacgaagagacaggctttgtgtacggcggcaaccggttcaattgcggcacctggatggacaagatgggcgagtctgaccgggccagaaacagaggaattcccgccacacctagagatggcagcgctgtggaaatcgtgggcctgtctaagtctgctgtgcggtggctgctcgaactgagcaagaagaatatctttccgtaccacgaagtgaccgtgaagcggcacggcaaggccatcaaggtgtcctacgacgagtggaacagaaagatccaggacaacttcgaaaagctgttccatgtgtctgaggaccccagcgacctgaacgaaaagcaccccaacctggtgcacaagcgcggcatctacaaggacagctacggcgcctcttctccttggtgcgattaccagctgcggcccaacttcaccattgccatggtggttgcccctgagctgttcaccacagagaaggcctggaaggccctggaaatcgccgagaagaaactgctgggccctctgggcatgaagacactggaccccgacgacatggtgtactgcggaatctacgacaacgccctggataacgacaactacaatctggccaaggggttcaattaccatcagggacccgagtggctgtggcctatcggctatttcctgcgggccaagctgtacttctccagactgatgggccctgagacaaccgccaagacaatcgtgctcgtgaagaacgtgctgagccggcactatgtgcacctggaaagaagcccctggaagggactgcccgagctgaccaatgagaacgcccagtactgccccttcagctgcgaaacacaggcctggtctatcgccaccatcctggaaaccctgtacgacctgtga

SEQ ID NO: 24 - DNA, 4020 bp, artificial
  Nucleic acid sequence encoding D4 hGDE WT
atgggacacagtaaacagattcgaattttacttctgaacgaaatggagaaactggaaaagaccctcttcagacttgaacaagggtatgagctacagttccgattaggcccaactttacagggaaaagcagttaccgtgtatacaaattacccatttcctggagaaacatttaatagagaaaaattccgttctctggattgggaaaatccaacagaaagagaagatgattctgataaatactgtaaacttaatctgcaacaatctggttcatttcagtattatttccttcaaggaaatgagaaaagtggtggaggttacatagttgtggaccccattttacgtgttggtgctgataatcatgtgctacccttggactgtgttactcttcagacatttttagctaagtgtttgggaccttttgatgaatgggaaagcagacttagggttgcaaaagaatcaggctacaacatgattcattttaccccattgcagactcttggactatctaggtcatgctactcccttgccaatcagttagaattaaatcctgacttttcaagacctaatagaaagtatacctggaatgatgttggacagctagtggaaaaattaaaaaaggaatggaatgttatttgtattactgatgttgtctacaatcatactgctgctaatagtaaatggatccaggaacatccagaatgtgcctataatcttgtaaattctccacacttaaaacctgcctgggtcttagacagagcactttggcgtttctcctgtgatgttgcagaagggaaatacaaagaaaagggaatacctgctttgattgaaaatgatcaccatatgaactccatccgaaaaataatttgggaggatatttttccaaagcttaaactctgggaatttttccaagtagatgtcaacaaagcggttgagcaatttagaagacttcttacacaagaaaataggcgagtaaccaagtctgatccaaaccaacaccttacgattattcaagatcctgaatacagacggtttggctgtactgtagatatgaacattgcactaacgactttcataccacatgacaaggggccagcagcaattgaagaatgctgtaattggtttcataaaagaatggaggaattaaattcagagaagcatcgactcattaactatcatcaggaacaggcagttaattgccttttgggaaatgtgttttatgaacgactggctggccatggtccaaaactaggacctgtcactagaaagcatcctttagttaccaggtattttactttcccatttgaagagatagacttctccatggaagaatctatgattcatctgccaaataaagcttgttttctgatggcacacaatggatgggtaatgggagatgatcctcttcgaaactttgctgaaccgggttcagaagtttacctaaggagagaacttatttgctggggagacagtgttaaattacgctatgggaataaaccagaggactgtccttatctctgggcacacatgaaaaaatacactgaaataactgcaacttatttccagggagtacgtcttgataactgccactcaacacctcttcacgtagctgagtacatgttggatgctgctaggaatttgcaacccaatttatatgtagtagctgaactgttcacaggaagtgaggacctagacaatgtctttgttactagactgggcattagttccttaataagagaggcaatgagtgcatataatagtcatgaagagggcagattagtttaccgatatggaggagaacctgttggatcctttgttcagccctgtttgaggcctttaatgccagctattgcacatgccctgtttatggatattacgcatgataatgagtgtcctattgtgcatagatcagcgtatgatgctcttccaagtactacaattgtttctatggcatgttgtgctagtggaagtacaagaggctatgatgaattagtgcctcatcagatttcagtggtttctgaagaacggttttacactaagtggaatcctgaagcattgccttcaaacacaggtgaagttaatttccaaagcggcattattgcagccaggtgtgctatcagtaaacttcatcaggagcttggagccaagggttttattcaggtgtatgtggatcaagttgatgaagacatagtggcagtaacaagacactcacctagcatccatcagtctgttgtggctgtaactagaactgctttcaggaatcccaagacttcattttacagcaaggaagtgcctcaaatgtgcatccctggcaaaattgaagaagtagttcttgaagctagaactattgagagaaacacgaaaccttataggaaggatgaaaattcaatcaatggaacaccagatatcacagtagaaattagagaacatattcagcttaatgaaagtaaaattgttaaacaagctggagttgccacaaaagggcccaatgaatatattcaagaaatagaatttgaaaacttgtctccaggaagtgttattatattcagagttagtcttgatccacatgcacaagtcgctgttggcattcttcgaaatcatctgacacaattcagtcctcactttaaatctggcagcctagctgttgacaatgcagatcctatattaaaaattccttttgcttctttacctcatttttcttctggtattttccgctgctggggaagggatacttttattgcacttagaggtatactgctgattactggacgctatgtagaagccaggaatattattttagcatttgcgggtaccctgaggcatggtctcattcctaatctactgggtgaaggaatttatgccagatacaattgtcgggatgctgtgtggtggtggctgcagtgtatccaggattactgtaaaatggttccaaatggactagacattctcaagtgcccagtttccagaatgtatcctacagatgattctgctcctttgcctgctggcacactggatcagccattgtttgaagtcatacaggaagcaatgcaaaaacacatgcagggcatacagttccgagaaaggaatgctggtccccagatagatcgaaacatgaaggacgaaggttttaatataactgcaggagttgatgaagaaacaggatttgtttatggaggaaatcgtttcaattgtggcacatggatggataaaatgggagaaagtgacagagctagaaacagaggaatcccagccacaccaagagatgggtctgctgtggaaattgtgggcctgagtaaatctgctgttcgctggttgctggaattatccaaaaaaaatattttcccttatcatgaagtcacagtaaaaagacatggaaaggctataaaggtctcatatgatgagtggaacagaaaaatacaagacaactttgaaaagctatttcatgtttccgaagacccttcagatttaaatgaaaagcatccaaatctggttcacaaacgtggcatatacaaagatagttatggagcttcaagtccttggtgtgactatcagctcaggcctaattttaccatagcaatggttgtggcccctgagctctttactacagaaaaagcatggaaagctttggagattgcagaaaaaaaattgcttggtccccttggcatgaaaactttagatccagatgatatggtttactgtggaatttatgacaacgcattagacaatgacaactacaatcttgctaaaggtttcaattatcaccaaggacctgagtggctgtggcctattgggtattttcttcgtgcaaaattatatttttccagattgatgggcccggagactactgcaaagactatagttttggttaaaaatgttctttcccgacattatgttcatcttgagagatccccttggaaaggacttccagaactgaccaatgagaatgcccagtactgtcctttcagctgtgaaacacaagcctggtcaattgctactattcttgagacactttatgatttatag

SEQ ID NO: 25 - DNA, 4020 bp, artificial
  Nucleic acid sequence encoding D4 hGDE co2
atgggccacagcaagcagatcagaatcctgctgctgaacgagatggaaaagctggaaaagaccctgttccggctcgagcagggctacgagctgcagtttagactgggccctacactgcagggcaaagccgtgaccgtgtacacaaactaccccttccctggcgaaaccttcaaccgcgagaagttcagaagcctggactgggagaaccccaccgagagagaggacgacagcgacaagtactgcaagctgaacctgcagcagagcggctccttccagtactacttcctgcaaggcaacgagaagtccggcggaggctacatcgtggtggaccctattctgagagtgggcgccgacaatcacgtgctgcctctggattgtgtgaccctgcagaccttcctggccaagtgtctgggccctttcgatgagtgggagagcagactgcgcgtggccaaagaaagcggctacaacatgatccacttcacccctctgcagaccctgggcctgagcagaagctgttacagcctggccaaccagctggaactgaaccccgacttcagcagacccaaccggaagtacacctggaacgatgtgggccagctggtggaaaaactgaagaaagaatggaacgtgatctgcatcaccgacgtggtgtacaaccacaccgccgccaacagcaagtggatccaagagcaccctgagtgcgcctacaacctggtcaacagccctcacctgaaacctgcctgggtgctcgatagagccctgtggcggtttagctgtgatgtggccgagggcaagtacaaagagaagggcatccccgctctgatcgagaacgaccaccacatgaacagcatccggaagatcatctgggaagatattttccccaagctgaagctgtgggagttcttccaggtggacgtgaacaaggccgtggaacagttcagacggctgctgacccaagagaacagaagagtgaccaagagcgaccccaaccagcacctgaccatcattcaggaccccgagtatcggagattcggctgcaccgtggacatgaatatcgccctgaccaccttcattccccacgacaaaggacctgccgccatcgaggaatgctgcaactggttccacaagcggatggaagaattgaacagcgagaagcaccggctgatcaactaccaccaagagcaggccgtgaactgcctgctgggcaacgtgttctatgagagactggccggacacggccctaagctgggacctgtgacaagaaagcaccctctggttacccggtacttcacctttccattcgaagagatcgacttctccatggaagagagcatgatccatctgcctaacaaggcctgcttcctgatggctcacaacggctgggttatgggcgacgaccctctgagaaatttcgccgagcctggcagcgaggtgtacctgagaagagaactgatctgttggggcgacagcgtgaagctgagatacggcaacaagcccgaggactgcccttacctgtgggcccatatgaagaagtacacagagatcaccgccacctactttcagggcgtcagactggacaactgccacagcacacctctgcacgtggccgagtacatgctggacgccgctagaaatctgcagcccaacctgtatgtggtggccgagctgtttaccggctccgaggacctggacaatgtgttcgtgaccagactgggcatcagcagcctgatcagagaagccatgtccgcctacaatagccacgaagagggcagactggtgtacagatatggcggcgagcctgtgggcagcttcgttcagccttgtctgaggcctctgatgcccgccattgctcacgccctgttcatggacatcacccacgataacgagtgccccatcgtgcacagaagcgcctacgacgctctgcctagcaccaccattgtgtccatggcctgttgtgccagcggcagcacaagaggctatgacgaactggtgccccaccagatttccgtggtgtccgaggaacggttctacaccaagtggaaccccgaggctctgcccagcaataccggcgaagtgaatttccagagcggcatcattgccgccagatgcgccatcagcaagctgcaccaagaactgggcgccaagggcttcattcaggtgtacgtggaccaggtcgacgaggacattgtggccgtgacaagacacagccccagcatccatcagagcgtggtggctgtgaccagaaccgccttcagaaaccccaagaccagcttctacagcaaagaggtgccccagatgtgcatccccggcaagattgaggaagtggtgctcgaggcccggaccatcgagagaaacaccaagccttaccggaaggacgagaactccatcaacggcacccctgacatcaccgtggaaatcagagagcacatccagctcaacgagagcaagatcgtgaaacaggccggcgtggccacaaagggccccaacgagtatatccaagagattgagttcgagaatctgagccccggcagcgtgatcatcttcagagtgtccctggatcctcacgctcaggtggccgtgggcatcctgagaaatcacctgacacagttcagcccacacttcaagagcggaagcctggccgtggacaacgccgatcctatcctgaagatccccttcgcctctctgcctcatttttccagcggcatcttccggtgttggggcagagacacctttattgccctgagaggcatcctgctgattaccggcagatacgtggaagcccggaacatcatcctggcctttgccggcacactgcggcacggactgattcctaatctgctcggcgagggcatctacgccagatacaactgcagagatgccgtgtggtggtggctccagtgcatccaggactactgcaagatggtgcccaacggcctggacatcctgaagtgccctgtgtccagaatgtaccctaccgacgatagcgcccctctgcctgccggaacacttgaccagcctctgttcgaagtgattcaagaggccatgcagaaacacatgcagggaatccagtttcgcgagcggaatgccggacctcagatcgacagaaacatgaaggatgagggcttcaacatcaccgctggcgtggacgaagagacaggctttgtgtacggcggcaaccggttcaattgcggcacctggatggacaagatgggcgagtctgaccgggccagaaacagaggaattcccgccacacctagagatggcagcgctgtggaaatcgtgggcctgtctaagtctgctgtgcggtggctgctcgaactgagcaagaagaatatctttccgtaccacgaagtgaccgtgaagcggcacggcaaggccatcaaggtgtcctacgacgagtggaacagaaagatccaggacaacttcgaaaagctgttccatgtgtctgaggaccccagcgacctgaacgaaaagcaccccaacctggtgcacaagcgcggcatctacaaggacagctacggcgcctcttctccttggtgcgattaccagctgcggcccaacttcaccattgccatggtggttgcccctgagctgttcaccacagagaaggcctggaaggccctggaaatcgccgagaagaaactgctgggccctctgggcatgaagacactggaccccgacgacatggtgtactgcggaatctacgacaacgccctggataacgacaactacaatctggccaaggggttcaattaccatcagggacccgagtggctgtggcctatcggctatttcctgcgggccaagctgtacttctccagactgatgggccctgagacaaccgccaagacaatcgtgctcgtgaagaacgtgctgagccggcactatgtgcacctggaaagaagcccctggaagggactgcccgagctgaccaatgagaacgcccagtactgccccttcagctgcgaaacacaggcctggtctatcgccaccatcctggaaaccctgtacgacctgtga

SEQ ID NO: 26 - DNA, 3942 bp, artificial
  Nucleic acid sequence encoding D5 hGDE
atgggacacagtaaacagattcgaattttacttctgaacgaaatggagaaactggaaaagaccctcttcagacttgaacaagggtatgagctacagttccgattaggcccaactttacagggaaaagcagttaccgtgtatacaaattacccatttcctggagaaacatttaatagagaaaaattccgttctctggattgggaaaatccaacagaaagagaagatgattctgataaatactgtaaacttaatctgcaacaatctggttcatttcagtattatttccttcaaggaaatgagaaaagtggtggaggttacatagttgtggaccccattttacgtgttggtgctgataatcatgtgctacccttggactgtgttactcttcagacatttttagctaagtgtttgggaccttttgatgaatgggaaagcagacttagggttgcaaaagaatcaggctacaacatgattcattttaccccattgcagactcttggactatctaggtcatgctactcccttgccaatcagttagaattaaatcctgacttttcaagacctaatagaaagtatacctggaatgatgttggacagctagtggaaaaattaaaaaaggaatggaatgttatttgtattactgatgttgtctacaatcatactgctaataggcgagtaaccaagtctgatccaaaccaacaccttacgattattcaagatcctgaatacagacggtttggctgtactgtagatatgaacattgcactaacgactttcataccatattttactttcccatttgaagagatagacttctccatggaagaatctatgattcatctgccaaataaagcttgttttctgatggcacacaatggatgggtaatgggagatgatcctcttcgaaactttgctgaaccgggttcagaagtttacctaaggagagaacttatttgctggggagacagtgttaaattacgctatgggaataaaccagaggactgtccttatctctgggcacacatgaaaaaatacactgaaataactgcaacttatttccagggagtacgtcttgataactgccactcaacacctcttcacgtagctgagtacatgttggatgctgctaggaatttgcaacccaatttatatgtagtagctgaactgttcacaggaagtgaggacctagacaatgtctttgttactagactgggcattagttccttaataagagaggcaatgagtgcatataatagtcatgaagagggcagattagtttaccgatatggaggagaacctgttggatcctttgttcagccctgtttgaggcctttaatgccagctattgcacatgccctgtttatggatattacgcatgataatgagtgtcctattgtgcatagatcagcgtatgatgctcttccaagtactacaattgtttctatggcatgttgtgctagtggaagtacaagaggctatgatgaattagtgcctcatcagatttatgtggatcaagttgatgaagacatagtggcagtaacaagacactcacctagcatccatcagtctgttgtggctgtaactagaactgctttcaggaatcccaagacttcattttacagcaaggaagtgcctcaaatgtgcatccctggcaaaattgaagaagtagttcttgaagctagaactattgagagaaacacgaaaccttataggaaggatgaaaattcaatcaatggaacaccagatatcacagtagaaattagagaacatattcagcttaatgaaagtaaaattgttaaacaagctggagttgccacaaaagggcccaatgaatatattcaagaaatagaatttgaaaacttgtctccaggaagtgttattatattcagagttagtcttgatccacatgcacaagtcgctgttggcattcttcgaaatcatctgacacaattcagtcctcactttaaatctggcagcctagctgttgacaatgcagatcctatattaaaaattccttttgcttctcttgcctatagattaactttggctgagctaaatcagatcctttaccgatgtgaatcagaagaaaaggaagatggtggagggtgctatgacataccaaactggtcagcccttaaatatgcaggtcttcaaggtttaatgtctgtattggcagaaataagaccaaagaatgacttggggcatcctttttgtaataatttgaggtctggagattggatgattgactatgtcagtaaccggcttatttcacgatcaggaactattgctgaagttggtaaatggttgcaggctatgttcttctacctgaagcagatcccacgttaccttatcccatgttactttgatgctatattaattggtgcatataccactcttctggatacagcatggaagcagatgtcaagctttgttcagaatggttcaacctttgtgaaacacctttcattgggttcagttcaactgtgtggagtaggaaaattcccttccctgccaattctttcacctgccctaatggatgtaccttataggttaaatgagatcacaaaagaaaaggagcaatgttgtgtttctctagctgcaggcttacctcatttttcttctggtattttccgctgctggggaagggatacttttattgcacttagaggtatactgctgattactggacgctatgtagaagccaggaatattattttagcatttgcgggtaccctgaggcatggtctcattcctaatctactgggtgaaggaatttatgccagatacaattgtcgggatgctgtgtggtggtggctgcagtgtatccaggattactgtaaaatggttccaaatggactagacattctcaagtgcccagtttccagaatgtatcctacagatgattctgctcctttgcctgctggcacactggatcagccattgtttgaagtcatacaggaagcaatgcaaaaacacatgcagggcatacagttccgagaaaggaatgctggtccccagatagatcgaaacatgaaggacgaaggttttaatataactgcaggagttgatgaagaaacaggatttgtttatggaggaaatcgtttcaattgtggcacatggatggataaaatgggagaaagtgacagagctagaaacagaggaatcccagccacaccaagagatgggtctgctgtggaaattgtgggcctgagtaaatctgctgttcgctggttgctggaattatccaaaaaaaatattttcccttatcatgaagtcacagtaaaaagacatggaaaggctataaaggtctcatatgatgagtggaacagaaaaatacaagacaactttgaaaagctatttcatgtttccgaagacccttcagatttaaatgaaaagcatccaaatctggttcacaaacgtggcatatacaaagatagttatggagcttcaagtccttggtgtgactatcagctcaggcctaattttaccatagcaatggttgtggcccctgagctctttactacagaaaaagcatggaaagctttggagattgcagaaaaaaaattgcttggtccccttggcatgaaaactttagatccagatgatatggtttactgtggaatttatgacaacgcattagacaatgacaactacaatcttgctaaaggtttcaattatcaccaaggacctgagtggctgtggcctattgggtattttcttcgtgcaaaattatatttttccagattgatgggcccggagactactgcaaagactatagttttggttaaaaatgttctttcccgacattatgttcatcttgagagatccccttggaaaggacttccagaactgaccaatgagaatgcccagtactgtcctttcagctgtgaaacacaagcctggtcaattgctactattcttgagacactttatgatttatag

SEQ ID NO: 27 - DNA, 3759 bp, artificial
  Nucleic acid sequence encoding D6 hGDE
atgaactccatccgaaaaataatttgggaggatatttttccaaagcttaaactctgggaatttttccaagtagatgtcaacaaagcggttgagcaatttagaagacttcttacacaagaaaataggcgagtaaccaagtctgatccaaaccaacaccttacgattattcaagatcctgaatacagacggtttggctgtactgtagatatgaacattgcactaacgactttcataccacatgacaaggggccagcagcaattgaagaatgctgtaattggtttcataaaagaatggaggaattaaattcagagaagcatcgactcattaactatcatcaggaacaggcagttaattgccttttgggaaatgtgttttatgaacgactggctggccatggtccaaaactaggacctgtcactagaaagcatcctttagttaccaggtattttactttcccatttgaagagatagacttctccatggaagaatctatgattcatctgccaaataaagcttgttttctgatggcacacaatggatgggtaatgggagatgatcctcttcgaaactttgctgaaccgggttcagaagtttacctaaggagagaacttatttgctggggagacagtgttaaattacgctatgggaataaaccagaggactgtccttatctctgggcacacatgaaaaaatacactgaaataactgcaacttatttccagggagtacgtcttgataactgccactcaacacctcttcacgtagctgagtacatgttggatgctgctaggaatttgcaacccaatttatatgtagtagctgaactgttcacaggaagtgaggacctagacaatgtctttgttactagactgggcattagttccttaataagagaggcaatgagtgcatataatagtcatgaagagggcagattagtttaccgatatggaggagaacctgttggatcctttgttcagccctgtttgaggcctttaatgccagctattgcacatgccctgtttatggatattacgcatgataatgagtgtcctattgtgcatagatcagcgtatgatgctcttccaagtactacaattgtttctatggcatgttgtgctagtggaagtacaagaggctatgatgaattagtgcctcatcagatttcagtggtttctgaagaacggttttacactaagtggaatcctgaagcattgccttcaaacacaggtgaagttaatttccaaagcggcattattgcagccaggtgtgctatcagtaaacttcatcaggagcttggagccaagggttttattcaggtgtatgtggatcaagttgatgaagacatagtggcagtaacaagacactcacctagcatccatcagtctgttgtggctgtaactagaactgctttcaggaatcccaagacttcattttacagcaaggaagtgcctcaaatgtgcatccctggcaaaattgaagaagtagttcttgaagctagaactattgagagaaacacgaaaccttataggaaggatgaaaattcaatcaatggaacaccagatatcacagtagaaattagagaacatattcagcttaatgaaagtaaaattgttaaacaagctggagttgccacaaaagggcccaatgaatatattcaagaaatagaatttgaaaacttgtctccaggaagtgttattatattcagagttagtcttgatccacatgcacaagtcgctgttggcattcttcgaaatcatctgacacaattcagtcctcactttaaatctggcagcctagctgttgacaatgcagatcctatattaaaaattccttttgcttctcttgcctatagattaactttggctgagctaaatcagatcctttaccgatgtgaatcagaagaaaaggaagatggtggagggtgctatgacataccaaactggtcagcccttaaatatgcaggtcttcaaggtttaatgtctgtattggcagaaataagaccaaagaatgacttggggcatcctttttgtaataatttgaggtctggagattggatgattgactatgtcagtaaccggcttatttcacgatcaggaactattgctgaagttggtaaatggttgcaggctatgttcttctacctgaagcagatcccacgttaccttatcccatgttactttgatgctatattaattggtgcatataccactcttctggatacagcatggaagcagatgtcaagctttgttcagaatggttcaacctttgtgaaacacctttcattgggttcagttcaactgtgtggagtaggaaaattcccttccctgccaattctttcacctgccctaatggatgtaccttataggttaaatgagatcacaaaagaaaaggagcaatgttgtgtttctctagctgcaggcttacctcatttttcttctggtattttccgctgctggggaagggatacttttattgcacttagaggtatactgctgattactggacgctatgtagaagccaggaatattattttagcatttgcgggtaccctgaggcatggtctcattcctaatctactgggtgaaggaatttatgccagatacaattgtcgggatgctgtgtggtggtggctgcagtgtatccaggattactgtaaaatggttccaaatggactagacattctcaagtgcccagtttccagaatgtatcctacagatgattctgctcctttgcctgctggcacactggatcagccattgtttgaagtcatacaggaagcaatgcaaaaacacatgcagggcatacagttccgagaaaggaatgctggtccccagatagatcgaaacatgaaggacgaaggttttaatataactgcaggagttgatgaagaaacaggatttgtttatggaggaaatcgtttcaattgtggcacatggatggataaaatgggagaaagtgacagagctagaaacagaggaatcccagccacaccaagagatgggtctgctgtggaaattgtgggcctgagtaaatctgctgttcgctggttgctggaattatccaaaaaaaatattttcccttatcatgaagtcacagtaaaaagacatggaaaggctataaaggtctcatatgatgagtggaacagaaaaatacaagacaactttgaaaagctatttcatgtttccgaagacccttcagatttaaatgaaaagcatccaaatctggttcacaaacgtggcatatacaaagatagttatggagcttcaagtccttggtgtgactatcagctcaggcctaattttaccatagcaatggttgtggcccctgagctctttactacagaaaaagcatggaaagctttggagattgcagaaaaaaaattgcttggtccccttggcatgaaaactttagatccagatgatatggtttactgtggaatttatgacaacgcattagacaatgacaactacaatcttgctaaaggtttcaattatcaccaaggacctgagtggctgtggcctattgggtattttcttcgtgcaaaattatatttttccagattgatgggcccggagactactgcaaagactatagttttggttaaaaatgttctttcccgacattatgttcatcttgagagatccccttggaaaggacttccagaactgaccaatgagaatgcccagtactgtcctttcagctgtgaaacacaagcctggtcaattgctactattcttgagacactttatgatttatag

SEQ ID NO: 28 - DNA, 3327 bp, artificial
  Nucleic acid sequence encoding D7 hGDE
atggttaccaggtattttactttcccatttgaagagatagacttctccatggaagaatctatgattcatctgccaaataaagcttgttttctgatggcacacaatggatgggtaatgggagatgatcctcttcgaaactttgctgaaccgggttcagaagtttacctaaggagagaacttatttgctggggagacagtgttaaattacgctatgggaataaaccagaggactgtccttatctctgggcacacatgaaaaaatacactgaaataactgcaacttatttccagggagtacgtcttgataactgccactcaacacctcttcacgtagctgagtacatgttggatgctgctaggaatttgcaacccaatttatatgtagtagctgaactgttcacaggaagtgaggacctagacaatgtctttgttactagactgggcattagttccttaataagagaggcaatgagtgcatataatagtcatgaagagggcagattagtttaccgatatggaggagaacctgttggatcctttgttcagccctgtttgaggcctttaatgccagctattgcacatgccctgtttatggatattacgcatgataatgagtgtcctattgtgcatagatcagcgtatgatgctcttccaagtactacaattgtttctatggcatgttgtgctagtggaagtacaagaggctatgatgaattagtgcctcatcagatttcagtggtttctgaagaacggttttacactaagtggaatcctgaagcattgccttcaaacacaggtgaagttaatttccaaagcggcattattgcagccaggtgtgctatcagtaaacttcatcaggagcttggagccaagggttttattcaggtgtatgtggatcaagttgatgaagacatagtggcagtaacaagacactcacctagcatccatcagtctgttgtggctgtaactagaactgctttcaggaatcccaagacttcattttacagcaaggaagtgcctcaaatgtgcatccctggcaaaattgaagaagtagttcttgaagctagaactattgagagaaacacgaaaccttataggaaggatgaaaattcaatcaatggaacaccagatatcacagtagaaattagagaacatattcagcttaatgaaagtaaaattgttaaacaagctggagttgccacaaaagggcccaatgaatatattcaagaaatagaatttgaaaacttgtctccaggaagtgttattatattcagagttagtcttgatccacatgcacaagtcgctgttggcattcttcgaaatcatctgacacaattcagtcctcactttaaatctggcagcctagctgttgacaatgcagatcctatattaaaaattccttttgcttctcttgcctatagattaactttggctgagctaaatcagatcctttaccgatgtgaatcagaagaaaaggaagatggtggagggtgctatgacataccaaactggtcagcccttaaatatgcaggtcttcaaggtttaatgtctgtattggcagaaataagaccaaagaatgacttggggcatcctttttgtaataatttgaggtctggagattggatgattgactatgtcagtaaccggcttatttcacgatcaggaactattgctgaagttggtaaatggttgcaggctatgttcttctacctgaagcagatcccacgttaccttatcccatgttactttgatgctatattaattggtgcatataccactcttctggatacagcatggaagcagatgtcaagctttgttcagaatggttcaacctttgtgaaacacctttcattgggttcagttcaactgtgtggagtaggaaaattcccttccctgccaattctttcacctgccctaatggatgtaccttataggttaaatgagatcacaaaagaaaaggagcaatgttgtgtttctctagctgcaggcttacctcatttttcttctggtattttccgctgctggggaagggatacttttattgcacttagaggtatactgctgattactggacgctatgtagaagccaggaatattattttagcatttgcgggtaccctgaggcatggtctcattcctaatctactgggtgaaggaatttatgccagatacaattgtcgggatgctgtgtggtggtggctgcagtgtatccaggattactgtaaaatggttccaaatggactagacattctcaagtgcccagtttccagaatgtatcctacagatgattctgctcctttgcctgctggcacactggatcagccattgtttgaagtcatacaggaagcaatgcaaaaacacatgcagggcatacagttccgagaaaggaatgctggtccccagatagatcgaaacatgaaggacgaaggttttaatataactgcaggagttgatgaagaaacaggatttgtttatggaggaaatcgtttcaattgtggcacatggatggataaaatgggagaaagtgacagagctagaaacagaggaatcccagccacaccaagagatgggtctgctgtggaaattgtgggcctgagtaaatctgctgttcgctggttgctggaattatccaaaaaaaatattttcccttatcatgaagtcacagtaaaaagacatggaaaggctataaaggtctcatatgatgagtggaacagaaaaatacaagacaactttgaaaagctatttcatgtttccgaagacccttcagatttaaatgaaaagcatccaaatctggttcacaaacgtggcatatacaaagatagttatggagcttcaagtccttggtgtgactatcagctcaggcctaattttaccatagcaatggttgtggcccctgagctctttactacagaaaaagcatggaaagctttggagattgcagaaaaaaaattgcttggtccccttggcatgaaaactttagatccagatgatatggtttactgtggaatttatgacaacgcattagacaatgacaactacaatcttgctaaaggtttcaattatcaccaaggacctgagtggctgtggcctattgggtattttcttcgtgcaaaattatatttttccagattgatgggcccggagactactgcaaagactatagttttggttaaaaatgttctttcccgacattatgttcatcttgagagatccccttggaaaggacttccagaactgaccaatgagaatgcccagtactgtcctttcagctgtgaaacacaagcctggtcaattgctactattcttgagacactttatgatttatag

SEQ ID NO: 29 - DNA, 3912 bp, artificial
  Nucleic acid sequence encoding D8 hGDE
atgcatccagaatgtgcctataatcttgtaaattctccacacttaaaacctgcctgggtcttagacagagcactttggcgtttctcctgtgatgttgcagaagggaaatacaaagaaaagggaatacctgctttgattgaaaatgatcaccatatgaactccatccgaaaaataatttgggaggatatttttccaaagcttaaactctgggaatttttccaagtagatgtcaacaaagcggttgagcaatttagaagacttcttacacaagaaaataggcgagtaaccaagtctgatccaaaccaacaccttacgattattcaagatcctgaatacagacggtttggctgtactgtagatatgaacattgcactaacgactttcataccacatgacaaggggccagcagcaattgaagaatgctgtaattggtttcataaaagaatggaggaattaaattcagagaagcatcgactcattaactatcatcaggaacaggcagttaattgccttttgggaaatgtgttttatgaacgactggctggccatggtccaaaactaggacctgtcactagaaagcatcctttagttaccaggtattttactttcccatttgaagagatagacttctccatggaagaatctatgattcatctgccaaataaagcttgttttctgatggcacacaatggatgggtaatgggagatgatcctcttcgaaactttgctgaaccgggttcagaagtttacctaaggagagaacttatttgctggggagacagtgttaaattacgctatgggaataaaccagaggactgtccttatctctgggcacacatgaaaaaatacactgaaataactgcaacttatttccagggagtacgtcttgataactgccactcaacacctcttcacgtagctgagtacatgttggatgctgctaggaatttgcaacccaatttatatgtagtagctgaactgttcacaggaagtgaggacctagacaatgtctttgttactagactgggcattagttccttaataagagaggcaatgagtgcatataatagtcatgaagagggcagattagtttaccgatatggaggagaacctgttggatcctttgttcagccctgtttgaggcctttaatgccagctattgcacatgccctgtttatggatattacgcatgataatgagtgtcctattgtgcatagatcagcgtatgatgctcttccaagtactacaattgtttctatggcatgttgtgctagtggaagtacaagaggctatgatgaattagtgcctcatcagatttcagtggtttctgaagaacggttttacactaagtggaatcctgaagcattgccttcaaacacaggtgaagttaatttccaaagcggcattattgcagccaggtgtgctatcagtaaacttcatcaggagcttggagccaagggttttattcaggtgtatgtggatcaagttgatgaagacatagtggcagtaacaagacactcacctagcatccatcagtctgttgtggctgtaactagaactgctttcaggaatcccaagacttcattttacagcaaggaagtgcctcaaatgtgcatccctggcaaaattgaagaagtagttcttgaagctagaactattgagagaaacacgaaaccttataggaaggatgaaaattcaatcaatggaacaccagatatcacagtagaaattagagaacatattcagcttaatgaaagtaaaattgttaaacaagctggagttgccacaaaagggcccaatgaatatattcaagaaatagaatttgaaaacttgtctccaggaagtgttattatattcagagttagtcttgatccacatgcacaagtcgctgttggcattcttcgaaatcatctgacacaattcagtcctcactttaaatctggcagcctagctgttgacaatgcagatcctatattaaaaattccttttgcttctcttgcctatagattaactttggctgagctaaatcagatcctttaccgatgtgaatcagaagaaaaggaagatggtggagggtgctatgacataccaaactggtcagcccttaaatatgcaggtcttcaaggtttaatgtctgtattggcagaaataagaccaaagaatgacttggggcatcctttttgtaataatttgaggtctggagattggatgattgactatgtcagtaaccggcttatttcacgatcaggaactattgctgaagttggtaaatggttgcaggctatgttcttctacctgaagcagatcccacgttaccttatcccatgttactttgatgctatattaattggtgcatataccactcttctggatacagcatggaagcagatgtcaagctttgttcagaatggttcaacctttgtgaaacacctttcattgggttcagttcaactgtgtggagtaggaaaattcccttccctgccaattctttcacctgccctaatggatgtaccttataggttaaatgagatcacaaaagaaaaggagcaatgttgtgtttctctagctgcaggcttacctcatttttcttctggtattttccgctgctggggaagggatacttttattgcacttagaggtatactgctgattactggacgctatgtagaagccaggaatattattttagcatttgcgggtaccctgaggcatggtctcattcctaatctactgggtgaaggaatttatgccagatacaattgtcgggatgctgtgtggtggtggctgcagtgtatccaggattactgtaaaatggttccaaatggactagacattctcaagtgcccagtttccagaatgtatcctacagatgattctgctcctttgcctgctggcacactggatcagccattgtttgaagtcatacaggaagcaatgcaaaaacacatgcagggcatacagttccgagaaaggaatgctggtccccagatagatcgaaacatgaaggacgaaggttttaatataactgcaggagttgatgaagaaacaggatttgtttatggaggaaatcgtttcaattgtggcacatggatggataaaatgggagaaagtgacagagctagaaacagaggaatcccagccacaccaagagatgggtctgctgtggaaattgtgggcctgagtaaatctgctgttcgctggttgctggaattatccaaaaaaaatattttcccttatcatgaagtcacagtaaaaagacatggaaaggctataaaggtctcatatgatgagtggaacagaaaaatacaagacaactttgaaaagctatttcatgtttccgaagacccttcagatttaaatgaaaagcatccaaatctggttcacaaacgtggcatatacaaagatagttatggagcttcaagtccttggtgtgactatcagctcaggcctaattttaccatagcaatggttgtggcccctgagctctttactacagaaaaagcatggaaagctttggagattgcagaaaaaaaattgcttggtccccttggcatgaaaactttagatccagatgatatggtttactgtggaatttatgacaacgcattagacaatgacaactacaatcttgctaaaggtttcaattatcaccaaggacctgagtggctgtggcctattgggtattttcttcgtgcaaaattatatttttccagattgatgggcccggagactactgcaaagactatagttttggttaaaaatgttctttcccgacattatgttcatcttgagagatccccttggaaaggacttccagaactgaccaatgagaatgcccagtactgtcctttcagctgtgaaacacaagcctggtcaattgctactattcttgagacactttatgatttatag

SEQ ID NO: 30 - DNA, 4134 bp, Equus caballus
atgattcattttacaccattgcagactcttggactatctaggtcatcctactcccttgctgaccagttagaattaaatcctgacttttcaagacctaataaaaagtatacctggcatgatgttggacagctagtggaaaaattgaaaaaggaatgggatattctttgtattactgatgttgtctacaatcatactgctgctaatagtaaatggatccatgaacatccagaaagtgcatataaccttgtgaattctccacacttaaaacctgcctgggtcttagacagagcactttggcatttatcctgtgatgtggcagaagggaaatacagagaaaaaggagtacctgctctgattgaaaatgatcatcaaatgaattgcattcgaaaaataatttgggaggatatttatccaaagattcacctctgggaatttttccaagtagacgttcacaaagcagttgagcaatttagaggacttcttacacaagaaaataggaaaataatatctcagcctgatccaaagcaacaccttaagattattcaggatcctgaatacagacggcttggctgtactgtagatatgaacattgcactagcaactttcataccacatgataatgggccagctgcaattgatgaatgctgtaattggttccgtaagagaattgaggaattaaacgcagagaagcatcaacttgtgaactatcatcaggagcaggcagttaattgccttttgggaaatgtattttatgaacgactggctggccatggtcctaaactaggacctgtcaccagaaaacatcctttagttaccagatattttactttcccatttgaagaaatgaccccatccacagaagaatctatgattcatctcccaaataaagcttgttttctgatggcgcataatggatgggtaatgggagatgatccccttcggaactttgctgaaccaggttcagacgtttatctaaggagagaacttatctgctggggagacagtgttaaattacgctatgggaataagccagaggactgtccttacctctgggcgcacatgaaaaaatacactgaaataactgcaactcatttccagggagtacgtcttgataactgccactcaacaccaattcatgtagccgagtacatgttggatgccgctaggaaattgcaacccaatttatatgtagtagctgaactgttcacaggaagcgaagacctggacaatatctttgttactagactgggcattagttccttaataagagaggcaatgagtgcagctgatagccatgaggagggcagattagtttaccgatatggaggagagcctgttgggtcctttgttcagccctgtttgaggcctttaatgccagctattgcacatgccctgtttatggatatcacccatgataatgagtgtcctattgtgcataggtcagcatatgatgctctcccgagttccacgattgtttctatggcatcttgtgctagtggaagtactaaaggctatgatgaattagtgcctcatcagatttcagtggtttctgaagaacgattttatactaagtggaatcctgaagcattgccatcaaatacaggtgaagtcaatttccaaagcggaattattgcagccaggcgtgctatcaataaacttcatcaagagcttggggccaagggtttcattcaggtgtatgtggatcaggttgatcaagatatagtggcggtaacaaggcactcacctagcatccatcagtctgttgtgtctgtgtcgagaactgctttcaggaatcccaagacgtcattttacagcaaggaagtgcctcatatgtacatccctggcaaaattgaagaagtagttcttgaagctagaactattgagagacatacaataccttataagaaggatgaaaactcaatcaatggaatgccagatatcacagtagaaattagagaacatattcagcttaatgaaagtaaaattgttaaacatgctggaattgtcacaaaaggacccaatgaatttgttcaagaaatagagtttgaaaacttgactccaggaagtgttattatattcagagttagtcttgatccacatgcacaagttgctgttggaattcttcgaaatcatctgacacaattcagtcctcactttaaatctgggagccttgctgttgacaacgcagatcctatattgaaaattccttttgcttctattgcctctaaattaactttggctgagctaaatcaggtcctttatcgatgtgaatcagaagaacaagaagatggtggagggtgttataacataccaaactggtcgtctcttaaatatgcaggtcttcaaggattaatgtccatattggcagaaataagaccaaggaatgacttggggcatcccttttgtgacaatttgagatctggagattggatgattgactatgtcagtagccggcttatttcacgatcaggaactattgctgaagttggtaaatggttgcaggctatgttcctctacctgaagcagatcccccgttatcttattccatgttactttgatgctatattaattggtgcatacaccactctcctggatatagcatggaagcagatgtcaagctttgttcagaatggttctacctttgtgaaacacctttctctgggttcagtccaaatgtgtggagtaggaaaattcccttctctgccacttctttcaccttcccttacggatctaccatatagagtaaatgagatcacaaaagaaaaggagcagtgttgtgggtctctagctgcaggcttacctcatttttctgctggcattttccgctgctggggaagggataccttcattgcgctcagaggtctgctgctggttacgggacgctatttggaggccaggaatattattttagcatttgctggcaccctgagacacggtctcattcctaatctcctgggtgaaggaactcacgccagatacaattgccgggatgctgtgtggtggtggctacagtgtattcaggattactgtaaaattgttccaaatggcctggacatcctcaggtgcccggtttccagaatgtatcctacagatgattctgttcctttgtctgctggcacagtggatcaaccattgtttgaagtaatacaggaagctatgcaaagacatgtgcagggcatacagttccgagaaaggaatgctggtccacagatagatcgaaacatgaaggatgaaggttttaatataactgcaggagttgatgaagaaacgggatttgtttatggaggaaatcgcttcaattgcggcacatggatggataaaatgggagaaagtgacagagctagaaacagaggaatcccggccactccaagagatgggtctgctgtggaaattgtgggcctgagtaaatctgccgttcgttggttgctggaattatcccgaaaaaatattttcccttatcatgaagtccgagtaaaaagacatggaaagtttgtgacagtctcatatgatgagtggaacagaaaaatacaagacaactttgaaaagctatttcatgtgtcagaagacccttcagattttaacgaaaagcatcctgagctggttcacaaacgtggcatatacaaagatagttatggagcatcaagcccttggtgtgactaccagctcaggcctaattttaccatagcaatggtcgtagcccctgagctgtttaccccagaaaaagcatggaaagctttggagattgcagaaaaaaaattgcttggtccccttggcatgaaaactttggatccagatgatatggtttactgtggaatttatgacaatgccttagacaatgacaactacaatcttgctaaaggtttcaattatcaccaaggacctgagtggctgtggcccactggatattttcttcgtgcaaaattgtatttttccaaattaatgggtccagagactaatgcaaagactatgtttttggttaaaaacgtcctttccagacattatgttcatcttgagagatccccttggaaaggacttccagaactgactaatgagaatggccaatactgtcctttcagctgtgaaacacaagcctggtcaattgctactgttcttgaaacactctatgacttatag

SEQ ID NO: 31 - DNA, 4098 bp, Gorilla gorilla
atgggacacagtaaacagattcgaattttacttctgaacgaaatggagaaactggaaaagaccctcttcagacttgaacaagggtatgaactacagttccgattaggcccaactttacagggaaaagcagttaccgtgtatacaaattacccatttcctggagaaacatttaatagagaaaaattccgttctctggattgggaaaatccaacagaaagagaagatgattctgataaatactgtaaacttaatctgcaacaatctggttcatttcagtattatttccttcaaggaaatgagaaaagtggtggaggttacatagttgtggaccccattttacgtgttggtgctgataatcatgtgctacccttggactgtgttactcttcagacatttttagctaagtgtttgggaccttttgatgaatgggaaagcagacttagggttgcaaaagaatcaggctacaacatgattcattttaccccattgcagactcttggactatctaggtcatgctactcccttgccaatcagttagaattaaatcctgacttttcaagacctaatagaaagtatacctggaatgatgttggacagctagtggaaaaattaaaaaaggaatggaatgttatttgtattactgatgttgtctacaatcatactgctgctaatagtaaatggatccaggaacatccagaatgtgcctataatcttgtgaattctccacacttaaaacctgcctgggtcttagacagagcactttggcgtttctcctgtgatgttgcagaagggaaatacaaagaaaagggaatacctgctttgattgaaaatgatcaccatatgaattccatccgaaaaataatttgggaggatatttttccaaagcttaaactctgggaatttttccaagtagatgtcaacaaagcggttgagcaatttagaagacttcttacacaagaaaataggcgagtaaccaagtctgatccaaaccaacatcttacgattattcaagatcctgaatacagacggtttggctgtactgtagatatgaacattgcactaacgactttcataccacatgagtattttactttcccatttgaagagatagacttctccatggaagaatctatgattcatctcccaaataaagcttgttttctgatggcacacaatggatgggtaatgggagatgatcctcttcgaaactttgctgaaccgggttcagaagtttacctaaggagagaacttatttgctggggagacagtgttaaattacgctatgggaataaaccagaggactgtccttatctctgggcacacatgaaaaaatacactgaaataactgcaacttatttccagggagtacgtcttgataactgccactcaacacctcttcacgtagctgagtacatgttggatgctgctaggaatttgcaacccaatttatatgtagtagctgaactgttcacaggaagtgaagatctggacaatgtctttgttactagactgggcattagttccttaataagagaggcaatgagtgcatataatagtcatgaagagggcagattagtttaccgatatggaggagaacctgttggatcctttgttcagccctgtttgaggcctttaatgccagctattgcacatgccctgtttatggatattacgcatgataatgagtgtcctattgtgcatagatcagcgtatgatgctcttccaagtactacaattgtctctatggcgtgttgtgctagtggaagtacaagaggctatgatgaattagtgcctcatcagttcctaggcaaaattgaagaagtagttcttgaagctagaactattgagagaaacatgaaaccttataggaaggatgagaattcaatcaatggaacgccagatatcacagtagaaattagagaacatattcagcttaatgaaagtaaaattgttaaacaagctggagttgccacaaaagggcccaatgaatatattcaagaaatagaatttgaaaacttgtctccaggaagtgttattatattcagagttagtcttgatccacatgcacaagtcgctgttggaattcttcgaaatcatctgacacaattcagtcctcactttaaatctggcagcctagctgttgacaatgcagatcctatattaaaaattccttttgcttctattgcctccagattaactttggctgagctaaatcagatcctttaccgatgtgaatcagaagaaaaggaagatggtggagggtgctatgacataccaaactggtcagcccttaaatatgcaggtcttcaaggtttaatgtctgtattggcagaaataagaccaaagaatgacttggggcatcctttttgtaataatttgagatctggagattggatgattgactatgtcagtaaccggcttatttcacgatcaggaactattgctgaagttggtaaatggttgcaggctatgttcttctacctgaagcagatcccacgttaccttatcccatgttactttgatgctatattaattggtgcatataccactcttctggatacagcatggaagcagatgtcaagctttgttcagaatggttcaacctttgtgaaacacctttcattgggttcagttcaactgtgtggagtaggaaaattcccttccctgccaattctttcacctgccctaatggatgtaccttataggttaaatgagatcacaaaagaaaaggagcaatgttgtgtttctctagctgcaggcttacctcatttttcttctggtattttccgctgctggggaagggatacttttattgcacttagaggtatactgctgattactggacgctatgtagaagccaggaatattattttagcatttgcgggtaccctgaggcatggtctcattcctaatctactgggtgaaggaatttatgccagatacaattgtcgggatgctgtgtggtggtggctgcagtgtatccaggattactgtaaaatggttccaaatggtgtagacattctcaagtgcccagtttccagaatgtatcctacagatgattctgctcctttgcctgctggcacactggatcagccattgtttgaagtcatacaggaagcaatgcaaaaacacatgcagggcatacagttccgagaaaggaatgctggtccccagatagatcgaaacatgaaggacgaaggttttaatataactgcaggagttgatgaagaaacaggatttgtttatggaggaaatcgtttcaattgtggcacatggatggataaaatgggagaaagtgacagagctagaaacagaggaatcccagccacaccaagagatgggtctgctgtggaaattgtgggcctgagtaaatctgctgttcgctggttgctggaattatccaaaaaaaatattttcccttatcatgaagtcacagtaaaaagacatggaaaggctataaaggtctcatatgatgagtggaacagaaaaatacaagacaactttgaaaagctatttcatgtttcagaagacccttcagatttaaatgaaaagcatccaaatctggttcacaaacgtggcatatacaaagatagttatggagcgtcaagtccttggtgtgactatcagctcaggcctaattttaccatagcaatggttgtggcccctgagctctttactacagaaaaagcatggaaagctttggagattgcagaaaaaaaattgcttggtccccttggcatgaaaactttagatccagatgatatggtttactgtggaatttatgacaatgcattagacaatgacaactacaatcttgctaaaggtttcaattatcaccaaggacctgagtggctgtggcctattgggtattttcttcgtgcaaaattatatttttccagattgatgggcccggagactactgcaaagactatagttttggttaaaaatgttctttcccgacattatgttcatcttgagagatccccttggaaaggacttccagaactgaccaatgagaatgcccagtactgtcctttcagctgtgaaacacaagcctggtcaattgctactattcttgagacactttatgatttgtag

SEQ ID NO: 32 - DNA, 3900 bp, Pongo abelii
atggggcacagtaaacagattcgaattttacttctgaacgaaatggagaagctggaaaagaccctcttcagacttgaacaagggtatgaactacagttccgattaggcccaactttacagggaaaagcagttaccgtgtatacaaattacccatttcctggagaaacatttaatagagaaaaattccgttctctggattgggaaaatccaacagaaagagaagatgattctgataaatactgcaaacttaatctgcaacaatctggttcatttcagtattatttccttcaaggaaatgagaaaagtggtggaggttacatagttgtggaccccattttacgtgttggtgccgataatcatgtgctacccttggactgtgttactcttcagacatttttagctaagtgtttgggaccttttgatgaatgggaaagcagacttagggttgcaaaagaatcaggctacaacatgattcattttaccccactgcagactcttggactatctaggtcatgctactcccttgccaatcagttagaattaaatcctgacttttcaagacctaatagaaagtatacctggaatgatgttggacagctagtggaaaaattaaaaaaggaatggaatgttatttgtattaccgatgttgtctacaatcatactgctgctaatagtaaatggatccaggaacatccagaatgtgcctataatcttgtgaattctccacacttaaaacctgcctgggtcttagacagagcactttggcgtttctcctgtgatgttgcagaagggaaatacaaagaaaagggaatacctgctttgattgaaaatgatcaccatatgaattccatccgaaaaataatttgggaggatatttttccaaagcttaaactctgggaatttttcgaagtagatgtcaacaaagcggttgagcaatttagaagacttcttacacaagaaaataggcgagtaaccaagtctgatccaaaccaacatcttacgattattcaggatcctgaatacagacggtttggctgtactgtagatatgaacattgcactaacgactttcataccacatgacaatgggccagcagcaattgaagagtgctgtaactggtttcgtaagagaattgaggaattaaattcagagaagcatcaactcattaactatcatcaggaacaggcagtgaattgccttttgggaaatgtgttttatgaacgactggctggccatggtccaaaactaggacctgtcactagaaagcatcctttagttaccaggtattttactttcccatttgaagagatggacttctccatggaagaatctatgattcatctcccaaataaagcttgtttactgatggcacacaatggatgggtaatgggagatgatcctcttcgaaactttgctgaaccgggttcagaagtttacctaaggagagaacttatttgctggggagacagtgttaaattacgctatgggaataaaccagaggactgtccttatctctgggcacacatgaaaaaatacactgaaataactgcaacttatttccagggagtacgtcttgataactgccactcaacacctcttcacgtagctgagtacatgttggatgctgctaggaatttgcaacccaatttatatgtagtagctgaactgttcacaggaagtgaagatctggacaatgtctttgttactagactgggcattagttccttaataagagaggcaatgagtgcatatgatagtcatgaagagggcagattagtttaccgatatggaggagaacctgttggatcctttgttcagccctgtttgaggcctttaatgccggctattgcacatgccctgtttatggatattacacatgataatgagtgtcctattgtgcatagatcagcgtatgatgctcttccaagtactacaattgtttctatggcgtgttgtgctagtggaagtacaagaggctatgatgaattagtgcctcatcagatttcggtggtttctgaagaacggttttacactaagtggaatcctgaagcattgccttcaaatacaggtgaagttaatttccaaagcggcattattgcagccaggtgtgctatcaataaacttcatcaggagcttggagccaagggttttattcaggtgtatgttgatcaagttgatgaagacatagtggcagtaacaagacactcacctagcatccatcagtctgttgtggctgtatctagaactgctttcaggaatcccaagacttcattttacagcaaggaagtgcctcaaatgtgcatccctggcaaaattgaagaagtagttcttgaagctagaactattgagagaaacacgaaaccttataggaaggatgagaattcaatcaatggaacgccagatatcacagtagaaattagagaacatattcagcttaatgaaagtaaaattgttaaacaagctggagttgccacaaaagggcccaatgaatttattcaagaaatagaatttgaaaacttgtctccaggaagtgttattatattcagagttagtcttgatccacatgcacaagtcgctgttggaattcttcgaaatcatctgacacaattcagtcctcactttaaatctggcagcctagctgttgacaatgcagatcctatattaaaaattccttttgctttacctcatttttcttctggtattttccgctgctggggaagggatacttttattgcacttagaggtatgctgctgattactggacgctatgtagaagccaggaatattattttagcatttgctggtaccctgaggcatggtctcattcctaatctactgggtgaaggaacttatgccagatacaattgtcgggacgctgtgtggtggtggctgcagtgtatccaggattactgtaaagtggttccaaatggtctagacattctcaagtgcccagtttccagaatgtatcctacagatgattctgctcctttgcctgctggcgcactgtttaatataactgcaggagttgatgaagaaacaggatttgtttatggaggaaatcgtttcaattgtggcacatggatggataaaatgggagaaagtgacagagctagaaacagaggaatcccagccacaccaagagatgggtctgctgtggaaattgtgggcctgagtaaatctgctgttcgctggttgctggaattatccaaaaaaaatattttcccttatcatgaagtcacagtaaaacatggaaaggctataaaggtctcatatgatgagtggaacagaaaaatacaggataactttgaaaagctgtttcatgtttcagaagacccttcagatttaaatgaaaagcatccaaatttggttcacaaacgtggcatatacaaagatagttatggagcttcaagtccttggtgtgactatcagctcaggcctaattttaccatagcaatggttgtggcccctgagctctttactacagaaaaagcatggaaagctttggagattgcagaaaaaaaattgcttggtccccttggcatgaaaactttagatccagatgatatggtttactgtggaatttatgacaatgcattagacaatgacaactacaatcttgctaaaggtttcaattatcaccaaggacctgagtggctgtggcctattgggtattttcttcgtgcaaaattatatttttccagattgatgggcccggagactactgcaaagactatagttttggttaaaaatgttctttcccgacattatgttcatcttgagagatccccttggaaaggacttccagaactgaccaatgagaatgcccagtactgtcctttcagctgtgaaacacaagcctggtcagttgctactattcttgagacactttatgatttatag

SEQ ID NO: 33 - DNA, 4173 bp, Pteropus alecto
atgggtcacggtaaacagattagaattttacttctgaacgaaatggaaaagcttgaaaagaccctctttagacttgaacaagggtttgaactacagttccgattaggcccaactttacaaggaaaaacagttactgtgcatacaaattacccatatcctggagaaacatttaatcgagaaaaattccgttccctggaatgggaaaatccatcagaaagagaagatgattctgataaatactgtaaacttaatctccaacaagcgggatcatttcagtattacttccttcgaggaaatgagaagagtggtgggggttacatagttgtggatcctgtattacgtgttggtactgataatcatgtgttacccttagactgtgttactctccagacatttttagctaagtgtttgggacccttggatgaatgggaaagcagacttagggttgcaaaagaatcaggttacaacatgattcactttaccccattgcagactcttggccagtctaggtcatgctactctcttgctgatcagttagaattaaatcctgacttttccagacctaataaaaagtgtacctgggatgatgttggacagctagtggaaaaattgaaaaaggaatggaatattctttgtatcaccgatgttgtctacaatcataccggaaataggaaaataaccaagcctgatccaaaagaacaccttaagataattcaggatcctgaatacaggaggcttggctgtactgtagatatgaacattgcactagcgactttcataccaaatgagtattttactttcccatttgaggaaatgaccctctccacagaagaatctatgattcatctcccaaataaagcttgttttctgatggcacataatggatgggtaatgggagatgatccccttcgaaactttgctgaaccaggttcagatgtttatctgaggagagaacttatttgctggggagacagtgttaaattacgctatgggaataaaccagaggactgtccttatctctgggcacacatgaaaaaatacactgaaataactgcaacttatttccagggagtacgtcttgataactgccactccacacctcttcatgtagctgagtacatgttggatgctgctaggaaattgcaacccaatttatatatagtggcagaactgttcacaggaagtgaagacttggacaatgtctttgttactagactgggaattagttccttaataagagaggcaatgagtgcacatgatagtcatgaagagggcagattagtttaccgatatggaggagaacccgttgggtcatttgttcagccctgtttgaggcctttgatgccagctattgcacatgccctgtttatggatattacccatgataatgagtgtcctattgtgcatagatcagcatatgatgctctcccaagttccatgattgtttctatggcgtgttgtgctagtggtagtactaaaggctatgatgaattagtgcctcatcaggtgtatgtggatcaggttgatgaagacatagtggcagtaacaagacactcacctagtatccatcagtctgttgtggctgtgtctagaactgctttcaagaatcccaagacttcattttacagcaaggaagtccctcaaatgtgcatccctggcaaaattgaagaagtagttcttgaagctagaactattgaaagaaatacaaaaccttataagagggatgaaaattcaatcaatggaatgccagatatcacagcagaaattagagaacatattcagcttaatgaaagtaaaattgttaaacaagctggaattgccacaaaaggacccaatgaatacattcaagaaatagaatttgaaaacttgtctccaggaagtgttattgtattcagagttagtctcgatccacatgcacaagtcgctgttggaattcttcgaaatcatttaactcagttcagtcctcactttaaatctgggagcctttctgccgacagctcagatcctatattaaaaattcctttcgcttatattgcctctaaattaactttggctgagctaaatcaaatactttaccggtgtgaatcagaagaacaagaagatggtgggggatgttataatataccaaactggtcatctcttaaatatgcaggtcttcaagagaatagttctttggagttagctccttatgtgggctttggtggaggttgtggggcagcacctgcaggtctaaatcggggtgggggtgttcggtccgaccaggcctcactagagcgattcctgactaccttgcttgccactgtggactatacagcccttgtgtccacttctgtatgttcaccccacatcactggacacgagcagcagcccaggctatgggaacgaattgcctctgccaataatatagcatgctatttctatgacttttcaggattaatgtctgtattagcagaaatgagaccaaagaatgacttggggcatcctttttgtgataatttgagatctggagattggatgattgactatgtcagtaatcggcttatttcacgatcgggaactattgctgaagttggcagatggttgcaggctatgttcttctacctgaagcagatcccacgctatcttatcccatgttatttcgatgctgtattaatcggtgcatacaccactcttctggatacggcatggaaacaaatgtcaagctttgttcagaatggttctacctttgtgaaacacctttcattgggttctgtccagctgtgtggagtaggaaaatacgcttctcttccacttctttcaccttcgcttatggatgtaccatacaggctaaatgagatcacaaaagaaaaggagcaatgttgtgtgactctagctgcaggcttgcctcatttttcttctggtattttccgctgctggggaagggatacttttattgcacttagaggtatactgctgattaccgggcgctatttagaagccaggaatattattttagcgtttgctggtaccttgagacacggtctcattcctaatctcctgggtgaaggaacttatgccagatacaactgccgggatgccgtgtggtggtggctgcagtgtattcaagactactgtaaagtggttccaaatggcctagacattctcaagtgccctgtctccagaatgtatcctacagatgattctgttcctttgtcggccggcacagtggatcagccattgtttgaagtaatacaagaagctatgcagaggcacatgcagggcatacagttccgagaaaggaatgctggtccacagatagatcgaaacatgaaggatgaaggttttaatataactgtaggggttgatgaagaaacaggatttgtttatggaggaaatcgcttcaattgcggcacatggatggataaaatgggagaaagtgacagagctagaaacagaggaatcccagccactccaagagatggatctgctgtggaaattgtgggcctaagtaaatctgccattcgctggttgctggaattatctaaaaaaaatatttttccttatcatgaagtcacagtaaaaagagatggaaaggttgtgacagtctcatatgatgagtggaacagaaaaatacaagacaactttgaaaagctattttatgtgtccgaagacccttcagactttaatgaaaagaatccaaatctggttcacaaacgtggtatatacaaagacagttatggagcttcaagcccttggtgtgactatcagctcaggcctaattttaccatagcaatggttgtagcccctgagctctttactacagaaaaagcatggaaagctttacaggtggcagaaaaaaaattgcttggtccccttggcatgaaaactttggatccagatgatatggtttactgtggagtttatgacaatgccttagacaatgacaactacaatcttgcgaaaggtttcaattatcatcaaggacctgagtggctttggctcattgggtattttcttcgtgcaaaattatatttttccaaattaatgggtccagagacgaatgcaaagactatttttttggttaaaaatgttctttcccggcactatgttcatcttgagagtctggcttgttttgccctcaccactctgctgcagctgctcaacaagatcctttctgcttcccagatcccatga

SEQ ID NO: 34 - DNA, 3759 bp, Cercocebus atys
atgaattccatccgaaaaatgatttgggaggatatttttccaaagcttaaactctgggaatttttccaagtagacgtcaacaaaaaaaaaaaaaaaaaaaaaagacttcttacacaagaaaataggagagtaaccaagtctgatccacaccaacatcttaagattattcaagatcctgaatacagacgatttggctgtactgtagatatgaacattgcactaacgactttcataccacatgacaatgggccagcagcaattgaagaatgctgtaattggtttcgtaagagaattgaggaattaaattcagagaagcatcgactcattaactatcatcaggaacaggcagttaattgccttttgggaaatgtgttttatgaacgactggctggccatggtccaaaactaggacctgtcactagaaagcatcctttagttaccaggtattttactttcccatttgaagaaatggacttctccgtggaagaatctatgattcatctcccaaataaagcttgttttctgatggcacacaatggatgggtaatgggagatgatcctcttcgaaactttgctgaaccaggctcagaagtttacctaaggagagaacttatttgctggggagacagtgttaaattgcgctatgggaataaaccagaggactgtccttttctctgggcacacatgaaaaaatacactgaaataactgcaacttatttccagggagtacgtcttgataactgccactcaacacctcttcatgtagctgagtacatgttggatgctgctaggaatttgcaacccaatttatatgtagtagctgaactgttcacaggaagtgaagatctggacaatatctttgttactagactgggcattagttccttaataagagaggcaatgagtgcatataatagtcatgaagagggcagattagtttaccgatatggaggagaacctgttggatcctttgttcagccctgtttgaggcctttaatgccagctattgcacatgccttgtttatggatattacccatgataatgagtgtcctattgtgcatagatcagcatatgatgctcttccaagtactacaattgtttctatggcgtgttgtgctagtggaagtacaagaggctatgatgaattagtgcctcatcagatttcagtggtttctgaggaacggttttacactaagtggaatcctggagcattgccttcaaatacaggtgaagttaatttccaaagcggcattattgcagccaggtgtgctatcaataagcttcatcaggagcttggagccaagggttttattcaggtgtatgtggatcaagttgatgaagacatagtggcagtaacaagacactcacctagcatccatcagtctgttgtggctgtatctagaactgctttcaggaatcccaagacttcattttacagcaaggaagtgcctcaaatgtgcatccctggcaaaattgaagaagtagttcttgaagctagaactattgagagaaatacgaaaccttacaggaaggatgagaattcaatcaatggaatgccagatatcacagtagaaattagagaacatattcagcttaatgaaagtaaaattgttaaacaagctggagttgccacaaaagggcccaatgaatatattcaagaaatagaatttgaaaacttgtctccaggaagcgttattatattcagagttagtcttgatccacacgcacaagtcgctgttggaattcttcgaaatcatctgacccaattcagtcctcactttaaatctgggagcctagctgttgacaattcagatcctatattaaaaattccctttgcttctattgcctccaaattaactttggctgagctaaatcagatcctttaccgatgtgaatcagaagaaaaggaagatggtggagggtgctatgacataccaaactggtcagcccttaaatatgcaggtcttcaaggtttaatgtctgtattggcagaaataagaccaaagaatgacttgggccatcctttttgtaataatttgagatctggagattggatgattgactatgtcagtaaccggcttatttcacgatcaggaactattgctgaagttggtaaatggttgcaggctatgttcttctacctgaagcagatcccacgttaccttatcccatgttactttgatgctatattaattggtgcatataccactcttctggatatagcatggaagcagatgtcaagctttgttcagaatggttcaacctttgtgaaacacctttcattgggttcagttcaactgtgtggagtaggaaaattcccttccctgccaattctttcacctgcactaacgggtgtaccttatagattaaatgagatcacaaaagaaaaggagcaatgttgtgtttctctagctgcaggcttacctcatttttcttctggtattttccgctgctggggaagggatacttttattgcacttagaggcatactgctgattactggacgctatgtagaagccaggaatattattttagcatttgctggtaccctgaggcatggtctcattcctaatctactgggtgaaggaacttatgccagatacaattgtcgggatgctgtgtggtggtggctgcagtgtatccaggattactgtaaaatggttccaaatggtctagacattctcaagtgtccagtttccagaatgtatcctacagatgattctgctcctttgcctgctggcacactggatcagccattgtttgaagtcatacaggaagcaatgcaaagacacatgcagggcatacagttccgagaaaggaatgctggtcccaagatagatcgaaacatgaaggatgaaggttttaatgtaactgcaggagttgatgaagaaacaggatttgtttatggaggaaatcgtttcaattgtggcacatggatggataaaatgggagaaagtgacagagctagaaacacaggaatcccagccacaccaagagatgggtctgctgtggaaattgtgggactgagtaaatctgctgttcgctggttgctggaattatccaaaaaaaatattttcccttatcatgaagtcacagtaaaaagacatggaaaggttgtaaaggtctcatatgatgagtggaacagaaaaatacaagacaactttgaaaagctatttcatgtttcagaagacccttcagatttaaatgaaaagcatccaaatctggttcacaaacgtggcatatacaaagatagttatggagcttcaagtccctggtgtgactatcagctcaggcctaattttactatagcaatggttgtggcccctgagctctttactacagcaaaagcatggaaagctttggagattgcagaaaaaaaattgcttggtccccttggcatgaaaactttagatccagatgatatggtttactgtggaatttatgacaatgcattagacaatgacaactacaatcttgcaaaaggtttcaattatcaccaaggacctgagtggctgtggcctattggatattttcttcgtgcaaaattatatttttccagattgatgggcccggagactactgcaaagactatagttttggttaaaaatgttctttcccgacactatgttcatcttgagagatccccttggaaaggacttccagaactgaccaatgagaatgcccaatactgtcctttcagctgtgaaacacaagcctggtcaatttctactattcttgagacactttatgatttatag

SEQ ID NO: 35 - DNA, 3351 bp, Ornithorhynchus anatinus
atgtttgaaggcagagcggaaggagtcgttggagagtactttacttttccgtatggagaaatgacttctgtagaagaagaatctttgatgcatcaacctgaaaaagcttgttttttcatggcccataatggttgggtcatgggagatgatccattgagaaattttgctgagccagggtcagatgtttacctcaggagagagcttgtttgctggggagacagtgttaaattacgttatggaaataaaccagaagactgcccttacctctgggcccacatgaaaaaatatactgaaataactgccaagtattttcaaggagtgcgtcttgacaactgccactcgacacctcttcacgtagctgagtatatgctggatgctgctaggaaattgcagcccaatttgtatgtagtggctgagctgttcacaggaagtgaggagctggacaatatctttgtgactagactgggcattagctccttaataagagaagctatgagtgcatataatagccatgaagaaggcagattagtgtaccgctttggaggagagccagtgggatctttcgttcagccgtgtttgagacctttgatgccagctattgcacatgctctgtttatggatatcactcatgataacgaatgtcctattgtgcatcgatcagcatatgatgctcttccgagctccaccatagtttccatggcttgctgtgctagtggaagtactaggggctatgatgaattagtacctcatcagatttctgtagtttctgaagaacggttttataccaagtggaacccagcagctactctatcaaacccatctgaagttaatctccagactggaattatagcaggaagacgtgccataaataagctgcaccaagaacttggagctaaaggttttattcaggtttatgtggatcaggttgatgaagacatagtagcagtgacgagacactgtcctagctctcaccagtccgtagtggccgtgtctcgcactgcttttagaaaccccaagacttctgcttacagcaaagaagtgccgcagatgtgcatcccaggtaaaattgaagaagtagttcttgaggccagaactgttgaaagaaatgttggttcctacgtaaaggatgcaaaatccatcaatggaatgcccgacatcacagtagaaattagagaacacatccagcttaatgaaagtaaaattgtaaaacaagctggagttgccacaaaaggtcttcatgaatatgtccaagaaatagaatttgaaaatttgaccccaggaagtgttattatatttcgagtaagccttgatccacacgcacaagtggctgttggaatacttcggaatcacctgacacaattcagtcctaattttaaaattggaagccttcctgttgacaattcagatcctatattaaaaattccttttgcttctatttcatctaaattaactttagctgacctaaatcaattactctaccgatgtgagtcagaagaacaagaagatggtggaggatgttatgatgtaccaaactggtcacccctcaaatatgggggccttcaaggattaatgtcagtaatggctgaaattaggccaaagaatgacttgggacatcctttttgcaataatttgcgatctggagattggatgattgattatgtcagtaatcgactgatttcgcgctcaggatctattgctgaagttggtaaatggttccaagctatgttcttctatctaaagcagattccacgttaccttatcccttgttattttgatgctatattaattggtgcgtacaccactcttctggatatagcctggaagcagatgtcaagctttgtccagaatggttcaacatttgtaaaacacctgtcattgggttcagttcaaatgtgcgggataggaaagttcccatctctgccttttctttctccatcacttggtgatgttccctatagactgaatgaaattacacaggaaaaggaacagtgctgtgtttctctagctgctgggttacctcatttttcatctggaatttttcgctgctggggaagagataccttcatagcacttagaggtctactgctaattactggtcgctttttagaggcaaggaacataattctagcatttgctggtactctgagacatggtcttattcccaatcttctcggccaggggacgtatgccagattcaattgtcgagatgcagtgtggtggtggcttcagtgtattcaggattactgtaaaattgttccaaagggcacggacattctcaagtgccccgtatccagaatgtatccatcagatgactcttctgctctaccagccggcacattggatcagccattgtatgaagtaatacaggaagctatgcagcgtcatatgcaaggcatacagttccgagaaaagaatgctggtccacagattgaccggaatatgaaggatgaaggttttaatgtcactgcaggagttgatgatgaaagtgggtttgtttatggaggcaatcacttcaactgtggaacatggatggataaaatgggagagagtgacagaggtcgcaacagaggaatcccagctacacccagagatgggtctgctgtggaaattgttggcctgagtaaatcaactgttcgctggttggtagaattatcgaaaaaaaatgtgttcccttatcacggagttacagtaaagagaaatgaaaaagaggtattaatcacatacgatgaatggaacaggaaaatccaagaccactttgaaaagctattctatgtttcagaggatccatcagatactaatgaaaagcatcctaatttggttcataagcgtggtatatacaaagatagctatggagcttcaagtccttggtgtgactaccagctcaggccaaactttaccatagcaatggttgtggctcctgaactctttactcctcagaaggcatggaaagctttggaaatagcagagaagaaattgcttggtcccctgggcatgaaaactctggatccagatgatatggtgtactgtggagtatatgataatgccctagacaatgacaactacaaccttgctaaaggttttaattaccaccaaggacctgaatggttgtggcctgttggatattttcttcgtgcaaagttatatttttccaagttaatgggtcaggaaacttacacaaagactgtgtttttgattaaaaatgttctttcccgtcattacgtccatcttgagagatccccttggaaagggcttccagagctgactaatgaaaatggacaatactgttctttcagctgtgaaacacaggcttggtcaattgccgttattcttgaaactctttatgatttatga

SEQ ID NO: 36 - DNA, 3915 bp, Anas platyrhynchos
atgcatccagaatgtggctataaccttgtaaattcccctcacctgaagccagcttgggtcttagatagagctctgtggcacttgacctgtatggtggctgatggaaagtgtattgataaaggggtccctccgttgattgaaaatgatcaccacctgaattgtgtccgtaaaataatttgggaagagatatatccaaaaattaaactgtgggaatttttccaagtggatgttaataaagctgtggaacaatttagaacccttctaactcaaggtaaagaaagcaaaatgagcactaaatctgatccaaatcaacatcttcagatagttcaggaccctgagtatagacgatttggctgtactgtagatatgaatatagcattggcaaccttcataccgcacagcaatggaccaggtgcaatagaagagtgttgtaactggtttcgcaagaggattgaggaactgaatgctgagcaacacagacagattcatcaccatcaagagcaggcagtcaactgtcttgcggggactgtggtttatgaacgactggctggtcatggtcctaaactgggtcctattagtagaaaatatcctttagttaccaggtattttacttacccattcaaagacatgactgtggaggaagaagaagctatgatacatcgcccagataaagcttgctatttcatggcccataatggatgggttatgggcgatgatcctcttagaaactttgcagaaccaggttcaaatgtttacttgagaagggagcttatttgctggggagacagtgtgaaactgcgttatgggaacaaacctgaagactgcccatacctctgggcacatatgaaaaaatacacagaaatcacagccaaatatttccatggcgttcgtcttgacaactgtcactcaacacctattcatgtagctgagtacatgctggacacagctagaaaattgcgagcagatttgtttgtagtggctgaactgttcacaggaaatgaggagctggacaatatctttgtgaataggctgggcattacctccttaataagagaggcaatgacagcttataatagccatgaggagggaaggttagtttatcgttttggaggtgaacctgttggctcttttgttcagccacgtttgagacccctgatgccagctattgctcatgcactgttcatggatattacacatgataatgagtgtccgatccagcaccgatctgcatatgatgctcttcccagtgcaatgattgtttccatggcatgctgtgctacaggtagcaccaaaggttatgatgaacttgtaccacaccagatatccgtagtatccgaagagagattttattcaacatggaatccagcagcacacctgacttctggtgaagttaatttccaaacaggaattctagcaggaaggctggccataaacaggctgcatcaggagctgggagctaaaggttttaatcaggtgtatgtagatcaagttgatgaagatatagtggcagtgacaagacattgccctaatacacaccagtctgttgtggctgtaagtagaactgctttcagagatccaaagacttccttctacagtaaagaagtgcctgaaatgtgtatcccagggaaaattgaagaagtagtacttgaggctagaaccattgagagaaatactaatccttacaaaaaagatgaacgttttataaatggattgcctaacttcacagtggaactcagagagcacattcagattaaagacagtaaaattataaagcaagctggaactgccataaaagggccaaatgaatttgttcaagaaatagaatttgaaaatttaacaccaggaagtgtaatagtattcagagttagtcttgatccaaaggcacaagaggctgttggtgtactccgtagtcatctgatccagtttagtcctcactttaaatctggaagtcttcctgatgatcattcagcacccatattaaaaacattattttcttcaattgcatctaaattaagtttggctgacctaaatcaagtgctgtataggtgtgaggcagaagaacaagaagatggtggaggctgttacaatataccaaactggtcaccgttgaagtatgcaggcctccaagggttaatgtcagtaatggcagacattagaccaaagaatgatttgggccacccgttttgtgataatttaagatctggagattggatgattgattatgtcagcaatcgtctgatttcacgtactggagcctgtgcagaagttggtaaatggttgaaggccatgtttatctatttaaagaaaattccacgttaccttatcccatgttattttgatgccatattagtgggtgcatacacaacgcttctggatgtgggatggcatcagatgtctagctttgtgcagaacggatcaacatttgttaaacacctttccttgggctcaatccagatgtgtgggataggaaaatactcatgtttgcccgatctgtctccttccttacatgatgttccctatagactgaatgagattacaaatgagaaagaacagtgttgtgtttctttggcagctggtttacctcacttttcttcagggatttttcgctcttggggaagggatacctttattgcactgagaggtctgatgttagttacagggcgttatctagaagcaagaaacataattttagcatttggtgggactttaagacatggtctcattcccaacctgctcggccaggggacgcatgccagatacaactgtcgtgatgctgtatggtggtggcttcagtgtatccaggactactgtaaaattgttccaaatggattagacattctcagatgtcctgtttccagaatgtacccaagagatgactcttctcctcaacctgcaggcagtgtggatcagccgctttatgaagtaatacaggaagcaatgcaacgacacatggaaggcataaatttccgagaaaggaatgccggcccacagatagatcaaaacatgagagatgaaggttttaatgtaacagcgggtgttgaccgtgaaactggctttgtcttcggagggaaccgtttcaattgtggcacctggatggataaaatgggggagagtgacagagctcgcaacagaggaattcctgctactccgagagatggctctgctgtggaaattgttggcttgtgcaagtcaactgtacgctggcttctggatttgtctaggaaaaatgagtttccattccatggagtcaccataaaaagacacggaaaggaggaaactatcacatatgatgaatgggacagaaaaattcaagcacactttgaaaagctcttctttgtctctgagaacccagcagatccaaatgaaaaacatccaaatcttgttcacaaacgtggaatctataaagacagctatggagcttcaagtccatggtgtgattaccaactcagaccaaattttacaatagcaatggttgtggcacctgagttgttcacacctgagagagcttggaaagctctgcagatagcagaggaaaaactacttggtccgttaggcatgaaaactttagacccagatgatatggtgtactgtggagtatatgataatgctcttgacaatgacaactataatgtagccagaggttttaattatcaccaaggacctgaatggctgtggccaattggatatttccttcgtgccaaattgtacttctcaaagctaattggtccacagatatacgcaaaaactgtagttatgataaagaatgtgctttctcgccactatgttcaccttgaaaggtcatcctggaaagggcttccagagctgaccaatgaaaatggacaatattgccctttcagctgtgaaactcaggcctggtcaattagtgttatccttgaaatcctttatgatttgtga

SEQ ID NO: 37 - DNA, 4599 bp, Homo sapiens
atgggacacagtaaacagattcgaattttacttctgaacgaaatggagaaactggaaaagaccctcttcagacttgaacaagggtatgagctacagttccgattaggcccaactttacagggaaaagcagttaccgtgtatacaaattacccatttcctggagaaacatttaatagagaaaaattccgttctctggattgggaaaatccaacagaaagagaagatgattctgataaatactgtaaacttaatctgcaacaatctggttcatttcagtattatttccttcaaggaaatgagaaaagtggtggaggttacatagttgtggaccccattttacgtgttggtgctgataatcatgtgctacccttggactgtgttactcttcagacatttttagctaagtgtttgggaccttttgatgaatgggaaagcagacttagggttgcaaaagaatcaggctacaacatgattcattttaccccattgcagactcttggactatctaggtcatgctactcccttgccaatcagttagaattaaatcctgacttttcaagacctaatagaaagtatacctggaatgatgttggacagctagtggaaaaattaaaaaaggaatggaatgttatttgtattactgatgttgtctacaatcatactgctgctaatagtaaatggatccaggaacatccagaatgtgcctataatcttgtaaattctccacacttaaaacctgcctgggtcttagacagagcactttggcgtttctcctgtgatgttgcagaagggaaatacaaagaaaagggaatacctgctttgattgaaaatgatcaccatatgaactccatccgaaaaataatttgggaggatatttttccaaagcttaaactctgggaatttttccaagtagatgtcaacaaagcggttgagcaatttagaagacttcttacacaagaaaataggcgagtaaccaagtctgatccaaaccaacaccttacgattattcaagatcctgaatacagacggtttggctgtactgtagatatgaacattgcactaacgactttcataccacatgacaaggggccagcagcaattgaagaatgctgtaattggtttcataaaagaatggaggaattaaattcagagaagcatcgactcattaactatcatcaggaacaggcagttaattgccttttgggaaatgtgttttatgaacgactggctggccatggtccaaaactaggacctgtcactagaaagcatcctttagttaccaggtattttactttcccatttgaagagatagacttctccatggaagaatctatgattcatctgccaaataaagcttgttttctgatggcacacaatggatgggtaatgggagatgatcctcttcgaaactttgctgaaccgggttcagaagtttacctaaggagagaacttatttgctggggagacagtgttaaattacgctatgggaataaaccagaggactgtccttatctctgggcacacatgaaaaaatacactgaaataactgcaacttatttccagggagtacgtcttgataactgccactcaacacctcttcacgtagctgagtacatgttggatgctgctaggaatttgcaacccaatttatatgtagtagctgaactgttcacaggaagtgaggacctagacaatgtctttgttactagactgggcattagttccttaataagagaggcaatgagtgcatataatagtcatgaagagggcagattagtttaccgatatggaggagaacctgttggatcctttgttcagccctgtttgaggcctttaatgccagctattgcacatgccctgtttatggatattacgcatgataatgagtgtcctattgtgcatagatcagcgtatgatgctcttccaagtactacaattgtttctatggcatgttgtgctagtggaagtacaagaggctatgatgaattagtgcctcatcagatttcagtggtttctgaagaacggttttacactaagtggaatcctgaagcattgccttcaaacacaggtgaagttaatttccaaagcggcattattgcagccaggtgtgctatcagtaaacttcatcaggagcttggagccaagggttttattcaggtgtatgtggatcaagttgatgaagacatagtggcagtaacaagacactcacctagcatccatcagtctgttgtggctgtaactagaactgctttcaggaatcccaagacttcattttacagcaaggaagtgcctcaaatgtgcatccctggcaaaattgaagaagtagttcttgaagctagaactattgagagaaacacgaaaccttataggaaggatgaaaattcaatcaatggaacaccagatatcacagtagaaattagagaacatattcagcttaatgaaagtaaaattgttaaacaagctggagttgccacaaaagggcccaatgaatatattcaagaaatagaatttgaaaacttgtctccaggaagtgttattatattcagagttagtcttgatccacatgcacaagtcgctgttggcattcttcgaaatcatctgacacaattcagtcctcactttaaatctggcagcctagctgttgacaatgcagatcctatattaaaaattccttttgcttctcttgcctatagattaactttggctgagctaaatcagatcctttaccgatgtgaatcagaagaaaaggaagatggtggagggtgctatgacataccaaactggtcagcccttaaatatgcaggtcttcaaggtttaatgtctgtattggcagaaataagaccaaagaatgacttggggcatcctttttgtaataatttgaggtctggagattggatgattgactatgtcagtaaccggcttatttcacgatcaggaactattgctgaagttggtaaatggttgcaggctatgttcttctacctgaagcagatcccacgttaccttatcccatgttactttgatgctatattaattggtgcatataccactcttctggatacagcatggaagcagatgtcaagctttgttcagaatggttcaacctttgtgaaacacctttcattgggttcagttcaactgtgtggagtaggaaaattcccttccctgccaattctttcacctgccctaatggatgtaccttataggttaaatgagatcacaaaagaaaaggagcaatgttgtgtttctctagctgcaggcttacctcatttttcttctggtattttccgctgctggggaagggatacttttattgcacttagaggtatactgctgattactggacgctatgtagaagccaggaatattattttagcatttgcgggtaccctgaggcatggtctcattcctaatctactgggtgaaggaatttatgccagatacaattgtcgggatgctgtgtggtggtggctgcagtgtatccaggattactgtaaaatggttccaaatggactagacattctcaagtgcccagtttccagaatgtatcctacagatgattctgctcctttgcctgctggcacactggatcagccattgtttgaagtcatacaggaagcaatgcaaaaacacatgcagggcatacagttccgagaaaggaatgctggtccccagatagatcgaaacatgaaggacgaaggttttaatataactgcaggagttgatgaagaaacaggatttgtttatggaggaaatcgtttcaattgtggcacatggatggataaaatgggagaaagtgacagagctagaaacagaggaatcccagccacaccaagagatgggtctgctgtggaaattgtgggcctgagtaaatctgctgttcgctggttgctggaattatccaaaaaaaatattttcccttatcatgaagtcacagtaaaaagacatggaaaggctataaaggtctcatatgatgagtggaacagaaaaatacaagacaactttgaaaagctatttcatgtttccgaagacccttcagatttaaatgaaaagcatccaaatctggttcacaaacgtggcatatacaaagatagttatggagcttcaagtccttggtgtgactatcagctcaggcctaattttaccatagcaatggttgtggcccctgagctctttactacagaaaaagcatggaaagctttggagattgcagaaaaaaaattgcttggtccccttggcatgaaaactttagatccagatgatatggtttactgtggaatttatgacaacgcattagacaatgacaactacaatcttgctaaaggtttcaattatcaccaaggacctgagtggctgtggcctattgggtattttcttcgtgcaaaattatatttttccagattgatgggcccggagactactgcaaagactatagttttggttaaaaatgttctttcccgacattatgttcatcttgagagatccccttggaaaggacttccagaactgaccaatgagaatgcccagtactgtcctttcagctgtgaaacacaagcctggtcaattgctactattcttgagacactttatgatttatag

SEQ ID NO: 38 - DNA, 4599 bp, artificial
  hGDE co1
atgggccatagtaaacagattcgcatactcctcttgaacgagatggagaaactggagaagacattgtttcggttggagcaggggtacgagctccagtttcgcctgggaccgacgctccaaggcaaagctgtgactgtatacacgaactatccattcccgggggagacgtttaacagggagaagtttaggtccctggactgggagaacccaaccgaacgagaggacgattccgataaatattgcaagctcaacttgcagcaaagtggcagctttcaatattactttctccaaggcaatgagaaaagtgggggggggtatattgttgtcgatccaatactgcgcgtaggggcagataatcacgttctcccgctggattgcgtcactctccagacattcttggctaaatgcttggggccgtttgatgaatgggagtctcgcttgcgagtggccaaagagtcaggttataacatgattcacttcacaccactccagacattgggacttagtcggagctgttactcactcgcaaatcaattggagcttaacccagacttcagtcggccaaatcggaagtacacgtggaacgacgttggacaacttgtcgaaaagttgaagaaagagtggaatgtgatttgcatcactgacgtggtgtacaatcacaccgcagccaacagcaagtggattcaggagcacccagagtgtgcgtacaacctggtgaactcacctcacctcaaacccgcctgggtgctcgatagggctttgtggcgcttttcttgcgacgtagcggaaggaaagtataaagagaaaggaatacccgccctcatagaaaacgatcatcacatgaattctatacggaaaatcatctgggaggatatatttccgaaacttaaactttgggagttctttcaagtagatgtaaacaaggcggtggagcaattcaggaggctcctcacccaagagaatcgccgggttactaaatctgacccgaatcaacaccttacaataatccaagatccggaatacaggaggtttggttgcactgtcgatatgaatattgcgcttactacgttcatcccccacgacaagggcccggccgcaatagaagaatgctgcaattggttccacaagcggatggaagaactgaactctgaaaagcaccgccttataaattatcaccaagagcaggctgtgaactgtctgctcggtaacgttttttacgagcgcctggccggacacggacctaaactcgggccagtcactcgaaaacacccactggttacgcgatacttcacattcccgttcgaggagatcgacttttctatggaggaatctatgatccacctcccaaataaagcttgttttcttatggcgcacaacggatgggttatgggggacgacccactgcgaaacttcgcagaaccgggtagtgaggtctaccttaggcgcgagctcatttgttggggcgacagcgtcaagctccggtatggaaataagccagaggattgcccttacttgtgggcacacatgaagaagtatacggaaataacagctacctacttccagggggtacgactggataactgccactccacaccgttgcacgtggccgagtatatgctcgacgctgcgcgcaatttgcagccaaatctgtacgtcgtggcagagcttttcactggaagtgaggacttggataacgtctttgtgactcgcctgggaattagtagcttgataagggaggctatgtccgcgtacaacagtcacgaggaaggacgattggtttatcgatatgggggcgagcctgtaggctcctttgtgcaaccctgcttgcggccccttatgcccgctatagcacacgcgctcttcatggatatcacgcacgataatgaatgccccatagtacacagatccgcctacgacgcccttccatctacgacaatcgtctctatggcctgctgcgcctccggcagcactagaggctacgacgaactcgtcccacaccagatttcagtggtatcagaggaacggttttacactaaatggaaccctgaggcgctcccatctaatactggcgaagtaaatttccagtccggaatcattgcggcccgctgtgctatctccaagttgcatcaggaacttggagctaaaggtttcattcaagtatatgtcgatcaggtcgatgaagatattgtggctgtgacccgacactccccatcaattcatcaaagtgtagtggctgtaactcggacggcttttcgcaacccaaagacttcattctactccaaagaggttccacagatgtgtattccgggaaagatagaagaagtggtattggaagcccggaccatcgagaggaacactaaaccatatcgaaaagacgagaactccattaacggaacccctgacatcactgttgagatccgcgagcatattcagcttaacgaaagcaaaatcgttaagcaggccggcgttgccactaagggaccaaacgaatatatccaagaaatcgaattcgaaaacctcagtcctggctccgttattatctttcgcgtatccctcgacccacacgcccaagttgcggtagggatcttgagaaaccacctcacacagttcagcccacactttaaatcaggctccctcgccgttgataacgcggacccaatacttaagatcccctttgcatcccttgcgtatcgacttactctcgcagagcttaatcaaatattgtaccgctgcgagtccgaagagaaggaagacggtggtggctgctacgacatccctaattggagtgcacttaagtacgcggggctgcagggactgatgtcagtgcttgcagagataaggccgaagaatgaccttggccatccattttgtaataatctccgaagtggtgattggatgatagattacgtatcaaaccgcttgatcagtcggtctggtaccatcgcggaagtgggaaagtggttgcaggcaatgttcttttatctcaaacaaatcccacggtacttgataccttgctatttcgacgcaattctcatcggtgcatacacgaccttgctggacacggcctggaagcagatgtctagcttcgttcagaacggttctaccttcgtaaagcacctctcattgggttcagtccaactctgcggagtcgggaaattcccttcacttcctattctctcacctgccctcatggacgtgccctaccggctgaacgaaattactaaggagaaggaacagtgttgtgtttctttggcggcaggcttgccgcacttttccagtggaatcttcagatgttggggacgggacacattcattgcgctccggggtattttgttgataacgggccgatacgttgaggcacgaaatattattctggcattcgccgggaccttgcggcacgggctgatacccaacctgctgggcgaagggatttacgctcgctataactgccgagacgcagtttggtggtggctgcagtgtattcaggactattgtaagatggtaccgaacgggctcgacatcttgaagtgtcccgttagtcgaatgtatcccaccgacgattcagctcccctgcccgcgggaacacttgaccaaccactctttgaagtgatccaagaggctatgcagaaacacatgcagggaatacagttccgagaacgaaacgcagggccgcagattgatcgaaatatgaaagacgaaggatttaatatcacggcaggggtcgacgaagagacggggtttgtctacggcgggaatagatttaactgcggcacctggatggataaaatgggagaaagtgaccgagcacggaaccggggcataccagcaaccccccgagacgggagcgctgttgagatcgtgggtctgtctaagagtgcggttcgctggcttctcgagctttcaaaaaaaaatatatttccttaccacgaggtcacggtcaaaaggcatggaaaagccataaaagtgtcatacgacgagtggaataggaaaatacaagataactttgaaaagctgtttcacgttagcgaagatcccagcgatctcaacgaaaaacatcccaatctggttcacaaacgcgggatctataaagactcatatggagctagttctccttggtgcgattatcaactgagaccgaactttacaatcgccatggtagttgcgcccgagctctttactacagaaaaagcctggaaggcacttgagattgcggaaaagaaactgcttggccctctcgggatgaaaacgcttgatcccgacgacatggtctattgcgggatttacgacaacgcattggacaacgacaactacaacttggcgaaaggatttaattatcaccagggtcctgagtggttgtggcccattggatactttcttcgagcgaagctgtatttttcaaggctgatggggccggaaacgacagcgaaaactattgtgcttgtcaaaaacgtgcttagcaggcattacgtgcacctcgagcgcagcccttggaaaggacttccggagcttacgaacgaaaacgcccagtattgtccatttagctgtgagacgcaggcctggtctattgctaccatcctcgagacactctacgacttgtag

SEQ ID NO: 39 - DNA, 4599 bp, artificial
  hGDE co2
atgggccacagcaagcagatcagaatcctgctgctgaacgagatggaaaagctggaaaagaccctgttccggctcgagcagggctacgagctgcagtttagactgggccctacactgcagggcaaagccgtgaccgtgtacacaaactaccccttccctggcgaaaccttcaaccgcgagaagttcagaagcctggactgggagaaccccaccgagagagaggacgacagcgacaagtactgcaagctgaacctgcagcagagcggctccttccagtactacttcctgcaaggcaacgagaagtccggcggaggctacatcgtggtggaccctattctgagagtgggcgccgacaatcacgtgctgcctctggattgtgtgaccctgcagaccttcctggccaagtgtctgggccctttcgatgagtgggagagcagactgcgcgtggccaaagaaagcggctacaacatgatccacttcacccctctgcagaccctgggcctgagcagaagctgttacagcctggccaaccagctggaactgaaccccgacttcagcagacccaaccggaagtacacctggaacgatgtgggccagctggtggaaaaactgaagaaagaatggaacgtgatctgcatcaccgacgtggtgtacaaccacaccgccgccaacagcaagtggatccaagagcaccctgagtgcgcctacaacctggtcaacagccctcacctgaaacctgcctgggtgctcgatagagccctgtggcggtttagctgtgatgtggccgagggcaagtacaaagagaagggcatccccgctctgatcgagaacgaccaccacatgaacagcatccggaagatcatctgggaagatattttccccaagctgaagctgtgggagttcttccaggtggacgtgaacaaggccgtggaacagttcagacggctgctgacccaagagaacagaagagtgaccaagagcgaccccaaccagcacctgaccatcattcaggaccccgagtatcggagattcggctgcaccgtggacatgaatatcgccctgaccaccttcattccccacgacaaaggacctgccgccatcgaggaatgctgcaactggttccacaagcggatggaagaattgaacagcgagaagcaccggctgatcaactaccaccaagagcaggccgtgaactgcctgctgggcaacgtgttctatgagagactggccggacacggccctaagctgggacctgtgacaagaaagcaccctctggttacccggtacttcacctttccattcgaagagatcgacttctccatggaagagagcatgatccatctgcctaacaaggcctgcttcctgatggctcacaacggctgggttatgggcgacgaccctctgagaaatttcgccgagcctggcagcgaggtgtacctgagaagagaactgatctgttggggcgacagcgtgaagctgagatacggcaacaagcccgaggactgcccttacctgtgggcccatatgaagaagtacacagagatcaccgccacctactttcagggcgtcagactggacaactgccacagcacacctctgcacgtggccgagtacatgctggacgccgctagaaatctgcagcccaacctgtatgtggtggccgagctgtttaccggctccgaggacctggacaatgtgttcgtgaccagactgggcatcagcagcctgatcagagaagccatgtccgcctacaatagccacgaagagggcagactggtgtacagatatggcggcgagcctgtgggcagcttcgttcagccttgtctgaggcctctgatgcccgccattgctcacgccctgttcatggacatcacccacgataacgagtgccccatcgtgcacagaagcgcctacgacgctctgcctagcaccaccattgtgtccatggcctgttgtgccagcggcagcacaagaggctatgacgaactggtgccccaccagatttccgtggtgtccgaggaacggttctacaccaagtggaaccccgaggctctgcccagcaataccggcgaagtgaatttccagagcggcatcattgccgccagatgcgccatcagcaagctgcaccaagaactgggcgccaagggcttcattcaggtgtacgtggaccaggtcgacgaggacattgtggccgtgacaagacacagccccagcatccatcagagcgtggtggctgtgaccagaaccgccttcagaaaccccaagaccagcttctacagcaaagaggtgccccagatgtgcatccccggcaagattgaggaagtggtgctcgaggcccggaccatcgagagaaacaccaagccttaccggaaggacgagaactccatcaacggcacccctgacatcaccgtggaaatcagagagcacatccagctcaacgagagcaagatcgtgaaacaggccggcgtggccacaaagggccccaacgagtatatccaagagattgagttcgagaatctgagccccggcagcgtgatcatcttcagagtgtccctggatcctcacgctcaggtggccgtgggcatcctgagaaatcacctgacacagttcagcccacacttcaagagcggaagcctggccgtggacaacgccgatcctatcctgaagatccccttcgcctctctggcctacagactgacactggctgagctgaaccagatcctgtacagatgcgagtccgaagagaaagaggatggcggaggctgctacgacatccccaattggagcgccctgaagtatgccggactgcagggactgatgtctgtgctggccgagatcagacccaagaacgacctgggacaccccttctgcaacaacctgagatccggcgactggatgatcgactacgtgtccaacagactgatcagcagatccggcacaatcgccgaagtcggcaaatggctgcaggccatgttcttctacctgaagcagatccctcggtatctgatcccctgctacttcgacgccatcctgatcggcgcctacaccacactgctggataccgcctggaagcagatgtccagcttcgtgcagaacggcagcaccttcgtgaagcacctgtctctgggaagcgtgcagctgtgtggcgtgggcaaatttcccagcctgcctatcctgtctcctgcactgatggacgtgccctaccggctgaatgagatcaccaaagaaaaagagcagtgctgcgtcagcctggctgctggcctgcctcatttttccagcggcatcttccggtgttggggcagagacacctttattgccctgagaggcatcctgctgattaccggcagatacgtggaagcccggaacatcatcctggcctttgccggcacactgcggcacggactgattcctaatctgctcggcgagggcatctacgccagatacaactgcagagatgccgtgtggtggtggctccagtgcatccaggactactgcaagatggtgcccaacggcctggacatcctgaagtgccctgtgtccagaatgtaccctaccgacgatagcgcccctctgcctgccggaacacttgaccagcctctgttcgaagtgattcaagaggccatgcagaaacacatgcagggaatccagtttcgcgagcggaatgccggacctcagatcgacagaaacatgaaggatgagggcttcaacatcaccgctggcgtggacgaagagacaggctttgtgtacggcggcaaccggttcaattgcggcacctggatggacaagatgggcgagtctgaccgggccagaaacagaggaattcccgccacacctagagatggcagcgctgtggaaatcgtgggcctgtctaagtctgctgtgcggtggctgctcgaactgagcaagaagaatatctttccgtaccacgaagtgaccgtgaagcggcacggcaaggccatcaaggtgtcctacgacgagtggaacagaaagatccaggacaacttcgaaaagctgttccatgtgtctgaggaccccagcgacctgaacgaaaagcaccccaacctggtgcacaagcgcggcatctacaaggacagctacggcgcctcttctccttggtgcgattaccagctgcggcccaacttcaccattgccatggtggttgcccctgagctgttcaccacagagaaggcctggaaggccctggaaatcgccgagaagaaactgctgggccctctgggcatgaagacactggaccccgacgacatggtgtactgcggaatctacgacaacgccctggataacgacaactacaatctggccaaggggttcaattaccatcagggacccgagtggctgtggcctatcggctatttcctgcgggccaagctgtacttctccagactgatgggccctgagacaaccgccaagacaatcgtgctcgtgaagaacgtgctgagccggcactatgtgcacctggaaagaagcccctggaagggactgcccgagctgaccaatgagaacgcccagtactgccccttcagctgcgaaacacaggcctggtctatcgccaccatcctggaaaccctgtacgacctgtga

SEQ ID NO: 40 - protein, 1515 aa, Homo sapiens
MSLLTCAFYLGYELQFRLGPTLQGKAVTVYTNYPFPGETFNREKFRSLDWENPTEREDDSDKYCKLNLQQSGSFQYYFLQGNEKSGGGYIVVDPILRVGADNHVLPLDCVTLQTFLAKCLGPFDEWESRLRVAKESGYNMIHFTPLQTLGLSRSCYSLANQLELNPDFSRPNRKYTWNDVGQLVEKLKKEWNVICITDVVYNHTAANSKWIQEHPECAYNLVNSPHLKPAWVLDRALWRFSCDVAEGKYKEKGIPALIENDHHMNSIRKIIWEDIFPKLKLWEFFQVDVNKAVEQFRRLLTQENRRVTKSDPNQHLTIIQDPEYRRFGCTVDMNIALTTFIPHDKGPAAIEECCNWFHKRMEELNSEKHRLINYHQEQAVNCLLGNVFYERLAGHGPKLGPVTRKHPLVTRYFTFPFEEIDFSMEESMIHLPNKACFLMAHNGWVMGDDPLRNFAEPGSEVYLRRELICWGDSVKLRYGNKPEDCPYLWAHMKKYTEITATYFQGVRLDNCHSTPLHVAEYMLDAARNLQPNLYVVAELFTGSEDLDNVFVTRLGISSLIREAMSAYNSHEEGRLVYRYGGEPVGSFVQPCLRPLMPAIAHALFMDITHDNECPIVHRSAYDALPSTTIVSMACCASGSTRGYDELVPHQISVVSEERFYTKWNPEALPSNTGEVNFQSGIIAARCAISKLHQELGAKGFIQVYVDQVDEDIVAVTRHSPSIHQSVVAVTRTAFRNPKTSFYSKEVPQMCIPGKIEEVVLEARTIERNTKPYRKDENSINGTPDITVEIREHIQLNESKIVKQAGVATKGPNEYIQEIEFENLSPGSVIIFRVSLDPHAQVAVGILRNHLTQFSPHFKSGSLAVDNADPILKIPFASLAYRLTLAELNQILYRCESEEKEDGGGCYDIPNWSALKYAGLQGLMSVLAEIRPKNDLGHPFCNNLRSGDWMIDYVSNRLISRSGTIAEVGKWLQAMFFYLKQIPRYLIPCYFDAILIGAYTTLLDTAWKQMSSFVQNGSTFVKHLSLGSVQLCGVGKFPSLPILSPALMDVPYRLNEITKEKEQCCVSLAAGLPHFSSGIFRCWGRDTFIALRGILLITGRYVEARNIILAFAGTLRHGLIPNLLGEGIYARYNCRDAVWWWLQCIQDYCKMVPNGLDILKCPVSRMYPTDDSAPLPAGTLDQPLFEVIQEAMQKHMQGIQFRERNAGPQIDRNMKDEGFNITAGVDEETGFVYGGNRFNCGTWMDKMGESDRARNRGIPATPRDGSAVEIVGLSKSAVRWLLELSKKNIFPYHEVTVKRHGKAIKVSYDEWNRKIQDNFEKLFHVSEDPSDLNEKHPNLVHKRGIYKDSYGASSPWCDYQLRPNFTIAMVVAPELFTTEKAWKALEIAEKKLLGPLGMKTLDPDDMVYCGIYDNALDNDNYNLAKGFNYHQGPEWLWPIGYFLRAKLYFSRLMGPETTAKTIVLVKNVLSRHYVHLERSPWKGLPELTNENAQYCPFSCETQAWSIATILETLYDL

SEQ ID NO: 41 - protein, 1516 aa, Homo sapiens
MAPILSINLFIGYELQFRLGPTLQGKAVTVYTNYPFPGETFNREKFRSLDWENPTEREDDSDKYCKLNLQQSGSFQYYFLQGNEKSGGGYIVVDPILRVGADNHVLPLDCVTLQTFLAKCLGPFDEWESRLRVAKESGYNMIHFTPLQTLGLSRSCYSLANQLELNPDFSRPNRKYTWNDVGQLVEKLKKEWNVICITDVVYNHTAANSKWIQEHPECAYNLVNSPHLKPAWVLDRALWRFSCDVAEGKYKEKGIPALIENDHHMNSIRKIIWEDIFPKLKLWEFFQVDVNKAVEQFRRLLTQENRRVTKSDPNQHLTIIQDPEYRRFGCTVDMNIALTTFIPHDKGPAAIEECCNWFHKRMEELNSEKHRLINYHQEQAVNCLLGNVFYERLAGHGPKLGPVTRKHPLVTRYFTFPFEEIDFSMEESMIHLPNKACFLMAHNGWVMGDDPLRNFAEPGSEVYLRRELICWGDSVKLRYGNKPEDCPYLWAHMKKYTEITATYFQGVRLDNCHSTPLHVAEYMLDAARNLQPNLYVVAELFTGSEDLDNVFVTRLGISSLIREAMSAYNSHEEGRLVYRYGGEPVGSFVQPCLRPLMPAIAHALFMDITHDNECPIVHRSAYDALPSTTIVSMACCASGSTRGYDELVPHQISVVSEERFYTKWNPEALPSNTGEVNFQSGIIAARCAISKLHQELGAKGFIQVYVDQVDEDIVAVTRHSPSIHQSVVAVTRTAFRNPKTSFYSKEVPQMCIPGKIEEVVLEARTIERNTKPYRKDENSINGTPDITVEIREHIQLNESKIVKQAGVATKGPNEYIQEIEFENLSPGSVIIFRVSLDPHAQVAVGILRNHLTQFSPHFKSGSLAVDNADPILKIPFASLAYRLTLAELNQILYRCESEEKEDGGGCYDIPNWSALKYAGLQGLMSVLAEIRPKNDLGHPFCNNLRSGDWMIDYVSNRLISRSGTIAEVGKWLQAMFFYLKQIPRYLIPCYFDAILIGAYTTLLDTAWKQMSSFVQNGSTFVKHLSLGSVQLCGVGKFPSLPILSPALMDVPYRLNEITKEKEQCCVSLAAGLPHFSSGIFRCWGRDTFIALRGILLITGRYVEARNIILAFAGTLRHGLIPNLLGEGIYARYNCRDAVWWWLQCIQDYCKMVPNGLDILKCPVSRMYPTDDSAPLPAGTLDQPLFEVIQEAMQKHMQGIQFRERNAGPQIDRNMKDEGFNITAGVDEETGFVYGGNRFNCGTWMDKMGESDRARNRGIPATPRDGSAVEIVGLSKSAVRWLLELSKKNIFPYHEVTVKRHGKAIKVSYDEWNRKIQDNFEKLFHVSEDPSDLNEKHPNLVHKRGIYKDSYGASSPWCDYQLRPNFTIAMVVAPELFTTEKAWKALEIAEKKLLGPLGMKTLDPDDMVYCGIYDNALDNDNYNLAKGFNYHQGPEWLWPIGYFLRAKLYFSRLMGPETTAKTIVLVKNVLSRHYVHLERSPWKGLPELTNENAQYCPFSCETQAWSIATILETLYDL

SEQ ID NO: 42 - DNA, 441 bp, artificial
  HBB2 intron
gtacacatattgaccaaatcagggtaattttgcatttgtaattttaaaaaatgctttcttcttttaatatacttttttgtttatcttatttctaatactttccctaatctctttctttcagggcaataatgatacaatgtatcatgcctctttgcaccattctaaagaataacagtgataatttctgggttaaggcaatagcaatatttctgcatataaatatttctgcatataaattgtaactgatgtaagaggtttcatattgctaatagcagctacaatccagctaccattctgcttttattttatggttgggataaggctggattattctgagtccaagctaggcccttttgctaatcatgttcatacctcttatcttcctcccacagctcctgggcaacgtgctggtctgtgtgctggcccatcactttggcaaag

SEQ ID NO: 43 - DNA, 441 bp, artificial
  modified HBB2 intron
gtacacatattgaccaaatcagggtaattttgcatttgtaattttaaaaaatgctttcttcttttaatatacttttttgtttatcttatttctaatactttccctaatctctttctttcagggcaataatgatacaatgtatcatgcctctttgcaccattctaaagaataacagtgataatttctgggttaaggcaatagcaatatttctgcatataaatatttctgcatataaattgtaactgatgtaagaggtttcatattgctaatagcagctacaatccagctaccattctgcttttattttctggttgggataaggctggattattctgagtccaagctaggcccttttgctaatcttgttcatacctcttatcttcctcccacagctcctgggcaacctgctggtctctctgctggcccatcactttggcaaag

SEQ ID NO: 44 - DNA, 1438 bp, artificial
  FIX intron
ggtttgtttccttttttaaaatacattgagtatgcttgccttttagatatagaaatatctgatgctgtcttcttcactaaattttgattacatgatttgacagcaatattgaagagtctaacagccagcacgcaggttggtaagtactggttctttgttagctaggttttcttcttcttcatttttaaaactaaatagatcgacaatgcttatgatgcatttatgtttaataaacactgttcagttcatgatttggtcatgtaattcctgttagaaaacattcatctccttggtttaaaaaaattaaaagtgggaaaacaaagaaatagcagaatatagtgaaaaaaaataaccacattatttttgtttggacttaccactttgaaatcaaaatgggaaacaaaagcacaaacaatggccttatttacacaaaaagtctgattttaagatatatgacatttcaaggtttcagaagtatgtaatgaggtgtgtctctaattttttaaattatatatcttcaatttaaagttttagttaaaacataaagattaacctttcattagcaagctgttagttatcaccaacgcttttcatggattaggaaaaaatcattttgtctctatgtcaaacatcttggagttgatatttggggaaacacaatactcagttgagttccctaggggagaaaagcacgcttaagaattgacataaagagtaggaagttagctaatgcaacatatatcactttgttttttcacaactacagtgactttatgtatttcccagaggaaggcatacagggaagaaattatcccatttggacaaacagcatgttctcacaggaagcatttatcacacttacttgtcaactttctagaatcaaatctagtagctgacagtaccaggatcaggggtgccaaccctaagcacccccagaaagctgactggccctgtggttcccactccagacatgatgtcagctgtgaaatcgacgtcgctggaccataattaggcttctgttcttcaggagacatttgttcaaagtcatttgggcaaccatattctgaaaacagcccagccagggtgatggatcactttgcaaagatcctcaatgagctattttcaagtgatgacaaagtgtgaagttaaccgctcatttgagaactttctttttcatccaaagtaaattcaaatatgattagaaatctgaccttttattactggaattctcttgactaaaagtaaaattgaattttaattcctaaatctccatgtgtatacagtactgtgggaacatcacagattttggctccatgccctaaagagaaattggctttcagattatttggattaaaaacaaagactttcttaagagatgtaaaattttcatgatgttttcttttttgctaaaactaaagaattattcttttacatttca

SEQ ID NO: 45 - DNA, 1438 bp, artificial
  Modified FIX intron
ggtttgtttccttttttaaaatacattgagtatgcttgccttttagatatagaaatatctgatgctgtcttcttcactaaattttgattacatgatttgacagcaatattgaagagtctaacagccagcacgcaggttggtaagtactggttctttgttagctaggttttcttcttcttcatttttaaaactaaatagatcgacattgcttttgttgcatttatgtttaataaacactgttcagttcatgatttggtcatgtaattcctgttagaaaacattcatctccttggtttaaaaaaattaaaagtgggaaaacaaagaaatagcagaatatagtgaaaaaaaataaccacattatttttgtttggacttaccactttgaaatcaaattgggaaacaaaagcacaaacaatggccttatttacacaaaaagtctgattttaagatatatgacatttcaaggtttcagaagtatgtaatgaggtgtgtctctaattttttaaattatatatcttcaatttaaagttttagttaaaacataaagattaacctttcattagcaagctgttagttatcaccaacgcttttcatggattaggaaaaaatcattttgtctctttgtcaaacatcttggagttgatatttggggaaacacaatactcagttgagttccctaggggagaaaagcacgcttaagaattgacataaagagtaggaagttagctattgcaacatatatcactttgttttttcacaactacagtgactttttgtatttcccagaggaaggcatacagggaagaaattatcccatttggacaaacagcttgttctcacaggaagcatttatcacacttacttgtcaactttctagaatcaaatctagtagctgacagtaccaggatcaggggtgccaaccctaagcacccccagaaagctgactggccctgtggttcccactccagacatgatgtcagctgtgaaatcgacgtcgctggaccataattaggcttctgttcttcaggagacatttgttcaaagtcatttgggcaaccatattctgaaaacagcccagccagggtgttggatcactttgcaaagatcctcattgagctattttcaagtgttgacaaagtgtgaagttaaccgctcatttgagaactttctttttcatccaaagtaaattcaaatatgattagaaatctgaccttttattactggaattctcttgactaaaagtaaaattgaattttaattcctaaatctccatgtgtatacagtactgtgggaacatcacagattttggctccatgccctaaagagaaattggctttcagattatttggattaaaaacaaagactttcttaagagatgtaaaattttcttgttgttttcttttttgctaaaactaaagaattattcttttacatttca

SEQ ID NO: 46 - DNA, 881 bp, artificial
  Chicken beta-globin intron
gcgggagtcgctgcgttgccttcgccccgtgccccgctccgccgccgcctcgcgccgcccgccccggctctgactgaccgcgttactcccacaggtgagcgggcgggacggcccttctcctccgggctgtaattagcgcttggtttaatgacggcttgtttcttttctgtggctgcgtgaaagccttgaggggctccgggagggccctttgtgcggggggagcggctcggggggtgcgtgcgtgtgtgtgtgcgtggggagcgccgcgtgcggctccgcgctgcccggcggctgtgagcgctgcgggcgcggcgcggggctttgtgcgctccgcagtgtgcgcgaggggagcgcggccgggggcggtgccccgcggtgcggggggggctgcgaggggaacaaaggctgcgtgcggggtgtgtgcgtgggggggtgagcagggggtgtgggcgcgtcggtcgggctgcaaccccccctgcacccccctccccgagttgctgagcacggcccggcttcgggtgcggggctccgtacggggcgtggcgcggggctcgccgtgccgggcggggggtggcggcaggtgggggtgccgggcggggcggggccgcctcgggccggggagggctcgggggaggggcgcggcggcccccggagcgccggcggctgtcgaggcgcggcgagccgcagccattgccttttatggtaatcgtgcgagagggcgcagggacttcctttgtcccaaatctgtgcggagccgaaatctgggaggcgccgccgcaccccctctagcgggcgcggggcgaagcggtgcggcgccggcaggaaggaaatgggcggggagggccttcgtgcgtcgccgcgccgccgtccccttctccctc

SEQ ID NO: 47 - DNA, 881 bp, artificial
  modified chicken-beta globin intron
gcgggagtcgctgcgttgccttcgccccgtgccccgctccgccgccgcctcgcgccgcccgccccggctctgactgaccgcgttactcccacaggtgagcgggcgggacggcccttctcctccgggctgtaattagcgcttggtttaatgacggcttgtttcttttctgtggctgcgtgaaagccttgaggggctccgggagggccctttgtgcggggggagcggctcggggggtgcgtgcgtgtgtgtgtgcgtggggagcgccgcgtgcggctccgcgctgcccggcggctgtgagcgctgcgggcgcggcgcggggctttgtgcgctccgcagtgtgcgcgaggggagcgcggccgggggcggtgccccgcggtgcggggggggctgcgaggggaacaaaggctgcgtgcggggtgtgtgcgtgggggggtgagcagggggtgtgggcgcgtcggtcgggctgcaaccccccctgcacccccctccccgagttgctgagcacggcccggcttcgggtgcggggctccgtacggggcgtggcgcggggctcgccgtgccgggcggggggtggcggcaggtgggggtgccgggcggggcggggccgcctcgggccggggagggctcgggggaggggcgcggcggcccccggagcgccggcggctgtcgaggcgcggcgagccgcagccattgccttttttggtaatcgtgcgagagggcgcagggacttcctttgtcccaaatctgtgcggagccgaaatctgggaggcgccgccgcaccccctctagcgggcgcggggcgaagcggtgcggcgccggcaggaaggaattgggcggggagggccttcgtgcgtcgccgcgccgccgtccccttctccctc

SEQ ID NO: 48 - protein, 1518 aa, artificial
  D1a + D2,3 hGDE
MEKLEKTLFRLEQGYELQFRLGPTLQGKAVTVYTNYPFPGETFNREKFRSLDWENPTEREDDSDKYCKLNLQQSGSFQYYFLQGNEKSGGGYIVVDPILRVGADNHVLPLDCVTLQTFLAKCLGPFDEWESRLRVAKESGYNMIHFTPLQTLGLSRSCYSLANQLELNPDFSRPNRKYTWNDVGQLVEKLKKEWNVICITDVVYNHTAANSKWIQEHPECAYNLVNSPHLKPAWVLDRALWRFSCDVAEGKYKEKGIPALIENDHHMNSIRKIIWEDIFPKLKLWEFFQVDVNKAVEQFRRLLTQENRRVTKSDPNQHLTIIQDPEYRRFGCTVDMNIALTTFIPHDKGPAAIEECCNWFHKRMEELNSEKHRLINYHQEQAVNCLLGNVFYERLAGHGPKLGPVTRKHPLVTRYFTFPFEEIDFSMEESMIHLPNKACFLMAHNGWVMGDDPLRNFAEPGSEVYLRRELICWGDSVKLRYGNKPEDCPYLWAHMKKYTEITATYFQGVRLDNCHSTPLHVAEYMLDAARNLQPNLYVVAELFTGSEDLDNVFVTRLGISSLIREAMSAYNSHEEGRLVYRYGGEPVGSFVQPCLRPLMPAIAHALFMDITHDNECPIVHRSAYDALPSTTIVSMACCASGSTRGYDELVPHQISVVSEERFYTKWNPEALPSNTGEVNFQSGIIAARCAISKLHQELGAKGFIQVYVDQVDEDIVAVTRHSPSIHQSVVAVTRTAFRNPKTSFYSKEVPQMCIPGKIEEVVLEARTIERNTKPYRKDENSINGTPDITVEIREHIQLNESKIVKQAGVATKGPNEYIQEIEFENLSPGSVIIFRVSLDPHAQVAVGILRNHLTQFSPHFKSGSLAVDNADPILKIPFASLAYRLTLAELNQILYRCESEEKEDGGGCYDIPNWSALKYAGLQGLMSVLAEIRPKNDLGHPFCNNLRSGDWMIDYVSNRLISRSGTIAEVGKWLQAMFFYLKQIPRYLIPCYFDAILIGAYTTLLDTAWKQMSSFVQNGSTFVKHLSLGSVQLCGVGKFPSLPILSPALMDVPYRLNEITKEKEQCCVSLAAGLPHFSSGIFRCWGRDTFIALRGILLITGRYVEARNIILAFAGTLRHGLIPNLLGEGIYARYNCRDAVWWWLQCIQDYCKMVPNGLDILKCPVSRMYPTDDSAPLPAGTLDQPLFEVIQEAMQKHMQGIQFRERNAGPQIDRNMKDEGFNITAGVDEETGFVYGGNRFNCGTWMDKMGESDRARNRGIPATPRDGSAVEIVGLSKSAVRWLLELSKKNIFPYHEVTVKRHGKAIKVSYDEWNRKIQDNFEKLFHVSEDPSDLNEKHPNLVHKRGIYKDSYGASSPWCDYQLRPNFTIAMVVAPELFTTEKAWKALEIAEKKLLGPLGMKTLDPDDMVYCGIYDNALDNDNYNLAKGFNYHQGPEWLWPIGYFLRAKLYFSRLMGPETTAKTIVLVKNVLSRHYVHLERSPWKGLPELTNENAQYCPFSCETQAWSIATILETLYDL

SEQ ID NO: 49 - protein, 1503 aa, artificial
  D1b1 + D2,3 hGDE
MLQFRLGPTLQGKAVTVYTNYPFPGETFNREKFRSLDWENPTEREDDSDKYCKLNLQQSGSFQYYFLQGNEKSGGGYIVVDPILRVGADNHVLPLDCVTLQTFLAKCLGPFDEWESRLRVAKESGYNMIHFTPLQTLGLSRSCYSLANQLELNPDFSRPNRKYTWNDVGQLVEKLKKEWNVICITDVVYNHTAANSKWIQEHPECAYNLVNSPHLKPAWVLDRALWRFSCDVAEGKYKEKGIPALIENDHHMNSIRKIIWEDIFPKLKLWEFFQVDVNKAVEQFRRLLTQENRRVTKSDPNQHLTIIQDPEYRRFGCTVDMNIALTTFIPHDKGPAAIEECCNWFHKRMEELNSEKHRLINYHQEQAVNCLLGNVFYERLAGHGPKLGPVTRKHPLVTRYFTFPFEEIDFSMEESMIHLPNKACFLMAHNGWVMGDDPLRNFAEPGSEVYLRRELICWGDSVKLRYGNKPEDCPYLWAHMKKYTEITATYFQGVRLDNCHSTPLHVAEYMLDAARNLQPNLYVVAELFTGSEDLDNVFVTRLGISSLIREAMSAYNSHEEGRLVYRYGGEPVGSFVQPCLRPLMPAIAHALFMDITHDNECPIVHRSAYDALPSTTIVSMACCASGSTRGYDELVPHQISVVSEERFYTKWNPEALPSNTGEVNFQSGIIAARCAISKLHQELGAKGFIQVYVDQVDEDIVAVTRHSPSIHQSVVAVTRTAFRNPKTSFYSKEVPQMCIPGKIEEVVLEARTIERNTKPYRKDENSINGTPDITVEIREHIQLNESKIVKQAGVATKGPNEYIQEIEFENLSPGSVIIFRVSLDPHAQVAVGILRNHLTQFSPHFKSGSLAVDNADPILKIPFASLAYRLTLAELNQILYRCESEEKEDGGGCYDIPNWSALKYAGLQGLMSVLAEIRPKNDLGHPFCNNLRSGDWMIDYVSNRLISRSGTIAEVGKWLQAMFFYLKQIPRYLIPCYFDAILIGAYTTLLDTAWKQMSSFVQNGSTFVKHLSLGSVQLCGVGKFPSLPILSPALMDVPYRLNEITKEKEQCCVSLAAGLPHFSSGIFRCWGRDTFIALRGILLITGRYVEARNIILAFAGTLRHGLIPNLLGEGIYARYNCRDAVWWWLQCIQDYCKMVPNGLDILKCPVSRMYPTDDSAPLPAGTLDQPLFEVIQEAMQKHMQGIQFRERNAGPQIDRNMKDEGFNITAGVDEETGFVYGGNRFNCGTWMDKMGESDRARNRGIPATPRDGSAVEIVGLSKSAVRWLLELSKKNIFPYHEVTVKRHGKAIKVSYDEWNRKIQDNFEKLFHVSEDPSDLNEKHPNLVHKRGIYKDSYGASSPWCDYQLRPNFTIAMVVAPELFTTEKAWKALEIAEKKLLGPLGMKTLDPDDMVYCGIYDNALDNDNYNLAKGFNYHQGPEWLWPIGYFLRAKLYFSRLMGPETTAKTIVLVKNVLSRHYVHLERSPWKGLPELTNENAQYCPFSCETQAWSIATILETLYDL

SEQ ID NO: 50 - protein, 1452 aa, artificial
  D1b2 + D2,3 hGDE
MKLNLQQSGSFQYYFLQGNEKSGGGYIVVDPILRVGADNHVLPLDCVTLQTFLAKCLGPFDEWESRLRVAKESGYNMIHFTPLQTLGLSRSCYSLANQLELNPDFSRPNRKYTWNDVGQLVEKLKKEWNVICITDVVYNHTAANSKWIQEHPECAYNLVNSPHLKPAWVLDRALWRFSCDVAEGKYKEKGIPALIENDHHMNSIRKIIWEDIFPKLKLWEFFQVDVNKAVEQFRRLLTQENRRVTKSDPNQHLTIIQDPEYRRFGCTVDMNIALTTFIPHDKGPAAIEECCNWFHKRMEELNSEKHRLINYHQEQAVNCLLGNVFYERLAGHGPKLGPVTRKHPLVTRYFTFPFEEIDFSMEESMIHLPNKACFLMAHNGWVMGDDPLRNFAEPGSEVYLRRELICWGDSVKLRYGNKPEDCPYLWAHMKKYTEITATYFQGVRLDNCHSTPLHVAEYMLDAARNLQPNLYVVAELFTGSEDLDNVFVTRLGISSLIREAMSAYNSHEEGRLVYRYGGEPVGSFVQPCLRPLMPAIAHALFMDITHDNECPIVHRSAYDALPSTTIVSMACCASGSTRGYDELVPHQISVVSEERFYTKWNPEALPSNTGEVNFQSGIIAARCAISKLHQELGAKGFIQVYVDQVDEDIVAVTRHSPSIHQSVVAVTRTAFRNPKTSFYSKEVPQMCIPGKIEEVVLEARTIERNTKPYRKDENSINGTPDITVEIREHIQLNESKIVKQAGVATKGPNEYIQEIEFENLSPGSVIIFRVSLDPHAQVAVGILRNHLTQFSPHFKSGSLAVDNADPILKIPFASLAYRLTLAELNQILYRCESEEKEDGGGCYDIPNWSALKYAGLQGLMSVLAEIRPKNDLGHPFCNNLRSGDWMIDYVSNRLISRSGTIAEVGKWLQAMFFYLKQIPRYLIPCYFDAILIGAYTTLLDTAWKQMSSFVQNGSTFVKHLSLGSVQLCGVGKFPSLPILSPALMDVPYRLNEITKEKEQCCVSLAAGLPHFSSGIFRCWGRDTFIALRGILLITGRYVEARNIILAFAGTLRHGLIPNLLGEGIYARYNCRDAVWWWLQCIQDYCKMVPNGLDILKCPVSRMYPTDDSAPLPAGTLDQPLFEVIQEAMQKHMQGIQFRERNAGPQIDRNMKDEGFNITAGVDEETGFVYGGNRFNCGTWMDKMGESDRARNRGIPATPRDGSAVEIVGLSKSAVRWLLELSKKNIFPYHEVTVKRHGKAIKVSYDEWNRKIQDNFEKLFHVSEDPSDLNEKHPNLVHKRGIYKDSYGASSPWCDYQLRPNFTIAMVVAPELFTTEKAWKALEIAEKKLLGPLGMKTLDPDDMVYCGIYDNALDNDNYNLAKGFNYHQGPEWLWPIGYFLRAKLYFSRLMGPETTAKTIVLVKNVLSRHYVHLERSPWKGLPELTNENAQYCPFSCETQAWSIATILETLYDL

SEQ ID NO: 51 - protein, 1430 aa, artificial
  D1b3 + D2,3 hGDE
MGGYIVVDPILRVGADNHVLPLDCVTLQTFLAKCLGPFDEWESRLRVAKESGYNMIHFTPLQTLGLSRSCYSLANQLELNPDFSRPNRKYTWNDVGQLVEKLKKEWNVICITDVVYNHTAANSKWIQEHPECAYNLVNSPHLKPAWVLDRALWRFSCDVAEGKYKEKGIPALIENDHHMNSIRKIIWEDIFPKLKLWEFFQVDVNKAVEQFRRLLTQENRRVTKSDPNQHLTIIQDPEYRRFGCTVDMNIALTTFIPHDKGPAAIEECCNWFHKRMEELNSEKHRLINYHQEQAVNCLLGNVFYERLAGHGPKLGPVTRKHPLVTRYFTFPFEEIDFSMEESMIHLPNKACFLMAHNGWVMGDDPLRNFAEPGSEVYLRRELICWGDSVKLRYGNKPEDCPYLWAHMKKYTEITATYFQGVRLDNCHSTPLHVAEYMLDAARNLQPNLYVVAELFTGSEDLDNVFVTRLGISSLIREAMSAYNSHEEGRLVYRYGGEPVGSFVQPCLRPLMPAIAHALFMDITHDNECPIVHRSAYDALPSTTIVSMACCASGSTRGYDELVPHQISVVSEERFYTKWNPEALPSNTGEVNFQSGIIAARCAISKLHQELGAKGFIQVYVDQVDEDIVAVTRHSPSIHQSVVAVTRTAFRNPKTSFYSKEVPQMCIPGKIEEVVLEARTIERNTKPYRKDENSINGTPDITVEIREHIQLNESKIVKQAGVATKGPNEYIQEIEFENLSPGSVIIFRVSLDPHAQVAVGILRNHLTQFSPHFKSGSLAVDNADPILKIPFASLAYRLTLAELNQILYRCESEEKEDGGGCYDIPNWSALKYAGLQGLMSVLAEIRPKNDLGHPFCNNLRSGDWMIDYVSNRLISRSGTIAEVGKWLQAMFFYLKQIPRYLIPCYFDAILIGAYTTLLDTAWKQMSSFVQNGSTFVKHLSLGSVQLCGVGKFPSLPILSPALMDVPYRLNEITKEKEQCCVSLAAGLPHFSSGIFRCWGRDTFIALRGILLITGRYVEARNIILAFAGTLRHGLIPNLLGEGIYARYNCRDAVWWWLQCIQDYCKMVPNGLDILKCPVSRMYPTDDSAPLPAGTLDQPLFEVIQEAMQKHMQGIQFRERNAGPQIDRNMKDEGFNITAGVDEETGFVYGGNRFNCGTWMDKMGESDRARNRGIPATPRDGSAVEIVGLSKSAVRWLLELSKKNIFPYHEVTVKRHGKAIKVSYDEWNRKIQDNFEKLFHVSEDPSDLNEKHPNLVHKRGIYKDSYGASSPWCDYQLRPNFTIAMVVAPELFTTEKAWKALEIAEKKLLGPLGMKTLDPDDMVYCGIYDNALDNDNYNLAKGFNYHQGPEWLWPIGYFLRAKLYFSRLMGPETTAKTIVLVKNVLSRHYVHLERSPWKGLPELTNENAQYCPFSCETQAWSIATILETLYDL

SEQ ID NO: 52 - protein, 1404 aa, artificial
  D1c + D2,3 hGDE
MQTFLAKCLGPFDEWESRLRVAKESGYNMIHFTPLQTLGLSRSCYSLANQLELNPDFSRPNRKYTWNDVGQLVEKLKKEWNVICITDVVYNHTAANSKWIQEHPECAYNLVNSPHLKPAWVLDRALWRFSCDVAEGKYKEKGIPALIENDHHMNSIRKIIWEDIFPKLKLWEFFQVDVNKAVEQFRRLLTQENRRVTKSDPNQHLTIIQDPEYRRFGCTVDMNIALTTFIPHDKGPAAIEECCNWFHKRMEELNSEKHRLINYHQEQAVNCLLGNVFYERLAGHGPKLGPVTRKHPLVTRYFTFPFEEIDFSMEESMIHLPNKACFLMAHNGWVMGDDPLRNFAEPGSEVYLRRELICWGDSVKLRYGNKPEDCPYLWAHMKKYTEITATYFQGVRLDNCHSTPLHVAEYMLDAARNLQPNLYVVAELFTGSEDLDNVFVTRLGISSLIREAMSAYNSHEEGRLVYRYGGEPVGSFVQPCLRPLMPAIAHALFMDITHDNECPIVHRSAYDALPSTTIVSMACCASGSTRGYDELVPHQISVVSEERFYTKWNPEALPSNTGEVNFQSGIIAARCAISKLHQELGAKGFIQVYVDQVDEDIVAVTRHSPSIHQSVVAVTRTAFRNPKTSFYSKEVPQMCIPGKIEEVVLEARTIERNTKPYRKDENSINGTPDITVEIREHIQLNESKIVKQAGVATKGPNEYIQEIEFENLSPGSVIIFRVSLDPHAQVAVGILRNHLTQFSPHFKSGSLAVDNADPILKIPFASLAYRLTLAELNQILYRCESEEKEDGGGCYDIPNWSALKYAGLQGLMSVLAEIRPKNDLGHPFCNNLRSGDWMIDYVSNRLISRSGTIAEVGKWLQAMFFYLKQIPRYLIPCYFDAILIGAYTTLLDTAWKQMSSFVQNGSTFVKHLSLGSVQLCGVGKFPSLPILSPALMDVPYRLNEITKEKEQCCVSLAAGLPHFSSGIFRCWGRDTFIALRGILLITGRYVEARNIILAFAGTLRHGLIPNLLGEGIYARYNCRDAVWWWLQCIQDYCKMVPNGLDILKCPVSRMYPTDDSAPLPAGTLDQPLFEVIQEAMQKHMQGIQFRERNAGPQIDRNMKDEGFNITAGVDEETGFVYGGNRFNCGTWMDKMGESDRARNRGIPATPRDGSAVEIVGLSKSAVRWLLELSKKNIFPYHEVTVKRHGKAIKVSYDEWNRKIQDNFEKLFHVSEDPSDLNEKHPNLVHKRGIYKDSYGASSPWCDYQLRPNFTIAMVVAPELFTTEKAWKALEIAEKKLLGPLGMKTLDPDDMVYCGIYDNALDNDNYNLAKGFNYHQGPEWLWPIGYFLRAKLYFSRLMGPETTAKTIVLVKNVLSRHYVHLERSPWKGLPELTNENAQYCPFSCETQAWSIATILETLYDL

SEQ ID NO: 53 - DNA, 4557 bp, artificial
  D1a + D2,3 hGDE
atggaaaagctggaaaagaccctgttccggctcgagcagggctacgagctgcagtttagactgggccctacactgcagggcaaagccgtgaccgtgtacacaaactaccccttccctggcgaaaccttcaaccgcgagaagttcagaagcctggactgggagaaccccaccgagagagaggacgacagcgacaagtactgcaagctgaacctgcagcagagcggctccttccagtactacttcctgcaaggcaacgagaagtccggcggaggctacatcgtggtggaccctattctgagagtgggcgccgacaatcacgtgctgcctctggattgtgtgaccctgcagaccttcctggccaagtgtctgggccctttcgatgagtgggagagcagactgcgcgtggccaaagaaagcggctacaacatgatccacttcacccctctgcagaccctgggcctgagcagaagctgttacagcctggccaaccagctggaactgaaccccgacttcagcagacccaaccggaagtacacctggaacgatgtgggccagctggtggaaaaactgaagaaagaatggaacgtgatctgcatcaccgacgtggtgtacaaccacaccgccgccaacagcaagtggatccaagagcaccctgagtgcgcctacaacctggtcaacagccctcacctgaaacctgcctgggtgctcgatagagccctgtggcggtttagctgtgatgtggccgagggcaagtacaaagagaagggcatccccgctctgatcgagaacgaccaccacatgaacagcatccggaagatcatctgggaagatattttccccaagctgaagctgtgggagttcttccaggtggacgtgaacaaggccgtggaacagttcagacggctgctgacccaagagaacagaagagtgaccaagagcgaccccaaccagcacctgaccatcattcaggaccccgagtatcggagattcggctgcaccgtggacatgaatatcgccctgaccaccttcattccccacgacaaaggacctgccgccatcgaggaatgctgcaactggttccacaagcggatggaagaattgaacagcgagaagcaccggctgatcaactaccaccaagagcaggccgtgaactgcctgctgggcaacgtgttctatgagagactggccggacacggccctaagctgggacctgtgacaagaaagcaccctctggttacccggtacttcacctttccattcgaagagatcgacttctccatggaagagagcatgatccatctgcctaacaaggcctgcttcctgatggctcacaacggctgggttatgggcgacgaccctctgagaaatttcgccgagcctggcagcgaggtgtacctgagaagagaactgatctgttggggcgacagcgtgaagctgagatacggcaacaagcccgaggactgcccttacctgtgggcccatatgaagaagtacacagagatcaccgccacctactttcagggcgtcagactggacaactgccacagcacacctctgcacgtggccgagtacatgctggacgccgctagaaatctgcagcccaacctgtatgtggtggccgagctgtttaccggctccgaggacctggacaatgtgttcgtgaccagactgggcatcagcagcctgatcagagaagccatgtccgcctacaatagccacgaagagggcagactggtgtacagatatggcggcgagcctgtgggcagcttcgttcagccttgtctgaggcctctgatgcccgccattgctcacgccctgttcatggacatcacccacgataacgagtgccccatcgtgcacagaagcgcctacgacgctctgcctagcaccaccattgtgtccatggcctgttgtgccagcggcagcacaagaggctatgacgaactggtgccccaccagatttccgtggtgtccgaggaacggttctacaccaagtggaaccccgaggctctgcccagcaataccggcgaagtgaatttccagagcggcatcattgccgccagatgcgccatcagcaagctgcaccaagaactgggcgccaagggcttcattcaggtgtacgtggaccaggtcgacgaggacattgtggccgtgacaagacacagccccagcatccatcagagcgtggtggctgtgaccagaaccgccttcagaaaccccaagaccagcttctacagcaaagaggtgccccagatgtgcatccccggcaagattgaggaagtggtgctcgaggcccggaccatcgagagaaacaccaagccttaccggaaggacgagaactccatcaacggcacccctgacatcaccgtggaaatcagagagcacatccagctcaacgagagcaagatcgtgaaacaggccggcgtggccacaaagggccccaacgagtatatccaagagattgagttcgagaatctgagccccggcagcgtgatcatcttcagagtgtccctggatcctcacgctcaggtggccgtgggcatcctgagaaatcacctgacacagttcagcccacacttcaagagcggaagcctggccgtggacaacgccgatcctatcctgaagatccccttcgcctctctggcctacagactgacactggctgagctgaaccagatcctgtacagatgcgagtccgaagagaaagaggatggcggaggctgctacgacatccccaattggagcgccctgaagtatgccggactgcagggactgatgtctgtgctggccgagatcagacccaagaacgacctgggacaccccttctgcaacaacctgagatccggcgactggatgatcgactacgtgtccaacagactgatcagcagatccggcacaatcgccgaagtcggcaaatggctgcaggccatgttcttctacctgaagcagatccctcggtatctgatcccctgctacttcgacgccatcctgatcggcgcctacaccacactgctggataccgcctggaagcagatgtccagcttcgtgcagaacggcagcaccttcgtgaagcacctgtctctgggaagcgtgcagctgtgtggcgtgggcaaatttcccagcctgcctatcctgtctcctgcactgatggacgtgccctaccggctgaatgagatcaccaaagaaaaagagcagtgctgcgtcagcctggctgctggcctgcctcatttttccagcggcatcttccggtgttggggcagagacacctttattgccctgagaggcatcctgctgattaccggcagatacgtggaagcccggaacatcatcctggcctttgccggcacactgcggcacggactgattcctaatctgctcggcgagggcatctacgccagatacaactgcagagatgccgtgtggtggtggctccagtgcatccaggactactgcaagatggtgcccaacggcctggacatcctgaagtgccctgtgtccagaatgtaccctaccgacgatagcgcccctctgcctgccggaacacttgaccagcctctgttcgaagtgattcaagaggccatgcagaaacacatgcagggaatccagtttcgcgagcggaatgccggacctcagatcgacagaaacatgaaggatgagggcttcaacatcaccgctggcgtggacgaagagacaggctttgtgtacggcggcaaccggttcaattgcggcacctggatggacaagatgggcgagtctgaccgggccagaaacagaggaattcccgccacacctagagatggcagcgctgtggaaatcgtgggcctgtctaagtctgctgtgcggtggctgctcgaactgagcaagaagaatatctttccgtaccacgaagtgaccgtgaagcggcacggcaaggccatcaaggtgtcctacgacgagtggaacagaaagatccaggacaacttcgaaaagctgttccatgtgtctgaggaccccagcgacctgaacgaaaagcaccccaacctggtgcacaagcgcggcatctacaaggacagctacggcgcctcttctccttggtgcgattaccagctgcggcccaacttcaccattgccatggtggttgcccctgagctgttcaccacagagaaggcctggaaggccctggaaatcgccgagaagaaactgctgggccctctgggcatgaagacactggaccccgacgacatggtgtactgcggaatctacgacaacgccctggataacgacaactacaatctggccaaggggttcaattaccatcagggacccgagtggctgtggcctatcggctatttcctgcgggccaagctgtacttctccagactgatgggccctgagacaaccgccaagacaatcgtgctcgtgaagaacgtgctgagccggcactatgtgcacctggaaagaagcccctggaagggactgcccgagctgaccaatgagaacgcccagtactgccccttcagctgcgaaacacaggcctggtctatcgccaccatcctggaaaccctgtacgacctgtga

SEQ ID NO: 54 - DNA, 4512 bp, artificial
  D1b1 + D2,3 hGDE
atgctgcagtttagactgggccctacactgcagggcaaagccgtgaccgtgtacacaaactaccccttccctggcgaaaccttcaaccgcgagaagttcagaagcctggactgggagaaccccaccgagagagaggacgacagcgacaagtactgcaagctgaacctgcagcagagcggctccttccagtactacttcctgcaaggcaacgagaagtccggcggaggctacatcgtggtggaccctattctgagagtgggcgccgacaatcacgtgctgcctctggattgtgtgaccctgcagaccttcctggccaagtgtctgggccctttcgatgagtgggagagcagactgcgcgtggccaaagaaagcggctacaacatgatccacttcacccctctgcagaccctgggcctgagcagaagctgttacagcctggccaaccagctggaactgaaccccgacttcagcagacccaaccggaagtacacctggaacgatgtgggccagctggtggaaaaactgaagaaagaatggaacgtgatctgcatcaccgacgtggtgtacaaccacaccgccgccaacagcaagtggatccaagagcaccctgagtgcgcctacaacctggtcaacagccctcacctgaaacctgcctgggtgctcgatagagccctgtggcggtttagctgtgatgtggccgagggcaagtacaaagagaagggcatccccgctctgatcgagaacgaccaccacatgaacagcatccggaagatcatctgggaagatattttccccaagctgaagctgtgggagttcttccaggtggacgtgaacaaggccgtggaacagttcagacggctgctgacccaagagaacagaagagtgaccaagagcgaccccaaccagcacctgaccatcattcaggaccccgagtatcggagattcggctgcaccgtggacatgaatatcgccctgaccaccttcattccccacgacaaaggacctgccgccatcgaggaatgctgcaactggttccacaagcggatggaagaattgaacagcgagaagcaccggctgatcaactaccaccaagagcaggccgtgaactgcctgctgggcaacgtgttctatgagagactggccggacacggccctaagctgggacctgtgacaagaaagcaccctctggttacccggtacttcacctttccattcgaagagatcgacttctccatggaagagagcatgatccatctgcctaacaaggcctgcttcctgatggctcacaacggctgggttatgggcgacgaccctctgagaaatttcgccgagcctggcagcgaggtgtacctgagaagagaactgatctgttggggcgacagcgtgaagctgagatacggcaacaagcccgaggactgcccttacctgtgggcccatatgaagaagtacacagagatcaccgccacctactttcagggcgtcagactggacaactgccacagcacacctctgcacgtggccgagtacatgctggacgccgctagaaatctgcagcccaacctgtatgtggtggccgagctgtttaccggctccgaggacctggacaatgtgttcgtgaccagactgggcatcagcagcctgatcagagaagccatgtccgcctacaatagccacgaagagggcagactggtgtacagatatggcggcgagcctgtgggcagcttcgttcagccttgtctgaggcctctgatgcccgccattgctcacgccctgttcatggacatcacccacgataacgagtgccccatcgtgcacagaagcgcctacgacgctctgcctagcaccaccattgtgtccatggcctgttgtgccagcggcagcacaagaggctatgacgaactggtgccccaccagatttccgtggtgtccgaggaacggttctacaccaagtggaaccccgaggctctgcccagcaataccggcgaagtgaatttccagagcggcatcattgccgccagatgcgccatcagcaagctgcaccaagaactgggcgccaagggcttcattcaggtgtacgtggaccaggtcgacgaggacattgtggccgtgacaagacacagccccagcatccatcagagcgtggtggctgtgaccagaaccgccttcagaaaccccaagaccagcttctacagcaaagaggtgccccagatgtgcatccccggcaagattgaggaagtggtgctcgaggcccggaccatcgagagaaacaccaagccttaccggaaggacgagaactccatcaacggcacccctgacatcaccgtggaaatcagagagcacatccagctcaacgagagcaagatcgtgaaacaggccggcgtggccacaaagggccccaacgagtatatccaagagattgagttcgagaatctgagccccggcagcgtgatcatcttcagagtgtccctggatcctcacgctcaggtggccgtgggcatcctgagaaatcacctgacacagttcagcccacacttcaagagcggaagcctggccgtggacaacgccgatcctatcctgaagatccccttcgcctctctggcctacagactgacactggctgagctgaaccagatcctgtacagatgcgagtccgaagagaaagaggatggcggaggctgctacgacatccccaattggagcgccctgaagtatgccggactgcagggactgatgtctgtgctggccgagatcagacccaagaacgacctgggacaccccttctgcaacaacctgagatccggcgactggatgatcgactacgtgtccaacagactgatcagcagatccggcacaatcgccgaagtcggcaaatggctgcaggccatgttcttctacctgaagcagatccctcggtatctgatcccctgctacttcgacgccatcctgatcggcgcctacaccacactgctggataccgcctggaagcagatgtccagcttcgtgcagaacggcagcaccttcgtgaagcacctgtctctgggaagcgtgcagctgtgtggcgtgggcaaatttcccagcctgcctatcctgtctcctgcactgatggacgtgccctaccggctgaatgagatcaccaaagaaaaagagcagtgctgcgtcagcctggctgctggcctgcctcatttttccagcggcatcttccggtgttggggcagagacacctttattgccctgagaggcatcctgctgattaccggcagatacgtggaagcccggaacatcatcctggcctttgccggcacactgcggcacggactgattcctaatctgctcggcgagggcatctacgccagatacaactgcagagatgccgtgtggtggtggctccagtgcatccaggactactgcaagatggtgcccaacggcctggacatcctgaagtgccctgtgtccagaatgtaccctaccgacgatagcgcccctctgcctgccggaacacttgaccagcctctgttcgaagtgattcaagaggccatgcagaaacacatgcagggaatccagtttcgcgagcggaatgccggacctcagatcgacagaaacatgaaggatgagggcttcaacatcaccgctggcgtggacgaagagacaggctttgtgtacggcggcaaccggttcaattgcggcacctggatggacaagatgggcgagtctgaccgggccagaaacagaggaattcccgccacacctagagatggcagcgctgtggaaatcgtgggcctgtctaagtctgctgtgcggtggctgctcgaactgagcaagaagaatatctttccgtaccacgaagtgaccgtgaagcggcacggcaaggccatcaaggtgtcctacgacgagtggaacagaaagatccaggacaacttcgaaaagctgttccatgtgtctgaggaccccagcgacctgaacgaaaagcaccccaacctggtgcacaagcgcggcatctacaaggacagctacggcgcctcttctccttggtgcgattaccagctgcggcccaacttcaccattgccatggtggttgcccctgagctgttcaccacagagaaggcctggaaggccctggaaatcgccgagaagaaactgctgggccctctgggcatgaagacactggaccccgacgacatggtgtactgcggaatctacgacaacgccctggataacgacaactacaatctggccaaggggttcaattaccatcagggacccgagtggctgtggcctatcggctatttcctgcgggccaagctgtacttctccagactgatgggccctgagacaaccgccaagacaatcgtgctcgtgaagaacgtgctgagccggcactatgtgcacctggaaagaagcccctggaagggactgcccgagctgaccaatgagaacgcccagtactgccccttcagctgcgaaacacaggcctggtctatcgccaccatcctggaaaccctgtacgacctgtga

SEQ ID NO: 55 - DNA, 4359 bp, artificial
  D1b2 + D2,3 hGDE
atgaagctgaacctgcagcagagcggctccttccagtactacttcctgcaaggcaacgagaagtccggcggaggctacatcgtggtggaccctattctgagagtgggcgccgacaatcacgtgctgcctctggattgtgtgaccctgcagaccttcctggccaagtgtctgggccctttcgatgagtgggagagcagactgcgcgtggccaaagaaagcggctacaacatgatccacttcacccctctgcagaccctgggcctgagcagaagctgttacagcctggccaaccagctggaactgaaccccgacttcagcagacccaaccggaagtacacctggaacgatgtgggccagctggtggaaaaactgaagaaagaatggaacgtgatctgcatcaccgacgtggtgtacaaccacaccgccgccaacagcaagtggatccaagagcaccctgagtgcgcctacaacctggtcaacagccctcacctgaaacctgcctgggtgctcgatagagccctgtggcggtttagctgtgatgtggccgagggcaagtacaaagagaagggcatccccgctctgatcgagaacgaccaccacatgaacagcatccggaagatcatctgggaagatattttccccaagctgaagctgtgggagttcttccaggtggacgtgaacaaggccgtggaacagttcagacggctgctgacccaagagaacagaagagtgaccaagagcgaccccaaccagcacctgaccatcattcaggaccccgagtatcggagattcggctgcaccgtggacatgaatatcgccctgaccaccttcattccccacgacaaaggacctgccgccatcgaggaatgctgcaactggttccacaagcggatggaagaattgaacagcgagaagcaccggctgatcaactaccaccaagagcaggccgtgaactgcctgctgggcaacgtgttctatgagagactggccggacacggccctaagctgggacctgtgacaagaaagcaccctctggttacccggtacttcacctttccattcgaagagatcgacttctccatggaagagagcatgatccatctgcctaacaaggcctgcttcctgatggctcacaacggctgggttatgggcgacgaccctctgagaaatttcgccgagcctggcagcgaggtgtacctgagaagagaactgatctgttggggcgacagcgtgaagctgagatacggcaacaagcccgaggactgcccttacctgtgggcccatatgaagaagtacacagagatcaccgccacctactttcagggcgtcagactggacaactgccacagcacacctctgcacgtggccgagtacatgctggacgccgctagaaatctgcagcccaacctgtatgtggtggccgagctgtttaccggctccgaggacctggacaatgtgttcgtgaccagactgggcatcagcagcctgatcagagaagccatgtccgcctacaatagccacgaagagggcagactggtgtacagatatggcggcgagcctgtgggcagcttcgttcagccttgtctgaggcctctgatgcccgccattgctcacgccctgttcatggacatcacccacgataacgagtgccccatcgtgcacagaagcgcctacgacgctctgcctagcaccaccattgtgtccatggcctgttgtgccagcggcagcacaagaggctatgacgaactggtgccccaccagatttccgtggtgtccgaggaacggttctacaccaagtggaaccccgaggctctgcccagcaataccggcgaagtgaatttccagagcggcatcattgccgccagatgcgccatcagcaagctgcaccaagaactgggcgccaagggcttcattcaggtgtacgtggaccaggtcgacgaggacattgtggccgtgacaagacacagccccagcatccatcagagcgtggtggctgtgaccagaaccgccttcagaaaccccaagaccagcttctacagcaaagaggtgccccagatgtgcatccccggcaagattgaggaagtggtgctcgaggcccggaccatcgagagaaacaccaagccttaccggaaggacgagaactccatcaacggcacccctgacatcaccgtggaaatcagagagcacatccagctcaacgagagcaagatcgtgaaacaggccggcgtggccacaaagggccccaacgagtatatccaagagattgagttcgagaatctgagccccggcagcgtgatcatcttcagagtgtccctggatcctcacgctcaggtggccgtgggcatcctgagaaatcacctgacacagttcagcccacacttcaagagcggaagcctggccgtggacaacgccgatcctatcctgaagatccccttcgcctctctggcctacagactgacactggctgagctgaaccagatcctgtacagatgcgagtccgaagagaaagaggatggcggaggctgctacgacatccccaattggagcgccctgaagtatgccggactgcagggactgatgtctgtgctggccgagatcagacccaagaacgacctgggacaccccttctgcaacaacctgagatccggcgactggatgatcgactacgtgtccaacagactgatcagcagatccggcacaatcgccgaagtcggcaaatggctgcaggccatgttcttctacctgaagcagatccctcggtatctgatcccctgctacttcgacgccatcctgatcggcgcctacaccacactgctggataccgcctggaagcagatgtccagcttcgtgcagaacggcagcaccttcgtgaagcacctgtctctgggaagcgtgcagctgtgtggcgtgggcaaatttcccagcctgcctatcctgtctcctgcactgatggacgtgccctaccggctgaatgagatcaccaaagaaaaagagcagtgctgcgtcagcctggctgctggcctgcctcatttttccagcggcatcttccggtgttggggcagagacacctttattgccctgagaggcatcctgctgattaccggcagatacgtggaagcccggaacatcatcctggcctttgccggcacactgcggcacggactgattcctaatctgctcggcgagggcatctacgccagatacaactgcagagatgccgtgtggtggtggctccagtgcatccaggactactgcaagatggtgcccaacggcctggacatcctgaagtgccctgtgtccagaatgtaccctaccgacgatagcgcccctctgcctgccggaacacttgaccagcctctgttcgaagtgattcaagaggccatgcagaaacacatgcagggaatccagtttcgcgagcggaatgccggacctcagatcgacagaaacatgaaggatgagggcttcaacatcaccgctggcgtggacgaagagacaggctttgtgtacggcggcaaccggttcaattgcggcacctggatggacaagatgggcgagtctgaccgggccagaaacagaggaattcccgccacacctagagatggcagcgctgtggaaatcgtgggcctgtctaagtctgctgtgcggtggctgctcgaactgagcaagaagaatatctttccgtaccacgaagtgaccgtgaagcggcacggcaaggccatcaaggtgtcctacgacgagtggaacagaaagatccaggacaacttcgaaaagctgttccatgtgtctgaggaccccagcgacctgaacgaaaagcaccccaacctggtgcacaagcgcggcatctacaaggacagctacggcgcctcttctccttggtgcgattaccagctgcggcccaacttcaccattgccatggtggttgcccctgagctgttcaccacagagaaggcctggaaggccctggaaatcgccgagaagaaactgctgggccctctgggcatgaagacactggaccccgacgacatggtgtactgcggaatctacgacaacgccctggataacgacaactacaatctggccaaggggttcaattaccatcagggacccgagtggctgtggcctatcggctatttcctgcgggccaagctgtacttctccagactgatgggccctgagacaaccgccaagacaatcgtgctcgtgaagaacgtgctgagccggcactatgtgcacctggaaagaagcccctggaagggactgcccgagctgaccaatgagaacgcccagtactgccccttcagctgcgaaacacaggcctggtctatcgccaccatcctggaaaccctgtacgacctgtga

SEQ ID NO: 56 - DNA, 4293 bp, artificial
  D1b3 + D2,3 hGDE
atgggaggctacatcgtggtggaccctattctgagagtgggcgccgacaatcacgtgctgcctctggattgtgtgaccctgcagaccttcctggccaagtgtctgggccctttcgatgagtgggagagcagactgcgcgtggccaaagaaagcggctacaacatgatccacttcacccctctgcagaccctgggcctgagcagaagctgttacagcctggccaaccagctggaactgaaccccgacttcagcagacccaaccggaagtacacctggaacgatgtgggccagctggtggaaaaactgaagaaagaatggaacgtgatctgcatcaccgacgtggtgtacaaccacaccgccgccaacagcaagtggatccaagagcaccctgagtgcgcctacaacctggtcaacagccctcacctgaaacctgcctgggtgctcgatagagccctgtggcggtttagctgtgatgtggccgagggcaagtacaaagagaagggcatccccgctctgatcgagaacgaccaccacatgaacagcatccggaagatcatctgggaagatattttccccaagctgaagctgtgggagttcttccaggtggacgtgaacaaggccgtggaacagttcagacggctgctgacccaagagaacagaagagtgaccaagagcgaccccaaccagcacctgaccatcattcaggaccccgagtatcggagattcggctgcaccgtggacatgaatatcgccctgaccaccttcattccccacgacaaaggacctgccgccatcgaggaatgctgcaactggttccacaagcggatggaagaattgaacagcgagaagcaccggctgatcaactaccaccaagagcaggccgtgaactgcctgctgggcaacgtgttctatgagagactggccggacacggccctaagctgggacctgtgacaagaaagcaccctctggttacccggtacttcacctttccattcgaagagatcgacttctccatggaagagagcatgatccatctgcctaacaaggcctgcttcctgatggctcacaacggctgggttatgggcgacgaccctctgagaaatttcgccgagcctggcagcgaggtgtacctgagaagagaactgatctgttggggcgacagcgtgaagctgagatacggcaacaagcccgaggactgcccttacctgtgggcccatatgaagaagtacacagagatcaccgccacctactttcagggcgtcagactggacaactgccacagcacacctctgcacgtggccgagtacatgctggacgccgctagaaatctgcagcccaacctgtatgtggtggccgagctgtttaccggctccgaggacctggacaatgtgttcgtgaccagactgggcatcagcagcctgatcagagaagccatgtccgcctacaatagccacgaagagggcagactggtgtacagatatggcggcgagcctgtgggcagcttcgttcagccttgtctgaggcctctgatgcccgccattgctcacgccctgttcatggacatcacccacgataacgagtgccccatcgtgcacagaagcgcctacgacgctctgcctagcaccaccattgtgtccatggcctgttgtgccagcggcagcacaagaggctatgacgaactggtgccccaccagatttccgtggtgtccgaggaacggttctacaccaagtggaaccccgaggctctgcccagcaataccggcgaagtgaatttccagagcggcatcattgccgccagatgcgccatcagcaagctgcaccaagaactgggcgccaagggcttcattcaggtgtacgtggaccaggtcgacgaggacattgtggccgtgacaagacacagccccagcatccatcagagcgtggtggctgtgaccagaaccgccttcagaaaccccaagaccagcttctacagcaaagaggtgccccagatgtgcatccccggcaagattgaggaagtggtgctcgaggcccggaccatcgagagaaacaccaagccttaccggaaggacgagaactccatcaacggcacccctgacatcaccgtggaaatcagagagcacatccagctcaacgagagcaagatcgtgaaacaggccggcgtggccacaaagggccccaacgagtatatccaagagattgagttcgagaatctgagccccggcagcgtgatcatcttcagagtgtccctggatcctcacgctcaggtggccgtgggcatcctgagaaatcacctgacacagttcagcccacacttcaagagcggaagcctggccgtggacaacgccgatcctatcctgaagatccccttcgcctctctggcctacagactgacactggctgagctgaaccagatcctgtacagatgcgagtccgaagagaaagaggatggcggaggctgctacgacatccccaattggagcgccctgaagtatgccggactgcagggactgatgtctgtgctggccgagatcagacccaagaacgacctgggacaccccttctgcaacaacctgagatccggcgactggatgatcgactacgtgtccaacagactgatcagcagatccggcacaatcgccgaagtcggcaaatggctgcaggccatgttcttctacctgaagcagatccctcggtatctgatcccctgctacttcgacgccatcctgatcggcgcctacaccacactgctggataccgcctggaagcagatgtccagcttcgtgcagaacggcagcaccttcgtgaagcacctgtctctgggaagcgtgcagctgtgtggcgtgggcaaatttcccagcctgcctatcctgtctcctgcactgatggacgtgccctaccggctgaatgagatcaccaaagaaaaagagcagtgctgcgtcagcctggctgctggcctgcctcatttttccagcggcatcttccggtgttggggcagagacacctttattgccctgagaggcatcctgctgattaccggcagatacgtggaagcccggaacatcatcctggcctttgccggcacactgcggcacggactgattcctaatctgctcggcgagggcatctacgccagatacaactgcagagatgccgtgtggtggtggctccagtgcatccaggactactgcaagatggtgcccaacggcctggacatcctgaagtgccctgtgtccagaatgtaccctaccgacgatagcgcccctctgcctgccggaacacttgaccagcctctgttcgaagtgattcaagaggccatgcagaaacacatgcagggaatccagtttcgcgagcggaatgccggacctcagatcgacagaaacatgaaggatgagggcttcaacatcaccgctggcgtggacgaagagacaggctttgtgtacggcggcaaccggttcaattgcggcacctggatggacaagatgggcgagtctgaccgggccagaaacagaggaattcccgccacacctagagatggcagcgctgtggaaatcgtgggcctgtctaagtctgctgtgcggtggctgctcgaactgagcaagaagaatatctttccgtaccacgaagtgaccgtgaagcggcacggcaaggccatcaaggtgtcctacgacgagtggaacagaaagatccaggacaacttcgaaaagctgttccatgtgtctgaggaccccagcgacctgaacgaaaagcaccccaacctggtgcacaagcgcggcatctacaaggacagctacggcgcctcttctccttggtgcgattaccagctgcggcccaacttcaccattgccatggtggttgcccctgagctgttcaccacagagaaggcctggaaggccctggaaatcgccgagaagaaactgctgggccctctgggcatgaagacactggaccccgacgacatggtgtactgcggaatctacgacaacgccctggataacgacaactacaatctggccaaggggttcaattaccatcagggacccgagtggctgtggcctatcggctatttcctgcgggccaagctgtacttctccagactgatgggccctgagacaaccgccaagacaatcgtgctcgtgaagaacgtgctgagccggcactatgtgcacctggaaagaagcccctggaagggactgcccgagctgaccaatgagaacgcccagtactgccccttcagctgcgaaacacaggcctggtctatcgccaccatcctggaaaccctgtacgacctgtga

SEQ ID NO: 57 - DNA, 4215 bp, artificial
  D1c + D2,3 hGDE
atgcagaccttcctggccaagtgtctgggccctttcgatgagtgggagagcagactgcgcgtggccaaagaaagcggctacaacatgatccacttcacccctctgcagaccctgggcctgagcagaagctgttacagcctggccaaccagctggaactgaaccccgacttcagcagacccaaccggaagtacacctggaacgatgtgggccagctggtggaaaaactgaagaaagaatggaacgtgatctgcatcaccgacgtggtgtacaaccacaccgccgccaacagcaagtggatccaagagcaccctgagtgcgcctacaacctggtcaacagccctcacctgaaacctgcctgggtgctcgatagagccctgtggcggtttagctgtgatgtggccgagggcaagtacaaagagaagggcatccccgctctgatcgagaacgaccaccacatgaacagcatccggaagatcatctgggaagatattttccccaagctgaagctgtgggagttcttccaggtggacgtgaacaaggccgtggaacagttcagacggctgctgacccaagagaacagaagagtgaccaagagcgaccccaaccagcacctgaccatcattcaggaccccgagtatcggagattcggctgcaccgtggacatgaatatcgccctgaccaccttcattccccacgacaaaggacctgccgccatcgaggaatgctgcaactggttccacaagcggatggaagaattgaacagcgagaagcaccggctgatcaactaccaccaagagcaggccgtgaactgcctgctgggcaacgtgttctatgagagactggccggacacggccctaagctgggacctgtgacaagaaagcaccctctggttacccggtacttcacctttccattcgaagagatcgacttctccatggaagagagcatgatccatctgcctaacaaggcctgcttcctgatggctcacaacggctgggttatgggcgacgaccctctgagaaatttcgccgagcctggcagcgaggtgtacctgagaagagaactgatctgttggggcgacagcgtgaagctgagatacggcaacaagcccgaggactgcccttacctgtgggcccatatgaagaagtacacagagatcaccgccacctactttcagggcgtcagactggacaactgccacagcacacctctgcacgtggccgagtacatgctggacgccgctagaaatctgcagcccaacctgtatgtggtggccgagctgtttaccggctccgaggacctggacaatgtgttcgtgaccagactgggcatcagcagcctgatcagagaagccatgtccgcctacaatagccacgaagagggcagactggtgtacagatatggcggcgagcctgtgggcagcttcgttcagccttgtctgaggcctctgatgcccgccattgctcacgccctgttcatggacatcacccacgataacgagtgccccatcgtgcacagaagcgcctacgacgctctgcctagcaccaccattgtgtccatggcctgttgtgccagcggcagcacaagaggctatgacgaactggtgccccaccagatttccgtggtgtccgaggaacggttctacaccaagtggaaccccgaggctctgcccagcaataccggcgaagtgaatttccagagcggcatcattgccgccagatgcgccatcagcaagctgcaccaagaactgggcgccaagggcttcattcaggtgtacgtggaccaggtcgacgaggacattgtggccgtgacaagacacagccccagcatccatcagagcgtggtggctgtgaccagaaccgccttcagaaaccccaagaccagcttctacagcaaagaggtgccccagatgtgcatccccggcaagattgaggaagtggtgctcgaggcccggaccatcgagagaaacaccaagccttaccggaaggacgagaactccatcaacggcacccctgacatcaccgtggaaatcagagagcacatccagctcaacgagagcaagatcgtgaaacaggccggcgtggccacaaagggccccaacgagtatatccaagagattgagttcgagaatctgagccccggcagcgtgatcatcttcagagtgtccctggatcctcacgctcaggtggccgtgggcatcctgagaaatcacctgacacagttcagcccacacttcaagagcggaagcctggccgtggacaacgccgatcctatcctgaagatccccttcgcctctctggcctacagactgacactggctgagctgaaccagatcctgtacagatgcgagtccgaagagaaagaggatggcggaggctgctacgacatccccaattggagcgccctgaagtatgccggactgcagggactgatgtctgtgctggccgagatcagacccaagaacgacctgggacaccccttctgcaacaacctgagatccggcgactggatgatcgactacgtgtccaacagactgatcagcagatccggcacaatcgccgaagtcggcaaatggctgcaggccatgttcttctacctgaagcagatccctcggtatctgatcccctgctacttcgacgccatcctgatcggcgcctacaccacactgctggataccgcctggaagcagatgtccagcttcgtgcagaacggcagcaccttcgtgaagcacctgtctctgggaagcgtgcagctgtgtggcgtgggcaaatttcccagcctgcctatcctgtctcctgcactgatggacgtgccctaccggctgaatgagatcaccaaagaaaaagagcagtgctgcgtcagcctggctgctggcctgcctcatttttccagcggcatcttccggtgttggggcagagacacctttattgccctgagaggcatcctgctgattaccggcagatacgtggaagcccggaacatcatcctggcctttgccggcacactgcggcacggactgattcctaatctgctcggcgagggcatctacgccagatacaactgcagagatgccgtgtggtggtggctccagtgcatccaggactactgcaagatggtgcccaacggcctggacatcctgaagtgccctgtgtccagaatgtaccctaccgacgatagcgcccctctgcctgccggaacacttgaccagcctctgttcgaagtgattcaagaggccatgcagaaacacatgcagggaatccagtttcgcgagcggaatgccggacctcagatcgacagaaacatgaaggatgagggcttcaacatcaccgctggcgtggacgaagagacaggctttgtgtacggcggcaaccggttcaattgcggcacctggatggacaagatgggcgagtctgaccgggccagaaacagaggaattcccgccacacctagagatggcagcgctgtggaaatcgtgggcctgtctaagtctgctgtgcggtggctgctcgaactgagcaagaagaatatctttccgtaccacgaagtgaccgtgaagcggcacggcaaggccatcaaggtgtcctacgacgagtggaacagaaagatccaggacaacttcgaaaagctgttccatgtgtctgaggaccccagcgacctgaacgaaaagcaccccaacctggtgcacaagcgcggcatctacaaggacagctacggcgcctcttctccttggtgcgattaccagctgcggcccaacttcaccattgccatggtggttgcccctgagctgttcaccacagagaaggcctggaaggccctggaaatcgccgagaagaaactgctgggccctctgggcatgaagacactggaccccgacgacatggtgtactgcggaatctacgacaacgccctggataacgacaactacaatctggccaaggggttcaattaccatcagggacccgagtggctgtggcctatcggctatttcctgcgggccaagctgtacttctccagactgatgggccctgagacaaccgccaagacaatcgtgctcgtgaagaacgtgctgagccggcactatgtgcacctggaaagaagcccctggaagggactgcccgagctgaccaatgagaacgcccagtactgccccttcagctgcgaaacacaggcctggtctatcgccaccatcctggaaaccctgtacgacctgtga

SEQ ID NO: 58 - DNA, 17 bp, artificial
  sNRP1 polyadenylation signal
aaataaaatacgaaatg

SEQ ID NO: 59 - DNA, 4557 bp, artificial
  delta-9 GDE (isoform 1 (SEQ ID NO:1); wt version)
atggagaaactggaaaagaccctcttcagacttgaacaagggtatgagctacagttccgattaggcccaactttacagggaaaagcagttaccgtgtatacaaattacccatttcctggagaaacatttaatagagaaaaattccgttctctggattgggaaaatccaacagaaagagaagatgattctgataaatactgtaaacttaatctgcaacaatctggttcatttcagtattatttccttcaaggaaatgagaaaagtggtggaggttacatagttgtggaccccattttacgtgttggtgctgataatcatgtgctacccttggactgtgttactcttcagacatttttagctaagtgtttgggaccttttgatgaatgggaaagcagacttagggttgcaaaagaatcaggctacaacatgattcattttaccccattgcagactcttggactatctaggtcatgctactcccttgccaatcagttagaattaaatcctgacttttcaagacctaatagaaagtatacctggaatgatgttggacagctagtggaaaaattaaaaaaggaatggaatgttatttgtattactgatgttgtctacaatcatactgctgctaatagtaaatggatccaggaacatccagaatgtgcctataatcttgtaaattctccacacttaaaacctgcctgggtcttagacagagcactttggcgtttctcctgtgatgttgcagaagggaaatacaaagaaaagggaatacctgctttgattgaaaatgatcaccatatgaactccatccgaaaaataatttgggaggatatttttccaaagcttaaactctgggaatttttccaagtagatgtcaacaaagcggttgagcaatttagaagacttcttacacaagaaaataggcgagtaaccaagtctgatccaaaccaacaccttacgattattcaagatcctgaatacagacggtttggctgtactgtagatatgaacattgcactaacgactttcataccacatgacaaggggccagcagcaattgaagaatgctgtaattggtttcataaaagaatggaggaattaaattcagagaagcatcgactcattaactatcatcaggaacaggcagttaattgccttttgggaaatgtgttttatgaacgactggctggccatggtccaaaactaggacctgtcactagaaagcatcctttagttaccaggtattttactttcccatttgaagagatagacttctccatggaagaatctatgattcatctgccaaataaagcttgttttctgatggcacacaatggatgggtaatgggagatgatcctcttcgaaactttgctgaaccgggttcagaagtttacctaaggagagaacttatttgctggggagacagtgttaaattacgctatgggaataaaccagaggactgtccttatctctgggcacacatgaaaaaatacactgaaataactgcaacttatttccagggagtacgtcttgataactgccactcaacacctcttcacgtagctgagtacatgttggatgctgctaggaatttgcaacccaatttatatgtagtagctgaactgttcacaggaagtgaggacctagacaatgtctttgttactagactgggcattagttccttaataagagaggcaatgagtgcatataatagtcatgaagagggcagattagtttaccgatatggaggagaacctgttggatcctttgttcagccctgtttgaggcctttaatgccagctattgcacatgccctgtttatggatattacgcatgataatgagtgtcctattgtgcatagatcagcgtatgatgctcttccaagtactacaattgtttctatggcatgttgtgctagtggaagtacaagaggctatgatgaattagtgcctcatcagatttcagtggtttctgaagaacggttttacactaagtggaatcctgaagcattgccttcaaacacaggtgaagttaatttccaaagcggcattattgcagccaggtgtgctatcagtaaacttcatcaggagcttggagccaagggttttattcaggtgtatgtggatcaagttgatgaagacatagtggcagtaacaagacactcacctagcatccatcagtctgttgtggctgtaactagaactgctttcaggaatcccaagacttcattttacagcaaggaagtgcctcaaatgtgcatccctggcaaaattgaagaagtagttcttgaagctagaactattgagagaaacacgaaaccttataggaaggatgaaaattcaatcaatggaacaccagatatcacagtagaaattagagaacatattcagcttaatgaaagtaaaattgttaaacaagctggagttgccacaaaagggcccaatgaatatattcaagaaatagaatttgaaaacttgtctccaggaagtgttattatattcagagttagtcttgatccacatgcacaagtcgctgttggcattcttcgaaatcatctgacacaattcagtcctcactttaaatctggcagcctagctgttgacaatgcagatcctatattaaaaattccttttgcttctcttgcctatagattaactttggctgagctaaatcagatcctttaccgatgtgaatcagaagaaaaggaagatggtggagggtgctatgacataccaaactggtcagcccttaaatatgcaggtcttcaaggtttaatgtctgtattggcagaaataagaccaaagaatgacttggggcatcctttttgtaataatttgaggtctggagattggatgattgactatgtcagtaaccggcttatttcacgatcaggaactattgctgaagttggtaaatggttgcaggctatgttcttctacctgaagcagatcccacgttaccttatcccatgttactttgatgctatattaattggtgcatataccactcttctggatacagcatggaagcagatgtcaagctttgttcagaatggttcaacctttgtgaaacacctttcattgggttcagttcaactgtgtggagtaggaaaattcccttccctgccaattctttcacctgccctaatggatgtaccttataggttaaatgagatcacaaaagaaaaggagcaatgttgtgtttctctagctgcaggcttacctcatttttcttctggtattttccgctgctggggaagggatacttttattgcacttagaggtatactgctgattactggacgctatgtagaagccaggaatattattttagcatttgcgggtaccctgaggcatggtctcattcctaatctactgggtgaaggaatttatgccagatacaattgtcgggatgctgtgtggtggtggctgcagtgtatccaggattactgtaaaatggttccaaatggactagacattctcaagtgcccagtttccagaatgtatcctacagatgattctgctcctttgcctgctggcacactggatcagccattgtttgaagtcatacaggaagcaatgcaaaaacacatgcagggcatacagttccgagaaaggaatgctggtccccagatagatcgaaacatgaaggacgaaggttttaatataactgcaggagttgatgaagaaacaggatttgtttatggaggaaatcgtttcaattgtggcacatggatggataaaatgggagaaagtgacagagctagaaacagaggaatcccagccacaccaagagatgggtctgctgtggaaattgtgggcctgagtaaatctgctgttcgctggttgctggaattatccaaaaaaaatattttcccttatcatgaagtcacagtaaaaagacatggaaaggctataaaggtctcatatgatgagtggaacagaaaaatacaagacaactttgaaaagctatttcatgtttccgaagacccttcagatttaaatgaaaagcatccaaatctggttcacaaacgtggcatatacaaagatagttatggagcttcaagtccttggtgtgactatcagctcaggcctaattttaccatagcaatggttgtggcccctgagctctttactacagaaaaagcatggaaagctttggagattgcagaaaaaaaattgcttggtccccttggcatgaaaactttagatccagatgatatggtttactgtggaatttatgacaacgcattagacaatgacaactacaatcttgctaaaggtttcaattatcaccaaggacctgagtggctgtggcctattgggtattttcttcgtgcaaaattatatttttccagattgatgggcccggagactactgcaaagactatagttttggttaaaaatgttctttcccgacattatgttcatcttgagagatccccttggaaaggacttccagaactgaccaatgagaatgcccagtactgtcctttcagctgtgaaacacaagcctggtcaattgctactattcttgagacactttatgatttatag

SEQ ID NO: 60 - DNA, 4512 bp, artificial
  delta-10 GDE (isoform 1 (SEQ ID NO:1); wt version)
atgctacagttccgattaggcccaactttacagggaaaagcagttaccgtgtatacaaattacccatttcctggagaaacatttaatagagaaaaattccgttctctggattgggaaaatccaacagaaagagaagatgattctgataaatactgtaaacttaatctgcaacaatctggttcatttcagtattatttccttcaaggaaatgagaaaagtggtggaggttacatagttgtggaccccattttacgtgttggtgctgataatcatgtgctacccttggactgtgttactcttcagacatttttagctaagtgtttgggaccttttgatgaatgggaaagcagacttagggttgcaaaagaatcaggctacaacatgattcattttaccccattgcagactcttggactatctaggtcatgctactcccttgccaatcagttagaattaaatcctgacttttcaagacctaatagaaagtatacctggaatgatgttggacagctagtggaaaaattaaaaaaggaatggaatgttatttgtattactgatgttgtctacaatcatactgctgctaatagtaaatggatccaggaacatccagaatgtgcctataatcttgtaaattctccacacttaaaacctgcctgggtcttagacagagcactttggcgtttctcctgtgatgttgcagaagggaaatacaaagaaaagggaatacctgctttgattgaaaatgatcaccatatgaactccatccgaaaaataatttgggaggatatttttccaaagcttaaactctgggaatttttccaagtagatgtcaacaaagcggttgagcaatttagaagacttcttacacaagaaaataggcgagtaaccaagtctgatccaaaccaacaccttacgattattcaagatcctgaatacagacggtttggctgtactgtagatatgaacattgcactaacgactttcataccacatgacaaggggccagcagcaattgaagaatgctgtaattggtttcataaaagaatggaggaattaaattcagagaagcatcgactcattaactatcatcaggaacaggcagttaattgccttttgggaaatgtgttttatgaacgactggctggccatggtccaaaactaggacctgtcactagaaagcatcctttagttaccaggtattttactttcccatttgaagagatagacttctccatggaagaatctatgattcatctgccaaataaagcttgttttctgatggcacacaatggatgggtaatgggagatgatcctcttcgaaactttgctgaaccgggttcagaagtttacctaaggagagaacttatttgctggggagacagtgttaaattacgctatgggaataaaccagaggactgtccttatctctgggcacacatgaaaaaatacactgaaataactgcaacttatttccagggagtacgtcttgataactgccactcaacacctcttcacgtagctgagtacatgttggatgctgctaggaatttgcaacccaatttatatgtagtagctgaactgttcacaggaagtgaggacctagacaatgtctttgttactagactgggcattagttccttaataagagaggcaatgagtgcatataatagtcatgaagagggcagattagtttaccgatatggaggagaacctgttggatcctttgttcagccctgtttgaggcctttaatgccagctattgcacatgccctgtttatggatattacgcatgataatgagtgtcctattgtgcatagatcagcgtatgatgctcttccaagtactacaattgtttctatggcatgttgtgctagtggaagtacaagaggctatgatgaattagtgcctcatcagatttcagtggtttctgaagaacggttttacactaagtggaatcctgaagcattgccttcaaacacaggtgaagttaatttccaaagcggcattattgcagccaggtgtgctatcagtaaacttcatcaggagcttggagccaagggttttattcaggtgtatgtggatcaagttgatgaagacatagtggcagtaacaagacactcacctagcatccatcagtctgttgtggctgtaactagaactgctttcaggaatcccaagacttcattttacagcaaggaagtgcctcaaatgtgcatccctggcaaaattgaagaagtagttcttgaagctagaactattgagagaaacacgaaaccttataggaaggatgaaaattcaatcaatggaacaccagatatcacagtagaaattagagaacatattcagcttaatgaaagtaaaattgttaaacaagctggagttgccacaaaagggcccaatgaatatattcaagaaatagaatttgaaaacttgtctccaggaagtgttattatattcagagttagtcttgatccacatgcacaagtcgctgttggcattcttcgaaatcatctgacacaattcagtcctcactttaaatctggcagcctagctgttgacaatgcagatcctatattaaaaattccttttgcttctcttgcctatagattaactttggctgagctaaatcagatcctttaccgatgtgaatcagaagaaaaggaagatggtggagggtgctatgacataccaaactggtcagcccttaaatatgcaggtcttcaaggtttaatgtctgtattggcagaaataagaccaaagaatgacttggggcatcctttttgtaataatttgaggtctggagattggatgattgactatgtcagtaaccggcttatttcacgatcaggaactattgctgaagttggtaaatggttgcaggctatgttcttctacctgaagcagatcccacgttaccttatcccatgttactttgatgctatattaattggtgcatataccactcttctggatacagcatggaagcagatgtcaagctttgttcagaatggttcaacctttgtgaaacacctttcattgggttcagttcaactgtgtggagtaggaaaattcccttccctgccaattctttcacctgccctaatggatgtaccttataggttaaatgagatcacaaaagaaaaggagcaatgttgtgtttctctagctgcaggcttacctcatttttcttctggtattttccgctgctggggaagggatacttttattgcacttagaggtatactgctgattactggacgctatgtagaagccaggaatattattttagcatttgcgggtaccctgaggcatggtctcattcctaatctactgggtgaaggaatttatgccagatacaattgtcgggatgctgtgtggtggtggctgcagtgtatccaggattactgtaaaatggttccaaatggactagacattctcaagtgcccagtttccagaatgtatcctacagatgattctgctcctttgcctgctggcacactggatcagccattgtttgaagtcatacaggaagcaatgcaaaaacacatgcagggcatacagttccgagaaaggaatgctggtccccagatagatcgaaacatgaaggacgaaggttttaatataactgcaggagttgatgaagaaacaggatttgtttatggaggaaatcgtttcaattgtggcacatggatggataaaatgggagaaagtgacagagctagaaacagaggaatcccagccacaccaagagatgggtctgctgtggaaattgtgggcctgagtaaatctgctgttcgctggttgctggaattatccaaaaaaaatattttcccttatcatgaagtcacagtaaaaagacatggaaaggctataaaggtctcatatgatgagtggaacagaaaaatacaagacaactttgaaaagctatttcatgtttccgaagacccttcagatttaaatgaaaagcatccaaatctggttcacaaacgtggcatatacaaagatagttatggagcttcaagtccttggtgtgactatcagctcaggcctaattttaccatagcaatggttgtggcccctgagctctttactacagaaaaagcatggaaagctttggagattgcagaaaaaaaattgcttggtccccttggcatgaaaactttagatccagatgatatggtttactgtggaatttatgacaacgcattagacaatgacaactacaatcttgctaaaggtttcaattatcaccaaggacctgagtggctgtggcctattgggtattttcttcgtgcaaaattatatttttccagattgatgggcccggagactactgcaaagactatagttttggttaaaaatgttctttcccgacattatgttcatcttgagagatccccttggaaaggacttccagaactgaccaatgagaatgcccagtactgtcctttcagctgtgaaacacaagcctggtcaattgctactattcttgagacactttatgatttatag

SEQ ID NO: 61 - DNA, 4359 bp, artificial
  delta-11 GDE (isoform 1 (SEQ ID NO:1); wt version)
atgaaacttaatctgcaacaatctggttcatttcagtattatttccttcaaggaaatgagaaaagtggtggaggttacatagttgtggaccccattttacgtgttggtgctgataatcatgtgctacccttggactgtgttactcttcagacatttttagctaagtgtttgggaccttttgatgaatgggaaagcagacttagggttgcaaaagaatcaggctacaacatgattcattttaccccattgcagactcttggactatctaggtcatgctactcccttgccaatcagttagaattaaatcctgacttttcaagacctaatagaaagtatacctggaatgatgttggacagctagtggaaaaattaaaaaaggaatggaatgttatttgtattactgatgttgtctacaatcatactgctgctaatagtaaatggatccaggaacatccagaatgtgcctataatcttgtaaattctccacacttaaaacctgcctgggtcttagacagagcactttggcgtttctcctgtgatgttgcagaagggaaatacaaagaaaagggaatacctgctttgattgaaaatgatcaccatatgaactccatccgaaaaataatttgggaggatatttttccaaagcttaaactctgggaatttttccaagtagatgtcaacaaagcggttgagcaatttagaagacttcttacacaagaaaataggcgagtaaccaagtctgatccaaaccaacaccttacgattattcaagatcctgaatacagacggtttggctgtactgtagatatgaacattgcactaacgactttcataccacatgacaaggggccagcagcaattgaagaatgctgtaattggtttcataaaagaatggaggaattaaattcagagaagcatcgactcattaactatcatcaggaacaggcagttaattgccttttgggaaatgtgttttatgaacgactggctggccatggtccaaaactaggacctgtcactagaaagcatcctttagttaccaggtattttactttcccatttgaagagatagacttctccatggaagaatctatgattcatctgccaaataaagcttgttttctgatggcacacaatggatgggtaatgggagatgatcctcttcgaaactttgctgaaccgggttcagaagtttacctaaggagagaacttatttgctggggagacagtgttaaattacgctatgggaataaaccagaggactgtccttatctctgggcacacatgaaaaaatacactgaaataactgcaacttatttccagggagtacgtcttgataactgccactcaacacctcttcacgtagctgagtacatgttggatgctgctaggaatttgcaacccaatttatatgtagtagctgaactgttcacaggaagtgaggacctagacaatgtctttgttactagactgggcattagttccttaataagagaggcaatgagtgcatataatagtcatgaagagggcagattagtttaccgatatggaggagaacctgttggatcctttgttcagccctgtttgaggcctttaatgccagctattgcacatgccctgtttatggatattacgcatgataatgagtgtcctattgtgcatagatcagcgtatgatgctcttccaagtactacaattgtttctatggcatgttgtgctagtggaagtacaagaggctatgatgaattagtgcctcatcagatttcagtggtttctgaagaacggttttacactaagtggaatcctgaagcattgccttcaaacacaggtgaagttaatttccaaagcggcattattgcagccaggtgtgctatcagtaaacttcatcaggagcttggagccaagggttttattcaggtgtatgtggatcaagttgatgaagacatagtggcagtaacaagacactcacctagcatccatcagtctgttgtggctgtaactagaactgctttcaggaatcccaagacttcattttacagcaaggaagtgcctcaaatgtgcatccctggcaaaattgaagaagtagttcttgaagctagaactattgagagaaacacgaaaccttataggaaggatgaaaattcaatcaatggaacaccagatatcacagtagaaattagagaacatattcagcttaatgaaagtaaaattgttaaacaagctggagttgccacaaaagggcccaatgaatatattcaagaaatagaatttgaaaacttgtctccaggaagtgttattatattcagagttagtcttgatccacatgcacaagtcgctgttggcattcttcgaaatcatctgacacaattcagtcctcactttaaatctggcagcctagctgttgacaatgcagatcctatattaaaaattccttttgcttctcttgcctatagattaactttggctgagctaaatcagatcctttaccgatgtgaatcagaagaaaaggaagatggtggagggtgctatgacataccaaactggtcagcccttaaatatgcaggtcttcaaggtttaatgtctgtattggcagaaataagaccaaagaatgacttggggcatcctttttgtaataatttgaggtctggagattggatgattgactatgtcagtaaccggcttatttcacgatcaggaactattgctgaagttggtaaatggttgcaggctatgttcttctacctgaagcagatcccacgttaccttatcccatgttactttgatgctatattaattggtgcatataccactcttctggatacagcatggaagcagatgtcaagctttgttcagaatggttcaacctttgtgaaacacctttcattgggttcagttcaactgtgtggagtaggaaaattcccttccctgccaattctttcacctgccctaatggatgtaccttataggttaaatgagatcacaaaagaaaaggagcaatgttgtgtttctctagctgcaggcttacctcatttttcttctggtattttccgctgctggggaagggatacttttattgcacttagaggtatactgctgattactggacgctatgtagaagccaggaatattattttagcatttgcgggtaccctgaggcatggtctcattcctaatctactgggtgaaggaatttatgccagatacaattgtcgggatgctgtgtggtggtggctgcagtgtatccaggattactgtaaaatggttccaaatggactagacattctcaagtgcccagtttccagaatgtatcctacagatgattctgctcctttgcctgctggcacactggatcagccattgtttgaagtcatacaggaagcaatgcaaaaacacatgcagggcatacagttccgagaaaggaatgctggtccccagatagatcgaaacatgaaggacgaaggttttaatataactgcaggagttgatgaagaaacaggatttgtttatggaggaaatcgtttcaattgtggcacatggatggataaaatgggagaaagtgacagagctagaaacagaggaatcccagccacaccaagagatgggtctgctgtggaaattgtgggcctgagtaaatctgctgttcgctggttgctggaattatccaaaaaaaatattttcccttatcatgaagtcacagtaaaaagacatggaaaggctataaaggtctcatatgatgagtggaacagaaaaatacaagacaactttgaaaagctatttcatgtttccgaagacccttcagatttaaatgaaaagcatccaaatctggttcacaaacgtggcatatacaaagatagttatggagcttcaagtccttggtgtgactatcagctcaggcctaattttaccatagcaatggttgtggcccctgagctctttactacagaaaaagcatggaaagctttggagattgcagaaaaaaaattgcttggtccccttggcatgaaaactttagatccagatgatatggtttactgtggaatttatgacaacgcattagacaatgacaactacaatcttgctaaaggtttcaattatcaccaaggacctgagtggctgtggcctattgggtattttcttcgtgcaaaattatatttttccagattgatgggcccggagactactgcaaagactatagttttggttaaaaatgttctttcccgacattatgttcatcttgagagatccccttggaaaggacttccagaactgaccaatgagaatgcccagtactgtcctttcagctgtgaaacacaagcctggtcaattgctactattcttgagacactttatgatttatag

SEQ ID NO: 62 - DNA, 4293 bp, artificial
  delta-12 GDE (isoform 1 (SEQ ID NO:1); wt version)
atgggaggttacatagttgtggaccccattttacgtgttggtgctgataatcatgtgctacccttggactgtgttactcttcagacatttttagctaagtgtttgggaccttttgatgaatgggaaagcagacttagggttgcaaaagaatcaggctacaacatgattcattttaccccattgcagactcttggactatctaggtcatgctactcccttgccaatcagttagaattaaatcctgacttttcaagacctaatagaaagtatacctggaatgatgttggacagctagtggaaaaattaaaaaaggaatggaatgttatttgtattactgatgttgtctacaatcatactgctgctaatagtaaatggatccaggaacatccagaatgtgcctataatcttgtaaattctccacacttaaaacctgcctgggtcttagacagagcactttggcgtttctcctgtgatgttgcagaagggaaatacaaagaaaagggaatacctgctttgattgaaaatgatcaccatatgaactccatccgaaaaataatttgggaggatatttttccaaagcttaaactctgggaatttttccaagtagatgtcaacaaagcggttgagcaatttagaagacttcttacacaagaaaataggcgagtaaccaagtctgatccaaaccaacaccttacgattattcaagatcctgaatacagacggtttggctgtactgtagatatgaacattgcactaacgactttcataccacatgacaaggggccagcagcaattgaagaatgctgtaattggtttcataaaagaatggaggaattaaattcagagaagcatcgactcattaactatcatcaggaacaggcagttaattgccttttgggaaatgtgttttatgaacgactggctggccatggtccaaaactaggacctgtcactagaaagcatcctttagttaccaggtattttactttcccatttgaagagatagacttctccatggaagaatctatgattcatctgccaaataaagcttgttttctgatggcacacaatggatgggtaatgggagatgatcctcttcgaaactttgctgaaccgggttcagaagtttacctaaggagagaacttatttgctggggagacagtgttaaattacgctatgggaataaaccagaggactgtccttatctctgggcacacatgaaaaaatacactgaaataactgcaacttatttccagggagtacgtcttgataactgccactcaacacctcttcacgtagctgagtacatgttggatgctgctaggaatttgcaacccaatttatatgtagtagctgaactgttcacaggaagtgaggacctagacaatgtctttgttactagactgggcattagttccttaataagagaggcaatgagtgcatataatagtcatgaagagggcagattagtttaccgatatggaggagaacctgttggatcctttgttcagccctgtttgaggcctttaatgccagctattgcacatgccctgtttatggatattacgcatgataatgagtgtcctattgtgcatagatcagcgtatgatgctcttccaagtactacaattgtttctatggcatgttgtgctagtggaagtacaagaggctatgatgaattagtgcctcatcagatttcagtggtttctgaagaacggttttacactaagtggaatcctgaagcattgccttcaaacacaggtgaagttaatttccaaagcggcattattgcagccaggtgtgctatcagtaaacttcatcaggagcttggagccaagggttttattcaggtgtatgtggatcaagttgatgaagacatagtggcagtaacaagacactcacctagcatccatcagtctgttgtggctgtaactagaactgctttcaggaatcccaagacttcattttacagcaaggaagtgcctcaaatgtgcatccctggcaaaattgaagaagtagttcttgaagctagaactattgagagaaacacgaaaccttataggaaggatgaaaattcaatcaatggaacaccagatatcacagtagaaattagagaacatattcagcttaatgaaagtaaaattgttaaacaagctggagttgccacaaaagggcccaatgaatatattcaagaaatagaatttgaaaacttgtctccaggaagtgttattatattcagagttagtcttgatccacatgcacaagtcgctgttggcattcttcgaaatcatctgacacaattcagtcctcactttaaatctggcagcctagctgttgacaatgcagatcctatattaaaaattccttttgcttctcttgcctatagattaactttggctgagctaaatcagatcctttaccgatgtgaatcagaagaaaaggaagatggtggagggtgctatgacataccaaactggtcagcccttaaatatgcaggtcttcaaggtttaatgtctgtattggcagaaataagaccaaagaatgacttggggcatcctttttgtaataatttgaggtctggagattggatgattgactatgtcagtaaccggcttatttcacgatcaggaactattgctgaagttggtaaatggttgcaggctatgttcttctacctgaagcagatcccacgttaccttatcccatgttactttgatgctatattaattggtgcatataccactcttctggatacagcatggaagcagatgtcaagctttgttcagaatggttcaacctttgtgaaacacctttcattgggttcagttcaactgtgtggagtaggaaaattcccttccctgccaattctttcacctgccctaatggatgtaccttataggttaaatgagatcacaaaagaaaaggagcaatgttgtgtttctctagctgcaggcttacctcatttttcttctggtattttccgctgctggggaagggatacttttattgcacttagaggtatactgctgattactggacgctatgtagaagccaggaatattattttagcatttgcgggtaccctgaggcatggtctcattcctaatctactgggtgaaggaatttatgccagatacaattgtcgggatgctgtgtggtggtggctgcagtgtatccaggattactgtaaaatggttccaaatggactagacattctcaagtgcccagtttccagaatgtatcctacagatgattctgctcctttgcctgctggcacactggatcagccattgtttgaagtcatacaggaagcaatgcaaaaacacatgcagggcatacagttccgagaaaggaatgctggtccccagatagatcgaaacatgaaggacgaaggttttaatataactgcaggagttgatgaagaaacaggatttgtttatggaggaaatcgtttcaattgtggcacatggatggataaaatgggagaaagtgacagagctagaaacagaggaatcccagccacaccaagagatgggtctgctgtggaaattgtgggcctgagtaaatctgctgttcgctggttgctggaattatccaaaaaaaatattttcccttatcatgaagtcacagtaaaaagacatggaaaggctataaaggtctcatatgatgagtggaacagaaaaatacaagacaactttgaaaagctatttcatgtttccgaagacccttcagatttaaatgaaaagcatccaaatctggttcacaaacgtggcatatacaaagatagttatggagcttcaagtccttggtgtgactatcagctcaggcctaattttaccatagcaatggttgtggcccctgagctctttactacagaaaaagcatggaaagctttggagattgcagaaaaaaaattgcttggtccccttggcatgaaaactttagatccagatgatatggtttactgtggaatttatgacaacgcattagacaatgacaactacaatcttgctaaaggtttcaattatcaccaaggacctgagtggctgtggcctattgggtattttcttcgtgcaaaattatatttttccagattgatgggcccggagactactgcaaagactatagttttggttaaaaatgttctttcccgacattatgttcatcttgagagatccccttggaaaggacttccagaactgaccaatgagaatgcccagtactgtcctttcagctgtgaaacacaagcctggtcaattgctactattcttgagacactttatgatttatag

SEQ ID NO: 63 - DNA, 4215 bp, artificial
  delta-13 GDE (isoform 1 (SEQ ID NO:1); wt version)
atgcagacatttttagctaagtgtttgggaccttttgatgaatgggaaagcagacttagggttgcaaaagaatcaggctacaacatgattcattttaccccattgcagactcttggactatctaggtcatgctactcccttgccaatcagttagaattaaatcctgacttttcaagacctaatagaaagtatacctggaatgatgttggacagctagtggaaaaattaaaaaaggaatggaatgttatttgtattactgatgttgtctacaatcatactgctgctaatagtaaatggatccaggaacatccagaatgtgcctataatcttgtaaattctccacacttaaaacctgcctgggtcttagacagagcactttggcgtttctcctgtgatgttgcagaagggaaatacaaagaaaagggaatacctgctttgattgaaaatgatcaccatatgaactccatccgaaaaataatttgggaggatatttttccaaagcttaaactctgggaatttttccaagtagatgtcaacaaagcggttgagcaatttagaagacttcttacacaagaaaataggcgagtaaccaagtctgatccaaaccaacaccttacgattattcaagatcctgaatacagacggtttggctgtactgtagatatgaacattgcactaacgactttcataccacatgacaaggggccagcagcaattgaagaatgctgtaattggtttcataaaagaatggaggaattaaattcagagaagcatcgactcattaactatcatcaggaacaggcagttaattgccttttgggaaatgtgttttatgaacgactggctggccatggtccaaaactaggacctgtcactagaaagcatcctttagttaccaggtattttactttcccatttgaagagatagacttctccatggaagaatctatgattcatctgccaaataaagcttgttttctgatggcacacaatggatgggtaatgggagatgatcctcttcgaaactttgctgaaccgggttcagaagtttacctaaggagagaacttatttgctggggagacagtgttaaattacgctatgggaataaaccagaggactgtccttatctctgggcacacatgaaaaaatacactgaaataactgcaacttatttccagggagtacgtcttgataactgccactcaacacctcttcacgtagctgagtacatgttggatgctgctaggaatttgcaacccaatttatatgtagtagctgaactgttcacaggaagtgaggacctagacaatgtctttgttactagactgggcattagttccttaataagagaggcaatgagtgcatataatagtcatgaagagggcagattagtttaccgatatggaggagaacctgttggatcctttgttcagccctgtttgaggcctttaatgccagctattgcacatgccctgtttatggatattacgcatgataatgagtgtcctattgtgcatagatcagcgtatgatgctcttccaagtactacaattgtttctatggcatgttgtgctagtggaagtacaagaggctatgatgaattagtgcctcatcagatttcagtggtttctgaagaacggttttacactaagtggaatcctgaagcattgccttcaaacacaggtgaagttaatttccaaagcggcattattgcagccaggtgtgctatcagtaaacttcatcaggagcttggagccaagggttttattcaggtgtatgtggatcaagttgatgaagacatagtggcagtaacaagacactcacctagcatccatcagtctgttgtggctgtaactagaactgctttcaggaatcccaagacttcattttacagcaaggaagtgcctcaaatgtgcatccctggcaaaattgaagaagtagttcttgaagctagaactattgagagaaacacgaaaccttataggaaggatgaaaattcaatcaatggaacaccagatatcacagtagaaattagagaacatattcagcttaatgaaagtaaaattgttaaacaagctggagttgccacaaaagggcccaatgaatatattcaagaaatagaatttgaaaacttgtctccaggaagtgttattatattcagagttagtcttgatccacatgcacaagtcgctgttggcattcttcgaaatcatctgacacaattcagtcctcactttaaatctggcagcctagctgttgacaatgcagatcctatattaaaaattccttttgcttctcttgcctatagattaactttggctgagctaaatcagatcctttaccgatgtgaatcagaagaaaaggaagatggtggagggtgctatgacataccaaactggtcagcccttaaatatgcaggtcttcaaggtttaatgtctgtattggcagaaataagaccaaagaatgacttggggcatcctttttgtaataatttgaggtctggagattggatgattgactatgtcagtaaccggcttatttcacgatcaggaactattgctgaagttggtaaatggttgcaggctatgttcttctacctgaagcagatcccacgttaccttatcccatgttactttgatgctatattaattggtgcatataccactcttctggatacagcatggaagcagatgtcaagctttgttcagaatggttcaacctttgtgaaacacctttcattgggttcagttcaactgtgtggagtaggaaaattcccttccctgccaattctttcacctgccctaatggatgtaccttataggttaaatgagatcacaaaagaaaaggagcaatgttgtgtttctctagctgcaggcttacctcatttttcttctggtattttccgctgctggggaagggatacttttattgcacttagaggtatactgctgattactggacgctatgtagaagccaggaatattattttagcatttgcgggtaccctgaggcatggtctcattcctaatctactgggtgaaggaatttatgccagatacaattgtcgggatgctgtgtggtggtggctgcagtgtatccaggattactgtaaaatggttccaaatggactagacattctcaagtgcccagtttccagaatgtatcctacagatgattctgctcctttgcctgctggcacactggatcagccattgtttgaagtcatacaggaagcaatgcaaaaacacatgcagggcatacagttccgagaaaggaatgctggtccccagatagatcgaaacatgaaggacgaaggttttaatataactgcaggagttgatgaagaaacaggatttgtttatggaggaaatcgtttcaattgtggcacatggatggataaaatgggagaaagtgacagagctagaaacagaggaatcccagccacaccaagagatgggtctgctgtggaaattgtgggcctgagtaaatctgctgttcgctggttgctggaattatccaaaaaaaatattttcccttatcatgaagtcacagtaaaaagacatggaaaggctataaaggtctcatatgatgagtggaacagaaaaatacaagacaactttgaaaagctatttcatgtttccgaagacccttcagatttaaatgaaaagcatccaaatctggttcacaaacgtggcatatacaaagatagttatggagcttcaagtccttggtgtgactatcagctcaggcctaattttaccatagcaatggttgtggcccctgagctctttactacagaaaaagcatggaaagctttggagattgcagaaaaaaaattgcttggtccccttggcatgaaaactttagatccagatgatatggtttactgtggaatttatgacaacgcattagacaatgacaactacaatcttgctaaaggtttcaattatcaccaaggacctgagtggctgtggcctattgggtattttcttcgtgcaaaattatatttttccagattgatgggcccggagactactgcaaagactatagttttggttaaaaatgttctttcccgacattatgttcatcttgagagatccccttggaaaggacttccagaactgaccaatgagaatgcccagtactgtcctttcagctgtgaaacacaagcctggtcaattgctactattcttgagacactttatgatttatag